European Patent Application EP 4 434 328 A2, published September 25, 2024. Title: NOVEL GENETIC LOCI ASSOCIATED WITH EAR ROT RESISTANCE IN MAIZE. Applicant: CHINA AGRICULTURAL UNIVERSITY. Application EP. The sequence listing filed with the application follows.

SEQUENCE LISTING (1392 sequences)

SEQ ID NO: 1 - DNA, 21 bp, Zea mays;
  source 1..21: mol_type = unassigned DNA
agaccaattcgttctttttct

SEQ ID NO: 2 - DNA, 19 bp, Zea mays;
  source 1..19: mol_type = unassigned DNA
accaattcgttccttttct

SEQ ID NO: 3 - DNA, 25 bp, Zea mays;
  source 1..25: mol_type = unassigned DNA
tttgtacatgtttcgcggagatttc

SEQ ID NO: 4 - DNA, 19 bp, Zea mays;
  source 1..19: mol_type = unassigned DNA
tggctggtacacgcagaag

SEQ ID NO: 5 - DNA, 16 bp, Zea mays;
  source 1..16: mol_type = unassigned DNA
caggtccagttctgca

SEQ ID NO: 6 - DNA, 16 bp, Zea mays;
  source 1..16: mol_type = unassigned DNA
caggtccagtcctgca

SEQ ID NO: 7 - DNA, 24 bp, Zea mays;
  source 1..24: mol_type = unassigned DNA
gcatgatgctgatgggaaagatta

SEQ ID NO: 8 - DNA, 20 bp, Zea mays;
  source 1..20: mol_type = unassigned DNA
gcccctttcagtcatcgaac

SEQ ID NO: 9 - DNA, 14 bp, Zea mays;
  source 1..14: mol_type = unassigned DNA
tcccgcaaccaaat

SEQ ID NO: 10 - DNA, 14 bp, Zea mays;
  source 1..14: mol_type = unassigned DNA
tcccgcaaccaaac

SEQ ID NO: 11 - DNA, 24 bp, Zea mays;
  source 1..24: mol_type = unassigned DNA
tccccagttatccctcaaaattgg

SEQ ID NO: 12 - DNA, 21 bp, Zea mays;
  source 1..21: mol_type = unassigned DNA
tgaagccacgcaaccacttag

SEQ ID NO: 13 - DNA, 18 bp, Zea mays;
  source 1..18: mol_type = unassigned DNA
tcaacttgaatggattgg

SEQ ID NO: 14 - DNA, 17 bp, Zea mays;
  source 1..17: mol_type = unassigned DNA
caacttgaatggactgg

SEQ ID NO: 15 - DNA, 22 bp, Zea mays;
  source 1..22: mol_type = unassigned DNA
tttatctgaatttggaagtcct

SEQ ID NO: 16 - DNA, 19 bp, Zea mays;
  source 1..19: mol_type = unassigned DNA
catgggtcctagtattcgt

SEQ ID NO: 17 - DNA, 17 bp, Zea mays;
  source 1..17: mol_type = unassigned DNA
agcgggaaatgccacat

SEQ ID NO: 18 - DNA, 18 bp, Zea mays;
  source 1..18: mol_type = unassigned DNA
tagcgggaaaagccacat

SEQ ID NO: 19 - DNA, 25 bp, Zea mays;
  source 1..25: mol_type = unassigned DNA
gaatcaggtagtccaatagtagagc

SEQ ID NO: 20 - DNA, 17 bp, Zea mays;
  source 1..17: mol_type = unassigned DNA
tctgcagtcgccttccg

SEQ ID NO: 21 - DNA, 18 bp, Zea mays;
  source 1..18: mol_type = unassigned DNA
catcatgtgcctagaaag

SEQ ID NO: 22 - DNA, 18 bp, Zea mays;
  source 1..18: mol_type = unassigned DNA
catcatgtgcctagaaaa

SEQ ID NO: 23 - DNA, 27 bp, Zea mays;
  source 1..27: mol_type = unassigned DNA
gcatgatagagatatgcctaggagaag

SEQ ID NO: 24 - DNA, 21 bp, Zea mays;
  source 1..21: mol_type = unassigned DNA
tgcccctaatttcctagcaac

SEQ ID NO: 25 - DNA, 17 bp, Zea mays;
  source 1..17: mol_type = unassigned DNA
tcattgtatatctcggc

SEQ ID NO: 26 - DNA, 21 bp, Zea mays;
  source 1..21: mol_type = unassigned DNA
catattcattgtagatctcgg

SEQ ID NO: 27 - DNA, 24 bp, Zea mays;
  source 1..24: mol_type = unassigned DNA
acctagaatgctcaaaagggaaca

SEQ ID NO: 28 - DNA, 23 bp, Zea mays;
  source 1..23: mol_type = unassigned DNA
catgctgcgtcatcaatcatctg

SEQ ID NO: 29 - DNA, 15 bp, Zea mays;
  source 1..15: mol_type = unassigned DNA
cggcgctagctgcag

SEQ ID NO: 30 - DNA, 13 bp, Zea mays;
  source 1..13: mol_type = unassigned DNA
ccggcgccagctg

SEQ ID NO: 31 - DNA, 18 bp, Zea mays;
  source 1..18: mol_type = unassigned DNA
aggtcgcaggacgcgaag

SEQ ID NO: 32 - DNA, 20 bp, Zea mays;
  source 1..20: mol_type = unassigned DNA
ggcgactccatctgtaagca

SEQ ID NO: 33 - DNA, 14 bp, Zea mays;
  source 1..14: mol_type = unassigned DNA
ctgatgttcaggcc

SEQ ID NO: 34 - DNA, 15 bp, Zea mays;
  source 1..15: mol_type = unassigned DNA
ctgatgttcaagcct

SEQ ID NO: 35 - DNA, 21 bp, Zea mays;
  source 1..21: mol_type = unassigned DNA
ccacgaggaacattcgaccat

SEQ ID NO: 36 - DNA, 23 bp, Zea mays;
  source 1..23: mol_type = unassigned DNA
tctcgtcaagtccgctcttattg

SEQ ID NO: 37 - DNA, 13 bp, Zea mays;
  source 1..13: mol_type = unassigned DNA
actcctcgcctgc

SEQ ID NO: 38 - DNA, 15 bp, Zea mays;
  source 1..15: mol_type = unassigned DNA
aagtactccccgcct

SEQ ID NO: 39 - DNA, 18 bp, Zea mays;
  source 1..18: mol_type = unassigned DNA
tcctgactccggatccac

SEQ ID NO: 40 - DNA, 18 bp, Zea mays;
  source 1..18: mol_type = unassigned DNA
aggcacaggctggcagtg

SEQ ID NO: 41 - DNA, 13 bp, Zea mays;
  source 1..13: mol_type = unassigned DNA
ccgaacacgccct

SEQ ID NO: 42 - DNA, 12 bp, Zea mays;
  source 1..12: mol_type = unassigned DNA
cgaacacgcccc

SEQ ID NO: 43 - DNA, 22 bp, Zea mays;
  source 1..22: mol_type = unassigned DNA
ctgcaacagtgtcggcttgtag

SEQ ID NO: 44 - DNA, 20 bp, Zea mays;
  source 1..20: mol_type = unassigned DNA
gctccaagagcgagggatac

SEQ ID NO: 45 - DNA, 21 bp, Zea mays;
  source 1..21: mol_type = unassigned DNA
aagtttcaaattataatggta

SEQ ID NO: 46 - DNA, 22 bp, Zea mays;
  source 1..22: mol_type = unassigned DNA
tttcaaattataatgatagagt

SEQ ID NO: 47 - DNA, 23 bp, Zea mays;
  source 1..23: mol_type = unassigned DNA
tgactgatggaggttcgaagttg

SEQ ID NO: 48 - DNA, 28 bp, Zea mays;
  source 1..28: mol_type = unassigned DNA
cgactaataaaaagaaacggagggagta

SEQ ID NO: 49 - DNA, 19 bp, Zea mays;
  source 1..19: mol_type = unassigned DNA
tgggtaatttctaggaaac

SEQ ID NO: 50 - DNA, 19 bp, Zea mays;
  source 1..19: mol_type = unassigned DNA
tggtgggtaatttctaaga

SEQ ID NO: 51 - DNA, 23 bp, Zea mays;
  source 1..23: mol_type = unassigned DNA
cgattcggtggattataatggca

SEQ ID NO: 52 - DNA, 21 bp, Zea mays;
  source 1..21: mol_type = unassigned DNA
gctttcgttagggcctgtttg

SEQ ID NO: 53 - DNA, 19 bp, Zea mays;
  source 1..19: mol_type = unassigned DNA
atagaactcctagcaggca

SEQ ID NO: 54 - DNA, 16 bp, Zea mays;
  source 1..16: mol_type = unassigned DNA
aactccttgcaggcaa

SEQ ID NO: 55 - DNA, 21 bp, Zea mays;
  source 1..21: mol_type = unassigned DNA
gggatgttgcaagcaagagaa

SEQ ID NO: 56 - DNA, 18 bp, Zea mays;
  source 1..18: mol_type = unassigned DNA
gtcacgagccgtgtgaaa

SEQ ID NO: 57 - DNA, 20 bp, Zea mays;
  source 1..20: mol_type = unassigned DNA
catcttgagtgatgtaaatg

SEQ ID NO: 58 - DNA, 19 bp, Zea mays;
  source 1..19: mol_type = unassigned DNA
catcttgagtgatgtacat

SEQ ID NO: 59 - DNA, 21 bp, Zea mays;
  source 1..21: mol_type = unassigned DNA
ggcagggctaaatcaacttgc

SEQ ID NO: 60 - DNA, 26 bp, Zea mays;
  source 1..26: mol_type = unassigned DNA
caacagattggtgagatcaagagctg

SEQ ID NO: 61 - DNA, 14 bp, Zea mays;
  source 1..14: mol_type = unassigned DNA
acggacccaccttg

SEQ ID NO: 62 - DNA, 15 bp, Zea mays;
  source 1..15: mol_type = unassigned DNA
acggacccaccttaa

SEQ ID NO: 63 - DNA, 23 bp, Zea mays;
  source 1..23: mol_type = unassigned DNA
acggtcctgtatatgacaagcag

SEQ ID NO: 64 - DNA, 18 bp, Zea mays;
  source 1..18: mol_type = unassigned DNA
tgggctgagtggtgaagc

SEQ ID NO: 65 - DNA, 16 bp, Zea mays;
  source 1..16: mol_type = unassigned DNA
tgcagttgcaggtacg

SEQ ID NO: 66 - DNA, 18 bp, Zea mays;
  source 1..18: mol_type = unassigned DNA
attgcagttgcaggtacc

SEQ ID NO: 67 - DNA, 20 bp, Zea mays;
  source 1..20: mol_type = unassigned DNA
acagccactggtggttggtc

SEQ ID NO: 68 - DNA, 24 bp, Zea mays;
  source 1..24: mol_type = unassigned DNA
ggcgtacgtgccacttatatagtc

SEQ ID NO: 69 - DNA, 15 bp, Zea mays;
  source 1..15: mol_type = unassigned DNA
tggagcgtctacacc

SEQ ID NO: 70 - DNA, 17 bp, Zea mays;
  source 1..17: mol_type = unassigned DNA
catggagcatctacacc

SEQ ID NO: 71 - DNA, 22 bp, Zea mays;
  source 1..22: mol_type = unassigned DNA
cttgttctaagcgcctcctgat

SEQ ID NO: 72 - DNA, 22 bp, Zea mays;
  source 1..22: mol_type = unassigned DNA
tggtgactcttgatggagttca

SEQ ID NO: 73 - DNA, 19 bp, Zea mays;
  source 1..19: mol_type = unassigned DNA
ttctgtaattttatcaatt

SEQ ID NO: 74 - DNA, 16 bp, Zea mays;
  source 1..16: mol_type = unassigned DNA
ttctgtaattttacca

SEQ ID NO: 75 - DNA, 17 bp, Zea mays;
  source 1..17: mol_type = unassigned DNA
ctgcctacatgcagttt

SEQ ID NO: 76 - DNA, 17 bp, Zea mays;
  source 1..17: mol_type = unassigned DNA
tgccacgataagaaagg

SEQ ID NO: 77 - DNA, 16 bp, Zea mays;
  source 1..16: mol_type = unassigned DNA
tctccaggagttcgag

SEQ ID NO: 78 - DNA, 16 bp, Zea mays;
  source 1..16: mol_type = unassigned DNA
ctccaggagttcaagg

SEQ ID NO: 79 - DNA, 25 bp, Zea mays;
  source 1..25: mol_type = unassigned DNA
cctttggtgcaatctatgatcaggt

SEQ ID NO: 80 - DNA, 24 bp, Zea mays;
  source 1..24: mol_type = unassigned DNA
cgaaacgtagccaacgtaaacaac

SEQ ID NO: 81 - DNA, 17 bp, Zea mays;
  source 1..17: mol_type = unassigned DNA
cgcggaaatccgagtag

SEQ ID NO: 82 - DNA, 15 bp, Zea mays;
  source 1..15: mol_type = unassigned DNA
cggaaatccgagcag

SEQ ID NO: 83 - DNA, 20 bp, Zea mays;
  source 1..20: mol_type = unassigned DNA
gggtggactcactccgaatg

SEQ ID NO: 84 - DNA, 19 bp, Zea mays;
  source 1..19: mol_type = unassigned DNA
gagcccctctctcctcgtt

SEQ ID NO: 85 - DNA, 11 bp, Zea mays;
  source 1..11: mol_type = unassigned DNA
ctgcgccgcgt

SEQ ID NO: 86 - DNA, 12 bp, Zea mays;
  source 1..12: mol_type = unassigned DNA
ctgcgccgcatg

SEQ ID NO: 87 - DNA, 17 bp, Zea mays;
  source 1..17: mol_type = unassigned DNA
cgtcgccctgagcctac

SEQ ID NO: 88 - DNA, 20 bp, Zea mays;
  source 1..20: mol_type = unassigned DNA
tgcgacggtgatagacgatg

SEQ ID NO: 89 - DNA, 16 bp, Zea mays;
  source 1..16: mol_type = unassigned DNA
ccctataccccactac

SEQ ID NO: 90 - DNA, 15 bp, Zea mays;
  source 1..15: mol_type = unassigned DNA
cctataccccacaac

SEQ ID NO: 91 - DNA, 21 bp, Zea mays;
  source 1..21: mol_type = unassigned DNA
tccaccctgtacaatggttcc

SEQ ID NO: 92 - DNA, 24 bp, Zea mays;
  source 1..24: mol_type = unassigned DNA
gcgtacaccagtatttgtcagttc

SEQ ID NO: 93 - DNA, 17 bp, Zea mays;
  source 1..17: mol_type = unassigned DNA
tccttgtcaggatcatc

SEQ ID NO: 94 - DNA, 17 bp, Zea mays;
  source 1..17: mol_type = unassigned DNA
tccttgtcagcatcatc

SEQ ID NO: 95 - DNA, 25 bp, Zea mays;
  source 1..25: mol_type = unassigned DNA
cgccattaattcatgcttgtctctg

SEQ ID NO: 96 - DNA, 21 bp, Zea mays;
  source 1..21: mol_type = unassigned DNA
acacgctgcgttggagaatcc

SEQ ID NO: 97 - DNA, 17 bp, Zea mays;
  source 1..17: mol_type = unassigned DNA
cagccaaaatcgaacca

SEQ ID NO: 98 - DNA, 16 bp, Zea mays;
  source 1..16: mol_type = unassigned DNA
cagccaaaaccgaacc

SEQ ID NO: 99 - DNA, 15 bp, Zea mays;
  source 1..15: mol_type = unassigned DNA
gagcgagccgcctga

SEQ ID NO: 100 - DNA, 18 bp, Zea mays;
  source 1..18: mol_type = unassigned DNA
ccgtggcaactggtcctg

SEQ ID NO: 101 - DNA, 13 bp, Zea mays;
  source 1..13: mol_type = unassigned DNA
ccctgcgaacgcc

SEQ ID NO: 102 - DNA, 13 bp, Zea mays;
  source 1..13: mol_type = unassigned DNA
ccctgccaacgcc

SEQ ID NO: 103 - DNA, 18 bp, Zea mays;
  source 1..18: mol_type = unassigned DNA
tggaggccaagtcgaacg

SEQ ID NO: 104 - DNA, 15 bp, Zea mays;
  source 1..15: mol_type = unassigned DNA
ggctcgggtccagca

SEQ ID NO: 105 - DNA, 20 bp, Zea mays;
  source 1..20: mol_type = unassigned DNA
ctgcttgtgatagaaataaa

SEQ ID NO: 106 - DNA, 21 bp, Zea mays;
  source 1..21: mol_type = unassigned DNA
cttgtgatagaaacaaagatg

SEQ ID NO: 107 - DNA, 18 bp, Zea mays;
  source 1..18: mol_type = unassigned DNA
atgaagggaagaccgcat

SEQ ID NO: 108 - DNA, 19 bp, Zea mays;
  source 1..19: mol_type = unassigned DNA
tgggacatattagaccatc

SEQ ID NO: 109 - DNA, 18 bp, Zea mays;
  source 1..18: mol_type = unassigned DNA
ctttctctagccgtacta

SEQ ID NO: 110 - DNA, 18 bp, Zea mays;
  source 1..18: mol_type = unassigned DNA
ctttctctagccctacta

SEQ ID NO: 111 - DNA, 21 bp, Zea mays;
  source 1..21: mol_type = unassigned DNA
agctttgcttcctgggtgctt

SEQ ID NO: 112 - DNA, 20 bp, Zea mays;
  source 1..20: mol_type = unassigned DNA
tcggcatcacctgtatcaga

SEQ ID NO: 113 - DNA, 19 bp, Zea mays;
  source 1..19: mol_type = unassigned DNA
catgaaagttaatcctcaa

SEQ ID NO: 114 - DNA, 20 bp, Zea mays;
  source 1..20: mol_type = unassigned DNA
ttcatgaaagttaatcatca

SEQ ID NO: 115 - DNA, 28 bp, Zea mays;
  source 1..28: mol_type = unassigned DNA
cagctttttggtcgtttttctttgattg

SEQ ID NO: 116 - DNA, 23 bp, Zea mays;
  source 1..23: mol_type = unassigned DNA
ggtgagcttgtgttatgttctca

SEQ ID NO: 117 - DNA, 17 bp, Zea mays;
  source 1..17: mol_type = unassigned DNA
cgctagaccgtgatggt

SEQ ID NO: 118 - DNA, 17 bp, Zea mays;
  source 1..17: mol_type = unassigned DNA
cgctagaccctgatggt

SEQ ID NO: 119 - DNA, 21 bp, Zea mays;
  source 1..21: mol_type = unassigned DNA
tgcaaccagtgaatgtccttg

SEQ ID NO: 120 - DNA, 23 bp, Zea mays;
  source 1..23: mol_type = unassigned DNA
gtcgtttggagctagtagttgac

SEQ ID NO: 121 - DNA, 18 bp, Zea mays;
  source 1..18: mol_type = unassigned DNA
atggctgctgcttcatac

SEQ ID NO: 122 - DNA, 17 bp, Zea mays;
  source 1..17: mol_type = unassigned DNA
atggctgctgcgtcata

SEQ ID NO: 123 - DNA, 24 bp, Zea mays;
  source 1..24: mol_type = unassigned DNA
gttggaccttctctctgtaagtca

SEQ ID NO: 124 - DNA, 18 bp, Zea mays;
  source 1..18: mol_type = unassigned DNA
tgcttgcctcgctgtgat

SEQ ID NO: 125 - DNA, 21 bp, Zea mays;
  source 1..21: mol_type = unassigned DNA
attttattattcgtccgtcta

SEQ ID NO: 126 - DNA, 17 bp, Zea mays;
  source 1..17: mol_type = unassigned DNA
tattattcgcccgtcta

SEQ ID NO: 127 - DNA, 22 bp, Zea mays;
  source 1..22: mol_type = unassigned DNA
tccaaggttacctgaaccctaa

SEQ ID NO: 128 - DNA, 24 bp, Zea mays;
  source 1..24: mol_type = unassigned DNA
gagcatggacattacatggcataa

SEQ ID NO: 129 - DNA, 16 bp, Zea mays;
  source 1..16: mol_type = unassigned DNA
aattgatcacgcacta

SEQ ID NO: 130 - DNA, 18 bp, Zea mays;
  source 1..18: mol_type = unassigned DNA
aattgatcacacactatc

SEQ ID NO: 131 - DNA, 20 bp, Zea mays;
  source 1..20: mol_type = unassigned DNA
aggcaagctcgatggttcac

SEQ ID NO: 132 - DNA, 21 bp, Zea mays;
  source 1..21: mol_type = unassigned DNA
ccatgtggtcgtgggttcaag

SEQ ID NO: 133 - DNA, 15 bp, Zea mays;
  source 1..15: mol_type = unassigned DNA
cgcaaagggcgtgtg

SEQ ID NO: 134 - DNA, 17 bp, Zea mays;
  source 1..17: mol_type = unassigned DNA
acgcaaagagcgtgtgg

SEQ ID NO: 135 - DNA, 18 bp, Zea mays;
  source 1..18: mol_type = unassigned DNA
acccgcggcaaccgtaaa

SEQ ID NO: 136 - DNA, 17 bp, Zea mays;
  source 1..17: mol_type = unassigned DNA
cgtcgtcgtcggagaca

SEQ ID NO: 137 - DNA, 19 bp, Zea mays;
  source 1..19: mol_type = unassigned DNA
tctttcaagattaatgaag

SEQ ID NO: 138 - DNA, 19 bp, Zea mays;
  source 1..19: mol_type = unassigned DNA
ctttcaagattaaagaagg

SEQ ID NO: 139 - DNA, 23 bp, Zea mays;
  source 1..23: mol_type = unassigned DNA
gcagtgggttgacatcaacaatg

SEQ ID NO: 140 - DNA, 22 bp, Zea mays;
  source 1..22: mol_type = unassigned DNA
gtttagcaagctgaaagggtga

SEQ ID NO: 141 - DNA, 18 bp, Zea mays;
  source 1..18: mol_type = unassigned DNA
caggtattcgtgtgcatc

SEQ ID NO: 142 - DNA, 17 bp, Zea mays;
  source 1..17: mol_type = unassigned DNA
caggtattcgcgtgcat

SEQ ID NO: 143 - DNA, 20 bp, Zea mays;
  source 1..20: mol_type = unassigned DNA
agggcactcaggcacatgat

SEQ ID NO: 144 - DNA, 20 bp, Zea mays;
  source 1..20: mol_type = unassigned DNA
ccaccactcgcactaggaaa

SEQ ID NO: 145 - DNA, 21 bp, Zea mays;
  source 1..21: mol_type = unassigned DNA
aggttagtcgttcgaattgga

SEQ ID NO: 146 - DNA, 21 bp, Zea mays;
  source 1..21: mol_type = unassigned DNA
aaggttagtcgttcaaattgg

SEQ ID NO: 147 - DNA, 23 bp, Zea mays;
  source 1..23: mol_type = unassigned DNA
gtttggtttgtggctaaatgtgc

SEQ ID NO: 148 - DNA, 21 bp, Zea mays;
  source 1..21: mol_type = unassigned DNA
aggtgagtgtgacgtgcatag

SEQ ID NO: 149 - DNA, 14 bp, Zea mays;
  source 1..14: mol_type = unassigned DNA
catgctgcggtcgc

SEQ ID NO: 150 - DNA, 13 bp, Zea mays;
  source 1..13: mol_type = unassigned DNA
atgcggcggtcgc

SEQ ID NO: 151 - DNA, 22 bp, Zea mays;
  source 1..22: mol_type = unassigned DNA
acatgtagatgatgcggtcgtg

SEQ ID NO: 152 - DNA, 18 bp, Zea mays;
  source 1..18: mol_type = unassigned DNA
accagctcccgtttctgc

SEQ ID NO: 153 - DNA, 13 bp, Zea mays;
  source 1..13: mol_type = unassigned DNA
ccccgccttcgaa

SEQ ID NO: 154 - DNA, 13 bp, Zea mays;
  source 1..13: mol_type = unassigned DNA
tgccccaccttcg

SEQ ID NO: 155 - DNA, 18 bp, Zea mays;
  source 1..18: mol_type = unassigned DNA
gggccatcagcgttcgtc

SEQ ID NO: 156 - DNA, 20 bp, Zea mays;
  source 1..20: mol_type = unassigned DNA
agatggcgtgctcggtgttc

SEQ ID NO: 157 - DNA, 19 bp, Zea mays;
  source 1..19: mol_type = unassigned DNA
ccatccaatgtatcaattg

SEQ ID NO: 158 - DNA, 19 bp, Zea mays;
  source 1..19: mol_type = unassigned DNA
catccaatgtatcaactga

SEQ ID NO: 159 - DNA, 23 bp, Zea mays;
  source 1..23: mol_type = unassigned DNA
gaacttgatatgtagctaaagac

SEQ ID NO: 160 - DNA, 21 bp, Zea mays;
  source 1..21: mol_type = unassigned DNA
tcatgttgaagttgaattggt

SEQ ID NO: 161 - DNA, 19 bp, Zea mays;
  source 1..19: mol_type = unassigned DNA
cgagaggatgacactataa

SEQ ID NO: 162 - DNA, 19 bp, Zea mays;
  source 1..19: mol_type = unassigned DNA
agaggatgacactacaagt

SEQ ID NO: 163 - DNA, 22 bp, Zea mays;
  source 1..22: mol_type = unassigned DNA
gctatcgcccaccaataaagtg

SEQ ID NO: 164 - DNA, 23 bp, Zea mays;
  source 1..23: mol_type = unassigned DNA
atgtgtcctcaacccttagatga

SEQ ID NO: 165 - DNA, 17 bp, Zea mays;
  source 1..17: mol_type = unassigned DNA
tcaactggactaaataa

SEQ ID NO: 166 - DNA, 16 bp, Zea mays;
  source 1..16: mol_type = unassigned DNA
aagtcaactggacaaa

SEQ ID NO: 167 - DNA, 21 bp, Zea mays;
  source 1..21: mol_type = unassigned DNA
tccaagcagctatcagatcca

SEQ ID NO: 168 - DNA, 22 bp, Zea mays;
  source 1..22: mol_type = unassigned DNA
gctcttgccttctgttcttcac

SEQ ID NO: 169 - DNA, 21 bp, Zea mays;
  source 1..21: mol_type = unassigned DNA
aacaggactactcagattata

SEQ ID NO: 170 - DNA, 17 bp, Zea mays;
  source 1..17: mol_type = unassigned DNA
caggactactcagacta

SEQ ID NO: 171 - DNA, 25 bp, Zea mays;
  source 1..25: mol_type = unassigned DNA
gagggcattcttgtcttcctcatac

SEQ ID NO: 172 - DNA, 21 bp, Zea mays;
  source 1..21: mol_type = unassigned DNA
gcttcgggcctgtttgtttac

SEQ ID NO: 173 - DNA, 14 bp, Zea mays;
  source 1..14: mol_type = unassigned DNA
cccgatgcgacgtc

SEQ ID NO: 174 - DNA, 14 bp, Zea mays;
  source 1..14: mol_type = unassigned DNA
cccgaggcgacgtc

SEQ ID NO: 175 - DNA, 15 bp, Zea mays;
  source 1..15: mol_type = unassigned DNA
cgccttggcggcctt

SEQ ID NO: 176 - DNA, 20 bp, Zea mays;
  source 1..20: mol_type = unassigned DNA
ccgcgtcaagtgtttcatca

SEQ ID NO: 177 - DNA, 20 bp, Zea mays;
  source 1..20: mol_type = unassigned DNA
agcatggaaatcttgtcttc

SEQ ID NO: 178 - DNA, 20 bp, Zea mays;
  source 1..20: mol_type = unassigned DNA
tagcatggaaatcctgtctt

SEQ ID NO: 179 - DNA, 23 bp, Zea mays;
  source 1..23: mol_type = unassigned DNA
tccacccaaaagatatcatccga

SEQ ID NO: 180 - DNA, 21 bp, Zea mays;
  source 1..21: mol_type = unassigned DNA
ccacctgggaatgcaaggaat

SEQ ID NO: 181 - DNA, 19 bp, Zea mays;
  source 1..19: mol_type = unassigned DNA
caaagcatgtaccattaat

SEQ ID NO: 182 - DNA, 18 bp, Zea mays;
  source 1..18: mol_type = unassigned DNA
aaagcatgtaccatcaat

SEQ ID NO: 183 - DNA, 19 bp, Zea mays;
  source 1..19: mol_type = unassigned DNA
acgtatcccggccgtctac

SEQ ID NO: 184 - DNA, 22 bp, Zea mays;
  source 1..22: mol_type = unassigned DNA
gcggtgaaggaagatcatggtt

SEQ ID NO: 185 - DNA, 17 bp, Zea mays;
  source 1..17: mol_type = unassigned DNA
tccaggaagggccaaag

SEQ ID NO: 186 - DNA, 18 bp, Zea mays;
  source 1..18: mol_type = unassigned DNA
ccaggaaggcccaaagat

SEQ ID NO: 187 - DNA, 20 bp, Zea mays;
  source 1..20: mol_type = unassigned DNA
gcagacgtgatcctgaagca

SEQ ID NO: 188 - DNA, 17 bp, Zea mays;
  source 1..17: mol_type = unassigned DNA
tcaggcacgggctgaac

SEQ ID NO: 189 - DNA, 15 bp, Zea mays;
  source 1..15: mol_type = unassigned DNA
ccccggttgtcacat

SEQ ID NO: 190 - DNA, 16 bp, Zea mays;
  source 1..16: mol_type = unassigned DNA
cccggttatcacatgc

SEQ ID NO: 191 - DNA, 23 bp, Zea mays;
  source 1..23: mol_type = unassigned DNA
ggcaaagagggattgctacactt

SEQ ID NO: 192 - DNA, 25 bp, Zea mays;
  source 1..25: mol_type = unassigned DNA
catccacaacacaaacactgacatc

SEQ ID NO: 193 - DNA, 20 bp, Zea mays;
  source 1..20: mol_type = unassigned DNA
tcttcgtagagaaagtatgt

SEQ ID NO: 194 - DNA, 20 bp, Zea mays;
  source 1..20: mol_type = unassigned DNA
cgtagagaaagataccgtat

SEQ ID NO: 195 - DNA, 17 bp, Zea mays;
  source 1..17: mol_type = unassigned DNA
tgttcaggtaacacgag

SEQ ID NO: 196 - DNA, 20 bp, Zea mays;
  source 1..20: mol_type = unassigned DNA
cactcaatactccaaacagt

SEQ ID NO: 197 - DNA, 19 bp, Zea mays;
  source 1..19: mol_type = unassigned DNA
tccaatttctggttcacat

SEQ ID NO: 198 - DNA, 17 bp, Zea mays;
  source 1..17: mol_type = unassigned DNA
ccaatttctggctcaca

SEQ ID NO: 199 - DNA, 21 bp, Zea mays;
  source 1..21: mol_type = unassigned DNA
cctccaggccaaagatgcaat

SEQ ID NO: 200 - DNA, 23 bp, Zea mays;
  source 1..23: mol_type = unassigned DNA
cccgctctatccgttacacttct

SEQ ID NO: 201 - DNA, 16 bp, Zea mays;
  source 1..16: mol_type = unassigned DNA
taactaatagcaatgc

SEQ ID NO: 202 - DNA, 19 bp, Zea mays;
  source 1..19: mol_type = unassigned DNA
taataactaatagcaatac

SEQ ID NO: 203 - DNA, 21 bp, Zea mays;
  source 1..21: mol_type = unassigned DNA
atgaaccatatatcctaggaa

SEQ ID NO: 204 - DNA, 17 bp, Zea mays;
  source 1..17: mol_type = unassigned DNA
gaggtgctccaatcttc

SEQ ID NO: 205 - DNA, 16 bp, Zea mays;
  source 1..16: mol_type = unassigned DNA
cagtaggttgggcaac

SEQ ID NO: 206 - DNA, 14 bp, Zea mays;
  source 1..14: mol_type = unassigned DNA
ccagtaggttgcgc

SEQ ID NO: 207 - DNA, 23 bp, Zea mays;
  source 1..23: mol_type = unassigned DNA
tgttagtccaggccttctgaatc

SEQ ID NO: 208 - DNA, 25 bp, Zea mays;
  source 1..25: mol_type = unassigned DNA
acagcagaggttaaagtagcatagc

SEQ ID NO: 209 - DNA, 16 bp, Zea mays;
  source 1..16: mol_type = unassigned DNA
tggctttggatcgggt

SEQ ID NO: 210 - DNA, 18 bp, Zea mays;
  source 1..18: mol_type = unassigned DNA
ttggctttggatcgagtt

SEQ ID NO: 211 - DNA, 20 bp, Zea mays;
  source 1..20: mol_type = unassigned DNA
ttgacgtatcgggtcggatt

SEQ ID NO: 212 - DNA, 22 bp, Zea mays;
  source 1..22: mol_type = unassigned DNA
cgggctaagtacaagccatgat

SEQ ID NO: 213 - DNA, 15 bp, Zea mays;
  source 1..15: mol_type = unassigned DNA
tccgacggctagaga

SEQ ID NO: 214 - DNA, 18 bp, Zea mays;
  source 1..18: mol_type = unassigned DNA
caatatccgacagctaga

SEQ ID NO: 215 - DNA, 25 bp, Zea mays;
  source 1..25: mol_type = unassigned DNA
cagactaccatgaagagagttgtga

SEQ ID NO: 216 - DNA, 25 bp, Zea mays;
  source 1..25: mol_type = unassigned DNA
ggtagttgatttcttgtccgctgat

SEQ ID NO: 217 - DNA, 17 bp, Zea mays;
  source 1..17: mol_type = unassigned DNA
cgtttaggaatctctgg

SEQ ID NO: 218 - DNA, 18 bp, Zea mays;
  source 1..18: mol_type = unassigned DNA
cgtttaggaatatctggg

SEQ ID NO: 219 - DNA, 15 bp, Zea mays;
  source 1..15: mol_type = unassigned DNA
ggcgagaatgactgc

SEQ ID NO: 220 - DNA, 21 bp, Zea mays;
  source 1..21: mol_type = unassigned DNA
aatgacatgtgatctttgttt

SEQ ID NO: 221 - DNA, 19 bp, Zea mays;
  source 1..19: mol_type = unassigned DNA
cgagagtgtattatggtag

SEQ ID NO: 222 - DNA, 19 bp, Zea mays;
  source 1..19: mol_type = unassigned DNA
cgagagtgtattatgggag

SEQ ID NO: 223 - DNA, 17 bp, Zea mays;
  source 1..17: mol_type = unassigned DNA
tcctggcaaccgagacc

SEQ ID NO: 224 - DNA, 20 bp, Zea mays;
  source 1..20: mol_type = unassigned DNA
acaggccagcaggcagatag

SEQ ID NO: 225 - DNA, 16 bp, Zea mays;
  source 1..16: mol_type = unassigned DNA
tgttggtctgcgaggt

SEQ ID NO: 226 - DNA, 18 bp, Zea mays;
  source 1..18: mol_type = unassigned DNA
tgtgttggtctacgaggt

SEQ ID NO: 227 - DNA, 18 bp, Zea mays;
  source 1..18: mol_type = unassigned DNA
cgtcaggtgcttcaccga

SEQ ID NO: 228 - DNA, 21 bp, Zea mays;
  source 1..21: mol_type = unassigned DNA
gagggtggagacgcaagatac

SEQ ID NO: 229 - DNA, 18 bp, Zea mays;
  source 1..18: mol_type = unassigned DNA
tcacattccattggttgg

SEQ ID NO: 230 - DNA, 17 bp, Zea mays;
  source 1..17: mol_type = unassigned DNA
cacattccatcggttgg

SEQ ID NO: 231 - DNA, 18 bp, Zea mays;
  source 1..18: mol_type = unassigned DNA
ggtggaggcgcataggtt

SEQ ID NO: 232 - DNA, 19 bp, Zea mays;
  source 1..19: mol_type = unassigned DNA
acggcaggagaggaaggaa

SEQ ID NO: 233 - DNA, 18 bp, Zea mays;
  source 1..18: mol_type = unassigned DNA
atactatcctctccggga

SEQ ID NO: 234 - DNA, 14 bp, Zea mays;
  source 1..14: mol_type = unassigned DNA
tatcccctccggga

SEQ ID NO: 235 - DNA, 23 bp, Zea mays;
  source 1..23: mol_type = unassigned DNA
tgatttggatttgggaattggga

SEQ ID NO: 236 - DNA, 21 bp, Zea mays;
  source 1..21: mol_type = unassigned DNA
aaacgagcaggtgtttagcca

SEQ ID NO: 237 - DNA, 16 bp, Zea mays;
  source 1..16: mol_type = unassigned DNA
aatgacacccccttcc

SEQ ID NO: 238 - DNA, 15 bp, Zea mays;
  source 1..15: mol_type = unassigned DNA
atgacaccccctccc

SEQ ID NO: 239 - DNA, 20 bp, Zea mays;
  source 1..20: mol_type = unassigned DNA
ccaaccatttcttgctgcca

SEQ ID NO: 240 - DNA, 21 bp, Zea mays;
  source 1..21: mol_type = unassigned DNA
ttgagagctccgcgaaatgag

SEQ ID NO: 241 - DNA, 17 bp, Zea mays;
  source 1..17: mol_type = unassigned DNA
tcaccaagtactcccta

SEQ ID NO: 242 - DNA, 16 bp, Zea mays;
  source 1..16: mol_type = unassigned DNA
caccaagtactcccca

SEQ ID NO: 243 - DNA, 21 bp, Zea mays;
  source 1..21: mol_type = unassigned DNA
agcaaaggtgcggatgccatt

SEQ ID NO: 244 - DNA, 24 bp, Zea mays;
  source 1..24: mol_type = unassigned DNA
gcttccaaatcgctaccttgtttc

SEQ ID NO: 245 - DNA, 18 bp, Zea mays;
  source 1..18: mol_type = unassigned DNA
ctcgtatgccgttttgtt

SEQ ID NO: 246 - DNA, 18 bp, Zea mays;
  source 1..18: mol_type = unassigned DNA
tcgtatgccattttgttc

SEQ ID NO: 247 - DNA, 25 bp, Zea mays;
  source 1..25: mol_type = unassigned DNA
tccatcatcaaaccctaaacaccag

SEQ ID NO: 248 - DNA, 24 bp, Zea mays;
  source 1..24: mol_type = unassigned DNA
gaatgccaaccatcagaagtcaac

SEQ ID NO: 249 - DNA, 24 bp, Zea mays;
  source 1..24: mol_type = unassigned DNA
ccatgtatgttgataatttctaaa

SEQ ID NO: 250 - DNA, 23 bp, Zea mays;
  source 1..23: mol_type = unassigned DNA
accatgtatgttgataacttcta

SEQ ID NO: 251 - DNA, 23 bp, Zea mays;
  source 1..23: mol_type = unassigned DNA
gcagtatggcctatgtttgttgc

SEQ ID NO: 252 - DNA, 19 bp, Zea mays;
  source 1..19: mol_type = unassigned DNA
ccggtaccctggtgtcgtt

SEQ ID NO: 253 - DNA, 19 bp, Zea mays;
  source 1..19: mol_type = unassigned DNA
ttgaaggagagaggacaga

SEQ ID NO: 254 - DNA, 20 bp, Zea mays;
  source 1..20: mol_type = unassigned DNA
tttgaaggagagaggacaaa

SEQ ID NO: 255 - DNA, 24 bp, Zea mays;
  source 1..24: mol_type = unassigned DNA
aggagcacctcatttggttagaaa

SEQ ID NO: 256 - DNA, 19 bp, Zea mays;
  source 1..19: mol_type = unassigned DNA
ccgagcgaagtcgagaacc

SEQ ID NO: 257 - DNA, 18 bp, Zea mays;
  source 1..18: mol_type = unassigned DNA
ctgaggaacgatcgattc

SEQ ID NO: 258 - DNA, 18 bp, Zea mays;
  source 1..18: mol_type = unassigned DNA
tgaggaacgaccgattct

SEQ ID NO: 259 - DNA, 23 bp, Zea mays;
  source 1..23: mol_type = unassigned DNA
gctagtcaacacacacccacaag

SEQ ID NO: 260 - DNA, 21 bp, Zea mays;
  source 1..21: mol_type = unassigned DNA
ggagccaggctcatcacatac

SEQ ID NO: 261 - DNA, 13 bp, Zea mays;
  source 1..13: mol_type = unassigned DNA
cagtcggagcggg

SEQ ID NO: 262 - DNA, 14 bp, Zea mays;
  source 1..14: mol_type = unassigned DNA
agtcggagcagggc

SEQ ID NO: 263 - DNA, 24 bp, Zea mays;
  source 1..24: mol_type = unassigned DNA
aactcggttgttgtcagtcttacc

SEQ ID NO: 264 - DNA, 20 bp, Zea mays;
  source 1..20: mol_type = unassigned DNA
ctgaccgacctgacaggaaa

SEQ ID NO: 265 - DNA, 20 bp, Zea mays;
  source 1..20: mol_type = unassigned DNA
cggattctctctgaatgatg

SEQ ID NO: 266 - DNA, 19 bp, Zea mays;
  source 1..19: mol_type = unassigned DNA
acggattctctccgaatga

SEQ ID NO: 267 - DNA, 23 bp, Zea mays;
  source 1..23: mol_type = unassigned DNA
gatttgtgttcgacagtgggatg

SEQ ID NO: 268 - DNA, 25 bp, Zea mays;
  source 1..25: mol_type = unassigned DNA
gcaagcccgaaccaatataataacc

SEQ ID NO: 269 - DNA, 16 bp, Zea mays;
  source 1..16: mol_type = unassigned DNA
cagtgctttgacctcg

SEQ ID NO: 270 - DNA, 16 bp, Zea mays;
  source 1..16: mol_type = unassigned DNA
cagtgctttcacctcg

SEQ ID NO: 271 - DNA, 24 bp, Zea mays;
  source 1..24: mol_type = unassigned DNA
gccaagatgacaagatccaacaac

SEQ ID NO: 272 - DNA, 19 bp, Zea mays;
  source 1..19: mol_type = unassigned DNA
tgtccgccatctccagcat

SEQ ID NO: 273 - DNA, 18 bp, Zea mays;
  source 1..18: mol_type = unassigned DNA
cacattgacgttgatgac

SEQ ID NO: 274 - DNA, 17 bp, Zea mays;
  source 1..17: mol_type = unassigned DNA
cattgacgttgaggaca

SEQ ID NO: 275 - DNA, 18 bp, Zea mays;
  source 1..18: mol_type = unassigned DNA
gttgacaatggaaggaga

SEQ ID NO: 276 - DNA, 21 bp, Zea mays;
  source 1..21: mol_type = unassigned DNA
ccggatatgtatatgatgctg

SEQ ID NO: 277 - DNA, 22 bp, Zea mays;
  source 1..22: mol_type = unassigned DNA
agtattatagctaaaaatagac

SEQ ID NO: 278 - DNA, 22 bp, Zea mays;
  source 1..22: mol_type = unassigned DNA
cataagtattatagctaaaaaa

SEQ ID NO: 279 - DNA, 25 bp, Zea mays;
  source 1..25: mol_type = unassigned DNA
acacatatcacaagtcagaatgctc

SEQ ID NO: 280 - DNA, 24 bp, Zea mays;
  source 1..24: mol_type = unassigned DNA
acggttaattggtaggcacggtaa

SEQ ID NO: 281 - DNA, 15 bp, Zea mays;
  source 1..15: mol_type = unassigned DNA
cgacattgtgcgctt

SEQ ID NO: 282 - DNA, 17 bp, Zea mays;
  source 1..17: mol_type = unassigned DNA
ttcgacattgtacgctt

SEQ ID NO: 283 - DNA, 23 bp, Zea mays;
  source 1..23: mol_type = unassigned DNA
tttatgtcagaaagcttgaggca

SEQ ID NO: 284 - DNA, 22 bp, Zea mays;
  source 1..22: mol_type = unassigned DNA
tgtcggctaatcatctcaagga

SEQ ID NO: 285 - DNA, 18 bp, Zea mays;
  source 1..18: mol_type = unassigned DNA
ttcactaacgatgtaatt

SEQ ID NO: 286 - DNA, 16 bp, Zea mays;
  source 1..16: mol_type = unassigned DNA
tcactaacgatggaat

SEQ ID NO: 287 - DNA, 19 bp, Zea mays;
  source 1..19: mol_type = unassigned DNA
agtccctatgggtttccaa

SEQ ID NO: 288 - DNA, 18 bp, Zea mays;
  source 1..18: mol_type = unassigned DNA
cctcttcccatgagaact

SEQ ID NO: 289 - DNA, 19 bp, Zea mays;
  source 1..19: mol_type = unassigned DNA
tttatgctagtcaaacttt

SEQ ID NO: 290 - DNA, 19 bp, Zea mays;
  source 1..19: mol_type = unassigned DNA
tttatgctagtcaaacatt

SEQ ID NO: 291 - DNA, 23 bp, Zea mays;
  source 1..23: mol_type = unassigned DNA
tcagttaagtatcgtctagattt

SEQ ID NO: 292 - DNA, 18 bp, Zea mays;
  source 1..18: mol_type = unassigned DNA
accgcgatacatcattgg

SEQ ID NO: 293 - DNA, 17 bp, Zea mays;
  source 1..17: mol_type = unassigned DNA
ttgagaaccttcagtac

SEQ ID NO: 294 - DNA, 17 bp, Zea mays;
  source 1..17: mol_type = unassigned DNA
ttgagaaccatcagtac

SEQ ID NO: 295 - DNA, 20 bp, Zea mays;
  source 1..20: mol_type = unassigned DNA
cgttgtcagcattggtggac

SEQ ID NO: 296 - DNA, 20 bp, Zea mays;
  source 1..20: mol_type = unassigned DNA
gatcgtcgcacggatgtcta

SEQ ID NO: 297 - DNA, 20 bp, Zea mays;
  source 1..20: mol_type = unassigned DNA
caaaccatcgaatctgtaac

SEQ ID NO: 298 - DNA, 19 bp, Zea mays;
  source 1..19: mol_type = unassigned DNA
accatcgaatccgtaacaa

SEQ ID NO: 299 - DNA, 23 bp, Zea mays;
  source 1..23: mol_type = unassigned DNA
ttgccagagttgattccacctaa

SEQ ID NO: 300 - DNA, 21 bp, Zea mays;
  source 1..21: mol_type = unassigned DNA
ctgcgacattgcctctaacca

SEQ ID NO: 301 - DNA, 15 bp, Zea mays;
  source 1..15: mol_type = unassigned DNA
atcggactctcggct

SEQ ID NO: 302 - DNA, 15 bp, Zea mays;
  source 1..15: mol_type = unassigned DNA
aatcggactctcagc

SEQ ID NO: 303 - DNA, 21 bp, Zea mays;
  source 1..21: mol_type = unassigned DNA
caatccggtctcagtggttgg

SEQ ID NO: 304 - DNA, 20 bp, Zea mays;
  source 1..20: mol_type = unassigned DNA
cctgagctggctactgatga

SEQ ID NO: 305 - DNA, 22 bp, Zea mays;
  source 1..22: mol_type = unassigned DNA
atagcattagattctgagcatt

SEQ ID NO: 306 - DNA, 20 bp, Zea mays;
  source 1..20: mol_type = unassigned DNA
agcattagattctgagcata

SEQ ID NO: 307 - DNA, 22 bp, Zea mays;
  source 1..22: mol_type = unassigned DNA
ttcggcgtctacttcctgtatc

SEQ ID NO: 308 - DNA, 25 bp, Zea mays;
  source 1..25: mol_type = unassigned DNA
tgctttgtgttcgtatgcatgaata

SEQ ID NO: 309 - DNA, 15 bp, Zea mays;
  source 1..15: mol_type = unassigned DNA
ctgctgctgtttgca

SEQ ID NO: 310 - DNA, 16 bp, Zea mays;
  source 1..16: mol_type = unassigned DNA
tgctgctgctatttgc

SEQ ID NO: 311 - DNA, 24 bp, Zea mays;
  source 1..24: mol_type = unassigned DNA
ccaagacaaactctccctgtatgc

SEQ ID NO: 312 - DNA, 22 bp, Zea mays;
  source 1..22: mol_type = unassigned DNA
ggctcggaaggtctcaaagaag

SEQ ID NO: 313 - DNA, 17 bp, Zea mays;
  source 1..17: mol_type = unassigned DNA
tggttgtagtattgcaa

SEQ ID NO: 314 - DNA, 19 bp, Zea mays;
  source 1..19: mol_type = unassigned DNA
ttggttgtagtattgaaaa

SEQ ID NO: 315 - DNA, 25 bp, Zea mays;
  source 1..25: mol_type = unassigned DNA
ggtttgctcttgctgatcgatatgt

SEQ ID NO: 316 - DNA, 21 bp, Zea mays;
  source 1..21: mol_type = unassigned DNA
gctcagctactccctctgttc

SEQ ID NO: 317 - DNA, 17 bp, Zea mays;
  source 1..17: mol_type = unassigned DNA
cgaggtggtgacgatgt

SEQ ID NO: 318 - DNA, 17 bp, Zea mays;
  source 1..17: mol_type = unassigned DNA
cgaggtggtcacgatgt

SEQ ID NO: 319 - DNA, 20 bp, Zea mays;
  source 1..20: mol_type = unassigned DNA
cgggtcaagttctgctgtga

SEQ ID NO: 320 - DNA, 22 bp, Zea mays;
  source 1..22: mol_type = unassigned DNA
atcatacggcggaagtagttca

SEQ ID NO: 321 - DNA, 21 bp, Zea mays;
  source 1..21: mol_type = unassigned DNA
aaacatgaatactcgatctgc

SEQ ID NO: 322 - DNA, 20 bp, Zea mays;
  source 1..20: mol_type = unassigned DNA
caaacatgaatacccgatct

SEQ ID NO: 323 - DNA, 21 bp, Zea mays;
  source 1..21: mol_type = unassigned DNA
tggcttgagccattacctgat

SEQ ID NO: 324 - DNA, 22 bp, Zea mays;
  source 1..22: mol_type = unassigned DNA
gaaactgcaagaggcatgaaac

SEQ ID NO: 325 - DNA, 19 bp, Zea mays;
  source 1..19: mol_type = unassigned DNA
tgatgcgatttcgttgaat

SEQ ID NO: 326 - DNA, 20 bp, Zea mays;
  source 1..20: mol_type = unassigned DNA
cgtgatgcgatttagttgaa

SEQ ID NO: 327 - DNA, 22 bp, Zea mays;
  source 1..22: mol_type = unassigned DNA
cggattacaactctctgttgcc

SEQ ID NO: 328 - DNA, 24 bp, Zea mays;
  source 1..24: mol_type = unassigned DNA
cacactcaaggtgacttagaccaa

SEQ ID NO: 329 - DNA, 18 bp, Zea mays;
  source 1..18: mol_type = unassigned DNA
cagttgtttgtatagaca

SEQ ID NO: 330 - DNA, 20 bp, Zea mays;
  source 1..20: mol_type = unassigned DNA
atacagttgtttgtataaac

SEQ ID NO: 331 - DNA, 17 bp, Zea mays;
  source 1..17: mol_type = unassigned DNA
ggattggaccagcagat

SEQ ID NO: 332 - DNA, 19 bp, Zea mays;
  source 1..19: mol_type = unassigned DNA
gtgagacaaggctacatac

SEQ ID NO: 333 - DNA, 11 bp, Zea mays;
  source 1..11: mol_type = unassigned DNA
ccggccgcagt

SEQ ID NO: 334 - DNA, 13 bp, Zea mays;
  source 1..13: mol_type = unassigned DNA
ccgcagcggtgat

SEQ ID NO: 335 - DNA, 19 bp, Zea mays;
  source 1..19: mol_type = unassigned DNA
cgtcgcggtcctctctgat

SEQ ID NO: 336 - DNA, 21 bp, Zea mays;
  source 1..21: mol_type = unassigned DNA
ctgcgaatcgtccatcctgta

SEQ ID NO: 337 - DNA, 18 bp, Zea mays;
  source 1..18: mol_type = unassigned DNA
ccttgtgagaaaactcta

SEQ ID NO: 338 - DNA, 18 bp, Zea mays;
  source 1..18: mol_type = unassigned DNA
cttgtgagaaaaccctag

SEQ ID NO: 339 - DNA, 16 bp, Zea mays;
  source 1..16: mol_type = unassigned DNA
gtgcaatggctgactc

SEQ ID NO: 340 - DNA, 20 bp, Zea mays;
  source 1..20: mol_type = unassigned DNA
gcacgattatgcatgattag

SEQ ID NO: 341 - DNA, 18 bp, Zea mays;
  source 1..18: mol_type = unassigned DNA
tcaaagctaggtttatgc

SEQ ID NO: 342 - DNA, 18 bp, Zea mays;
  source 1..18: mol_type = unassigned DNA
tcaaagctaggtttaggc

SEQ ID NO: 343 - DNA, 21 bp, Zea mays;
  source 1..21: mol_type = unassigned DNA
agggttagggtttcacttcca

SEQ ID NO: 344 - DNA, 19 bp, Zea mays;
  source 1..19: mol_type = unassigned DNA
agcactggcgaggctacag

SEQ ID NO: 345 - DNA, 21 bp, Zea mays;
  source 1..21: mol_type = unassigned DNA
agatctgattggtatagggca

SEQ ID NO: 346 - DNA, 17 bp, Zea mays;
  source 1..17: mol_type = unassigned DNA
ctgattggtacagggca

SEQ ID NO: 347 - DNA, 19 bp, Zea mays;
  source 1..19: mol_type = unassigned DNA
aaggcagaggtgcttcggt

SEQ ID NO: 348 - DNA, 24 bp, Zea mays;
  source 1..24: mol_type = unassigned DNA
gtgctgcatttctaaggtgtcaag

SEQ ID NO: 349 - DNA, 22 bp, Zea mays;
  source 1..22: mol_type = unassigned DNA
ctagggaagttgtcgtttgaaa

SEQ ID NO: 350 - DNA, 19 bp, Zea mays;
  source 1..19: mol_type = unassigned DNA
agggaagttgtcgcttgaa

SEQ ID NO: 351 - DNA, 21 bp, Zea mays;
  source 1..21: mol_type = unassigned DNA
ggtgcaggcaagagagcattt

SEQ ID NO: 352 - DNA, 25 bp, Zea mays;
  source 1..25: mol_type = unassigned DNA
tggattatatggaaggtccgaaggt

SEQ ID NO: 353 - DNA, 15 bp, Zea mays;
  source 1..15: mol_type = unassigned DNA
aggcggcgaccaact

SEQ ID NO: 354 - DNA, 15 bp, Zea mays;
  source 1..15: mol_type = unassigned DNA
aggcggccaccaact

SEQ ID NO: 355 - DNA, 18 bp, Zea mays;
  source 1..18: mol_type = unassigned DNA
acgttcgccgacgaggag

SEQ ID NO: 356 - DNA, 20 bp, Zea mays;
  source 1..20: mol_type = unassigned DNA
cgcagcatgtcgacgatctc

SEQ ID NO: 357 - DNA, 19 bp, Zea mays;
  source 1..19: mol_type = unassigned DNA
agcggagcaatgactactt

SEQ ID NO: 358 - DNA, 17 bp, Zea mays;
  source 1..17: mol_type = unassigned DNA
cggagcaacgactactt

SEQ ID NO: 359 - DNA, 17 bp, Zea mays;
  source 1..17: mol_type = unassigned DNA
ggtgcacaccggactgt

SEQ ID NO: 360 - DNA, 19 bp, Zea mays;
  source 1..19: mol_type = unassigned DNA
caactgcgcgtcctctgtc

SEQ ID NO: 361 - DNA, 19 bp, Zea mays;
  source 1..19: mol_type = unassigned DNA
ccagtttcttctgtgagtg

SEQ ID NO: 362 - DNA, 18 bp, Zea mays;
  source 1..18: mol_type = unassigned DNA
cagtttcttccgtgagtg

SEQ ID NO: 363 - DNA, 23 bp, Zea mays;
  source 1..23: mol_type = unassigned DNA
tgcatctgagttcctgattgttg

SEQ ID NO: 364 - DNA, 18 bp, Zea mays;
  source 1..18: mol_type = unassigned DNA
ccgcagcacgacatcctt

SEQ ID NO: 365 - DNA, 23 bp, Zea mays;
  source 1..23: mol_type = unassigned DNA
ccatatataggttagttgatcga

SEQ ID NO: 366 - DNA, 24 bp, Zea mays;
  source 1..24: mol_type = unassigned DNA
ccatatataggttagttcatcgat

SEQ ID NO: 367 - DNA, 23 bp, Zea mays;
  source 1..23: mol_type = unassigned DNA
gcggtgagtacaagttaatccaa

SEQ ID NO: 368 - DNA, 23 bp, Zea mays;
  source 1..23: mol_type = unassigned DNA
gccgtcacttgacttgattcttc

SEQ ID NO: 369 - DNA, 12 bp, Zea mays;
  source 1..12: mol_type = unassigned DNA
acccagccccct

SEQ ID NO: 370 - DNA, 12 bp, Zea mays;
  source 1..12: mol_type = unassigned DNA
acccagcccccg

SEQ ID NO: 371 - DNA, 21 bp, Zea mays;
  source 1..21: mol_type = unassigned DNA
tgatctggctcacgtgggtag

SEQ ID NO: 372 - DNA, 20 bp, Zea mays;
  source 1..20: mol_type = unassigned DNA
cgcatgaacgtccatggaag

SEQ ID NO: 373 - DNA, 18 bp, Zea mays;
  source 1..18: mol_type = unassigned DNA
cacatgcacagtgctata

SEQ ID NO: 374 - DNA, 19 bp, Zea mays;
  source 1..19: mol_type = unassigned DNA
ccacatgcacagtactata

SEQ ID NO: 375 - DNA, 22 bp, Zea mays;
  source 1..22: mol_type = unassigned DNA
gagacccagctagagagttgac

SEQ ID NO: 376 - DNA, 19 bp, Zea mays;
  source 1..19: mol_type = unassigned DNA
tgggcacataggccagtag

SEQ ID NO: 377 - DNA, 16 bp, Zea mays;
  source 1..16: mol_type = unassigned DNA
tgcaaacaggagcatg

SEQ ID NO: 378 - DNA, 19 bp, Zea mays;
  source 1..19: mol_type = unassigned DNA
aaatgcaaacaggaacatg

SEQ ID NO: 379 - DNA, 19 bp, Zea mays;
  source 1..19: mol_type = unassigned DNA
gttgctgaaatgctaatgg

SEQ ID NO: 380 - DNA, 16 bp, Zea mays;
  source 1..16: mol_type = unassigned DNA
gtgtcgtcgtcttctc

SEQ ID NO: 381 - DNA, 14 bp, Zea mays;
  source 1..14: mol_type = unassigned DNA
ccaccaccggaatt

SEQ ID NO: 382 - DNA, 14 bp, Zea mays;
  source 1..14: mol_type = unassigned DNA
caccaccgcaattg

SEQ ID NO: 383 - DNA, 20 bp, Zea mays;
  source 1..20: mol_type = unassigned DNA
gagttcatcaagtagctcgt

SEQ ID NO: 384 - DNA, 17 bp, Zea mays;
  source 1..17: mol_type = unassigned DNA
tgcacatcagcattctc

SEQ ID NO: 385 - DNA, 19 bp, Zea mays;
  source 1..19: mol_type = unassigned DNA
cggttaccattgttgtgta

SEQ ID NO: 386 - DNA, 20 bp, Zea mays;
  source 1..20: mol_type = unassigned DNA
tcggttaccattattgtgta

SEQ ID NO: 387 - DNA, 25 bp, Zea mays;
  source 1..25: mol_type = unassigned DNA
ccttgtttgaaacctccttgtgttg

SEQ ID NO: 388 - DNA, 19 bp, Zea mays;
  source 1..19: mol_type = unassigned DNA
gtccaggtcgccttactga

SEQ ID NO: 389 - DNA, 15 bp, Zea mays;
  source 1..15: mol_type = unassigned DNA
tacaaagccgggttg

SEQ ID NO: 390 - DNA, 16 bp, Zea mays;
  source 1..16: mol_type = unassigned DNA
tacaaagccgggatgt

SEQ ID NO: 391 - DNA, 20 bp, Zea mays;
  source 1..20: mol_type = unassigned DNA
gaactgattcatctgggtaa

SEQ ID NO: 392 - DNA, 16 bp, Zea mays;
  source 1..16: mol_type = unassigned DNA
ctcctgctgtggtcac

SEQ ID NO: 393 - DNA, 22 bp, Zea mays;
  source 1..22: mol_type = unassigned DNA
caagtgaaatggtatataatac

SEQ ID NO: 394 - DNA, 21 bp, Zea mays;
  source 1..21: mol_type = unassigned DNA
aagtgaaatggtatataacac

SEQ ID NO: 395 - DNA, 21 bp, Zea mays;
  source 1..21: mol_type = unassigned DNA
catgccacaattgcagaagca

SEQ ID NO: 396 - DNA, 23 bp, Zea mays;
  source 1..23: mol_type = unassigned DNA
gcatagctcaacatgtgaactca

SEQ ID NO: 397 - DNA, 14 bp, Zea mays;
  source 1..14: mol_type = unassigned DNA
ccggctcaagccta

SEQ ID NO: 398 - DNA, 14 bp, Zea mays;
  source 1..14: mol_type = unassigned DNA
ccggcacaagccta

SEQ ID NO: 399 - DNA, 19 bp, Zea mays;
  source 1..19: mol_type = unassigned DNA
cgccctagtgctgggaatc

SEQ ID NO: 400 - DNA, 22 bp, Zea mays;
  source 1..22: mol_type = unassigned DNA
ggaccgacacgatccaataaag

SEQ ID NO: 401 - DNA, 15 bp, Zea mays;
  source 1..15: mol_type = unassigned DNA
cgggcggagtacgtg

SEQ ID NO: 402 - DNA, 14 bp, Zea mays;
  source 1..14: mol_type = unassigned DNA
cgggcggactacgt

SEQ ID NO: 403 - DNA, 16 bp, Zea mays;
  source 1..16: mol_type = unassigned DNA
agagggcgcggtctga

SEQ ID NO: 404 - DNA, 19 bp, Zea mays;
  source 1..19: mol_type = unassigned DNA
tggtcgcacttccttcttc

SEQ ID NO: 405 - DNA, 14 bp, Zea mays;
  source 1..14: mol_type = unassigned DNA
cgacagcggaggag

SEQ ID NO: 406 - DNA, 15 bp, Zea mays;
  source 1..15: mol_type = unassigned DNA
cgacagcggaagagg

SEQ ID NO: 407 - DNA, 17 bp, Zea mays;
  source 1..17: mol_type = unassigned DNA
ctcgtgcttgctttacg

SEQ ID NO: 408 - DNA, 17 bp, Zea mays;
  source 1..17: mol_type = unassigned DNA
cgcaagaggttgatagg

SEQ ID NO: 409 - DNA, 15 bp, Zea mays;
  source 1..15: mol_type = unassigned DNA
accagctactgcagc

SEQ ID NO: 410 - DNA, 14 bp, Zea mays;
  source 1..14: mol_type = unassigned DNA
ccagcgactgcagc

SEQ ID NO: 411 - DNA, 19 bp, Zea mays;
  source 1..19: mol_type = unassigned DNA
gtccctgcccgttttgtct

SEQ ID NO: 412 - DNA, 21 bp, Zea mays;
  source 1..21: mol_type = unassigned DNA
acacctctccgtcgtatcaag

SEQ ID NO: 413 - DNA, 21 bp, Zea mays;
  source 1..21: mol_type = unassigned DNA
tcattgtaatccatattacgt

SEQ ID NO: 414 - DNA, 20 bp, Zea mays;
  source 1..20: mol_type = unassigned DNA
cattgtaatccatactacgt

SEQ ID NO: 415 - DNA, 21 bp, Zea mays;
  source 1..21: mol_type = unassigned DNA
gccaacagttcactcccagta

SEQ ID NO: 416 - DNA, 25 bp, Zea mays;
  source 1..25: mol_type = unassigned DNA
acttgttacctttccttgctagaca

SEQ ID NO: 417 - DNA, 21 bp, Zea mays;
  source 1..21: mol_type = unassigned DNA
ttactggtacttagatatatg

SEQ ID NO: 418 - DNA, 20 bp, Zea mays;
  source 1..20: mol_type = unassigned DNA
tactggtacttagatagatg

SEQ ID NO: 419 - DNA, 21 bp, Zea mays;
  source 1..21: mol_type = unassigned DNA
agatacatgaagtaacatgct

SEQ ID NO: 420 - DNA, 21 bp, Zea mays;
  source 1..21: mol_type = unassigned DNA
ggtactcaagaacaattaacc

SEQ ID NO: 421 - DNA, 18 bp, Zea mays;
  source 1..18: mol_type = unassigned DNA
tcaaagaatctccggtca

SEQ ID NO: 422 - DNA, 17 bp, Zea mays;
  source 1..17: mol_type = unassigned DNA
caaagaatccccggtca

SEQ ID NO: 423 - DNA, 20 bp, Zea mays;
  source 1..20: mol_type = unassigned DNA
ggactgtgcgtagtatgagc

SEQ ID NO: 424 - DNA, 22 bp, Zea mays;
  source 1..22: mol_type = unassigned DNA
gtcacgtctatcctccagttca

SEQ ID NO: 425 - DNA, 14 bp, Zea mays;
  source 1..14: mol_type = unassigned DNA
accccgacactgct

SEQ ID NO: 426 - DNA, 14 bp, Zea mays;
  source 1..14: mol_type = unassigned DNA
caccccaacactgc

SEQ ID NO: 427 - DNA, 17 bp, Zea mays;
  source 1..17: mol_type = unassigned DNA
gtcgacgacggtgaagc

SEQ ID NO: 428 - DNA, 18 bp, Zea mays;
  source 1..18: mol_type = unassigned DNA
cacgctcgaggtgatcca

SEQ ID NO: 429 - DNA, 21 bp, Zea mays;
  source 1..21: mol_type = unassigned DNA
aagttatcttccattgtagtg

SEQ ID NO: 430 - DNA, 18 bp, Zea mays;
  source 1..18: mol_type = unassigned DNA
agttatcttccattgcag

SEQ ID NO: 431 - DNA, 20 bp, Zea mays;
  source 1..20: mol_type = unassigned DNA
catgtttattttgagagcca

SEQ ID NO: 432 - DNA, 17 bp, Zea mays;
  source 1..17: mol_type = unassigned DNA
gaaacgtgttgctgaag

SEQ ID NO: 433 - DNA, 14 bp, Zea mays;
  source 1..14: mol_type = unassigned DNA
cgacagccttcgat

SEQ ID NO: 434 - DNA, 14 bp, Zea mays;
  source 1..14: mol_type = unassigned DNA
cgacagccttcaat

SEQ ID NO: 435 - DNA, 17 bp, Zea mays;
  source 1..17: mol_type = unassigned DNA
ctagccgaactgtccta

SEQ ID NO: 436 - DNA, 17 bp, Zea mays;
  source 1..17: mol_type = unassigned DNA
cacaccaacggatcaag

SEQ ID NO: 437 - DNA, 17 bp, Zea mays;
  source 1..17: mol_type = unassigned DNA
cggtgacgaatactgat

SEQ ID NO: 438 - DNA, 17 bp, Zea mays;
  source 1..17: mol_type = unassigned DNA
cggtgacgaatactgac

SEQ ID NO: 439 - DNA, 19 bp, Zea mays;
  source 1..19: mol_type = unassigned DNA
gaaacatcccaacaacatc

SEQ ID NO: 440 - DNA, 16 bp, Zea mays;
  source 1..16: mol_type = unassigned DNA
agccttgctagtgctg

SEQ ID NO: 441 - DNA, 20 bp, Zea mays;
  source 1..20: mol_type = unassigned DNA
catcagagggaatataattt

SEQ ID NO: 442 - DNA, 19 bp, Zea mays;
  source 1..19: mol_type = unassigned DNA
catcagagggaatagaatt

SEQ ID NO: 443 - DNA, 23 bp, Zea mays;
  source 1..23: mol_type = unassigned DNA
agctatattttagagaccgtgtt

SEQ ID NO: 444 - DNA, 15 bp, Zea mays;
  source 1..15: mol_type = unassigned DNA
gcacgatgacgatga

SEQ ID NO: 445 - DNA, 19 bp, Zea mays;
  source 1..19: mol_type = unassigned DNA
cggtaacatgtagaatgca

SEQ ID NO: 446 - DNA, 18 bp, Zea mays;
  source 1..18: mol_type = unassigned DNA
cggtaacatgtagaacgc

SEQ ID NO: 447 - DNA, 22 bp, Zea mays;
  source 1..22: mol_type = unassigned DNA
tgaatgctctcagatgccacat

SEQ ID NO: 448 - DNA, 22 bp, Zea mays;
  source 1..22: mol_type = unassigned DNA
agcagcttcaagaaacaaagga

SEQ ID NO: 449 - DNA, 14 bp, Zea mays;
  source 1..14: mol_type = unassigned DNA
actgcgcgttgcaa

SEQ ID NO: 450 - DNA, 16 bp, Zea mays;
  source 1..16: mol_type = unassigned DNA
ctactgcgcattgcaa

SEQ ID NO: 451 - DNA, 15 bp, Zea mays;
  source 1..15: mol_type = unassigned DNA
ggccgccaaggtgct

SEQ ID NO: 452 - DNA, 20 bp, Zea mays;
  source 1..20: mol_type = unassigned DNA
gcctggtcgatcctgatgac

SEQ ID NO: 453 - DNA, 15 bp, Zea mays;
  source 1..15: mol_type = unassigned DNA
catgggccgtgacct

SEQ ID NO: 454 - DNA, 14 bp, Zea mays;
  source 1..14: mol_type = unassigned DNA
atgggccgcgacct

SEQ ID NO: 455 - DNA, 24 bp, Zea mays;
  source 1..24: mol_type = unassigned DNA
cctttaacaggttgtactcatgcc

SEQ ID NO: 456 - DNA, 18 bp, Zea mays;
  source 1..18: mol_type = unassigned DNA
tcgagtcagcacggttcg

SEQ ID NO: 457 - DNA, 15 bp, Zea mays;
  source 1..15: mol_type = unassigned DNA
caacctcacgaacct

SEQ ID NO: 458 - DNA, 15 bp, Zea mays;
  source 1..15: mol_type = unassigned DNA
cggcaacctcacaaa

SEQ ID NO: 459 - DNA, 21 bp, Zea mays;
  source 1..21: mol_type = unassigned DNA
caacctgagcttcaacagcct

SEQ ID NO: 460 - DNA, 15 bp, Zea mays;
  source 1..15: mol_type = unassigned DNA
ggcggttgctggaca

SEQ ID NO: 461 - DNA, 17 bp, Zea mays;
  source 1..17: mol_type = unassigned DNA
attctcaaagccgtaga

SEQ ID NO: 462 - DNA, 19 bp, Zea mays;
  source 1..19: mol_type = unassigned DNA
agattctcaaaaccgtaga

SEQ ID NO: 463 - DNA, 20 bp, Zea mays;
  source 1..20: mol_type = unassigned DNA
ggcagtttccgatgtccaga

SEQ ID NO: 464 - DNA, 20 bp, Zea mays;
  source 1..20: mol_type = unassigned DNA
gaacctgaccacgcttcttc

SEQ ID NO: 465 - DNA, 17 bp, Zea mays;
  source 1..17: mol_type = unassigned DNA
cacacaccgagagagag

SEQ ID NO: 466 - DNA, 16 bp, Zea mays;
  source 1..16: mol_type = unassigned DNA
ccacacaccgagaaag

SEQ ID NO: 467 - DNA, 20 bp, Zea mays;
  source 1..20: mol_type = unassigned DNA
agcacacgttctcttccaaa

SEQ ID NO: 468 - DNA, 21 bp, Zea mays;
  source 1..21: mol_type = unassigned DNA
cgggttcatcctcttcgtggt

SEQ ID NO: 469 - DNA, 15 bp, Zea mays;
  source 1..15: mol_type = unassigned DNA
ctgaagctgcctcaa

SEQ ID NO: 470 - DNA, 13 bp, Zea mays;
  source 1..13: mol_type = unassigned DNA
tgaagctgcccca

SEQ ID NO: 471 - DNA, 23 bp, Zea mays;
  source 1..23: mol_type = unassigned DNA
agcaaataaatttagatggaaca

SEQ ID NO: 472 - DNA, 20 bp, Zea mays;
  source 1..20: mol_type = unassigned DNA
gtcaaggtgaatatgtccta

SEQ ID NO: 473 - DNA, 16 bp, Zea mays;
  source 1..16: mol_type = unassigned DNA
agccagaaaacgggca

SEQ ID NO: 474 - DNA, 19 bp, Zea mays;
  source 1..19: mol_type = unassigned DNA
acaagccagaaaacggaca

SEQ ID NO: 475 - DNA, 18 bp, Zea mays;
  source 1..18: mol_type = unassigned DNA
gcgcgtacctgattcaca

SEQ ID NO: 476 - DNA, 22 bp, Zea mays;
  source 1..22: mol_type = unassigned DNA
agccagcagctgaagagaagac

SEQ ID NO: 477 - DNA, 14 bp, Zea mays;
  source 1..14: mol_type = unassigned DNA
ccgccaggtccgat

SEQ ID NO: 478 - DNA, 14 bp, Zea mays;
  source 1..14: mol_type = unassigned DNA
cgccacgtccgatg

SEQ ID NO: 479 - DNA, 16 bp, Zea mays;
  source 1..16: mol_type = unassigned DNA
tgggcagcctcaccgt

SEQ ID NO: 480 - DNA, 19 bp, Zea mays;
  source 1..19: mol_type = unassigned DNA
cggagctggaaaggatgga

SEQ ID NO: 481 - DNA, 21 bp, Zea mays;
  source 1..21: mol_type = unassigned DNA
caatagtgaatattgtagttt

SEQ ID NO: 482 - DNA, 21 bp, Zea mays;
  source 1..21: mol_type = unassigned DNA
caatagtgaatattgtaattt

SEQ ID NO: 483 - DNA, 24 bp, Zea mays;
  source 1..24: mol_type = unassigned DNA
agcagaaaaacattgggactgtac

SEQ ID NO: 484 - DNA, 21 bp, Zea mays;
  source 1..21: mol_type = unassigned DNA
agcctgaagctgtggatcttc

SEQ ID NO: 485 - DNA, 14 bp, Zea mays;
  source 1..14: mol_type = unassigned DNA
ctcaccgtggaccg

SEQ ID NO: 486 - DNA, 15 bp, Zea mays;
  source 1..15: mol_type = unassigned DNA
cctcacagtggaccg

SEQ ID NO: 487 - DNA, 19 bp, Zea mays;
  source 1..19: mol_type = unassigned DNA
catccgcaaggtcctgctc

SEQ ID NO: 488 - DNA, 21 bp, Zea mays;
  source 1..21: mol_type = unassigned DNA
gggcgatcgagttgtgctttg

SEQ ID NO: 489 - DNA, 21 bp, Zea mays;
  source 1..21: mol_type = unassigned DNA
cctaaacagatgtattatata

SEQ ID NO: 490 - DNA, 19 bp, Zea mays;
  source 1..19: mol_type = unassigned DNA
cctaaacagatgtactata

SEQ ID NO: 491 - DNA, 21 bp, Zea mays;
  source 1..21: mol_type = unassigned DNA
agttgtgccaagggctagttg

SEQ ID NO: 492 - DNA, 26 bp, Zea mays;
  source 1..26: mol_type = unassigned DNA
ggagtcatgcacatttgagaagaaac

SEQ ID NO: 493 - DNA, 14 bp, Zea mays;
  source 1..14: mol_type = unassigned DNA
aatggcaccattag

SEQ ID NO: 494 - DNA, 15 bp, Zea mays;
  source 1..15: mol_type = unassigned DNA
taatggcaccatcag

SEQ ID NO: 495 - DNA, 20 bp, Zea mays;
  source 1..20: mol_type = unassigned DNA
tggttgcttcggaagagttc

SEQ ID NO: 496 - DNA, 20 bp, Zea mays;
  source 1..20: mol_type = unassigned DNA
agggttgcgctcctagttct

SEQ ID NO: 497 - DNA, 20 bp, Zea mays;
  source 1..20: mol_type = unassigned DNA
cctaaagaaaggtgtagcct

SEQ ID NO: 498 - DNA, 22 bp, Zea mays;
  source 1..22: mol_type = unassigned DNA
ttcctaaagaaaggtatagcct

SEQ ID NO: 499 - DNA, 24 bp, Zea mays;
  source 1..24: mol_type = unassigned DNA
caagaccaggtctaacagagcata

SEQ ID NO: 500 - DNA, 25 bp, Zea mays;
  source 1..25: mol_type = unassigned DNA
ggacccgtaaattatcattgcttca

SEQ ID NO: 501 - DNA, 19 bp, Zea mays;
  source 1..19: mol_type = unassigned DNA
acgtctaagagattaaaag

SEQ ID NO: 502 - DNA, 21 bp, Zea mays;
  source 1..21: mol_type = unassigned DNA
aaatacgtctaagagataaaa

SEQ ID NO: 503 - DNA, 23 bp, Zea mays;
  source 1..23: mol_type = unassigned DNA
gtctgcaaataaattatcttggt

SEQ ID NO: 504 - DNA, 18 bp, Zea mays;
  source 1..18: mol_type = unassigned DNA
gacacaagatggtctcaa

SEQ ID NO: 505 - DNA, 19 bp, Zea mays;
  source 1..19: mol_type = unassigned DNA
ctgggagtcaatttcattg

SEQ ID NO: 506 - DNA, 19 bp, Zea mays;
  source 1..19: mol_type = unassigned DNA
ctgggagtcaattccattg

SEQ ID NO: 507 - DNA, 22 bp, Zea mays;
  source 1..22: mol_type = unassigned DNA
tggccggtaaacaaacaaagtc

SEQ ID NO: 508 - DNA, 20 bp, Zea mays;
  source 1..20: mol_type = unassigned DNA
tcagtgggtgatccggtaac

SEQ ID NO: 509 - DNA, 15 bp, Zea mays;
  source 1..15: mol_type = unassigned DNA
ctgcaggtgaagacc

SEQ ID NO: 510 - DNA, 15 bp, Zea mays;
  source 1..15: mol_type = unassigned DNA
ctgcaggtgaaaacc

SEQ ID NO: 511 - DNA, 16 bp, Zea mays;
  source 1..16: mol_type = unassigned DNA
gggcgcagccgtgtag

SEQ ID NO: 512 - DNA, 21 bp, Zea mays;
  source 1..21: mol_type = unassigned DNA
cacgactccatcaggcactct

SEQ ID NO: 513 - DNA, 17 bp, Zea mays;
  source 1..17: mol_type = unassigned DNA
agcaagagaagcagctg

SEQ ID NO: 514 - DNA, 18 bp, Zea mays;
  source 1..18: mol_type = unassigned DNA
tgagcaagagaagcaact

SEQ ID NO: 515 - DNA, 18 bp, Zea mays;
  source 1..18: mol_type = unassigned DNA
gtagtagcctcagtagga

SEQ ID NO: 516 - DNA, 23 bp, Zea mays;
  source 1..23: mol_type = unassigned DNA
tttgatagtttcatgatagatac

SEQ ID NO: 517 - DNA, 16 bp, Zea mays;
  source 1..16: mol_type = unassigned DNA
cgcgtatctcgattcc

SEQ ID NO: 518 - DNA, 17 bp, Zea mays;
  source 1..17: mol_type = unassigned DNA
cgcgtatctcaattcca

SEQ ID NO: 519 - DNA, 22 bp, Zea mays;
  source 1..22: mol_type = unassigned DNA
cattacaaacgcagccaaggta

SEQ ID NO: 520 - DNA, 17 bp, Zea mays;
  source 1..17: mol_type = unassigned DNA
gcgcccatctccagcaa

SEQ ID NO: 521 - DNA, 22 bp, Zea mays;
  source 1..22: mol_type = unassigned DNA
tacaacaaaggtcaataagtaa

SEQ ID NO: 522 - DNA, 20 bp, Zea mays;
  source 1..20: mol_type = unassigned DNA
caacaaaggtcaacaagtaa

SEQ ID NO: 523 - DNA, 24 bp, Zea mays;
  source 1..24: mol_type = unassigned DNA
gcaagtggagagaagaactaagga

SEQ ID NO: 524 - DNA, 21 bp, Zea mays;
  source 1..21: mol_type = unassigned DNA
cctgggcatatcagtggtgtt

SEQ ID NO: 525 - DNA, 18 bp, Zea mays;
  source 1..18: mol_type = unassigned DNA
ttcagcagtacttgacgt

SEQ ID NO: 526 - DNA, 16 bp, Zea mays;
  source 1..16: mol_type = unassigned DNA
tcagcagtacctgacg

SEQ ID NO: 527 - DNA, 22 bp, Zea mays;
  source 1..22: mol_type = unassigned DNA
ccgcaggaaatcaaacatgggt

SEQ ID NO: 528 - DNA, 20 bp, Zea mays;
  source 1..20: mol_type = unassigned DNA
acgtggtctccgtcgatgag

SEQ ID NO: 529 - DNA, 15 bp, Zea mays;
  source 1..15: mol_type = unassigned DNA
cgaggcgatggtgcc

SEQ ID NO: 530 - DNA, 14 bp, Zea mays;
  source 1..14: mol_type = unassigned DNA
aggcgacggtgcca

SEQ ID NO: 531 - DNA, 17 bp, Zea mays;
  source 1..17: mol_type = unassigned DNA
gacgtcaggtccagggt

SEQ ID NO: 532 - DNA, 24 bp, Zea mays;
  source 1..24: mol_type = unassigned DNA
agcctcatctcctacacttactac

SEQ ID NO: 533 - DNA, 18 bp, Zea mays;
  source 1..18: mol_type = unassigned DNA
tcagtattagtaaggtgc

SEQ ID NO: 534 - DNA, 21 bp, Zea mays;
  source 1..21: mol_type = unassigned DNA
aaatcagtattagtaagatgc

SEQ ID NO: 535 - DNA, 24 bp, Zea mays;
  source 1..24: mol_type = unassigned DNA
gatgtagttaacaagcgagcgtct

SEQ ID NO: 536 - DNA, 21 bp, Zea mays;
  source 1..21: mol_type = unassigned DNA
gcctgcactctttatgcttca

SEQ ID NO: 537 - DNA, 16 bp, Zea mays;
  source 1..16: mol_type = unassigned DNA
agccggttcgggtact

SEQ ID NO: 538 - DNA, 16 bp, Zea mays;
  source 1..16: mol_type = unassigned DNA
agccggttccggtact

SEQ ID NO: 539 - DNA, 16 bp, Zea mays;
  source 1..16: mol_type = unassigned DNA
cgtcgggcctgtgctg

SEQ ID NO: 540 - DNA, 18 bp, Zea mays;
  source 1..18: mol_type = unassigned DNA
cacggacgcgttgttggt

SEQ ID NO: 541 - DNA, 19 bp, Zea mays;
  source 1..19: mol_type = unassigned DNA
cagatccgatctctgttag

SEQ ID NO: 542 - DNA, 19 bp, Zea mays;
  source 1..19: mol_type = unassigned DNA
agatccgatcgctgttagt

SEQ ID NO: 543 - DNA, 22 bp, Zea mays;
  source 1..22: mol_type = unassigned DNA
gggaggatacatcccttcatca

SEQ ID NO: 544 - DNA, 21 bp, Zea mays;
  source 1..21: mol_type = unassigned DNA
aacaacgactgtgagggttca

SEQ ID NO: 545 - DNA, 18 bp, Zea mays;
  source 1..18: mol_type = unassigned DNA
cagccatagtgtgtggaa

SEQ ID NO: 546 - DNA, 18 bp, Zea mays;
  source 1..18: mol_type = unassigned DNA
agccatagtgcgtggaaa

SEQ ID NO: 547 - DNA, 16 bp, Zea mays;
  source 1..16: mol_type = unassigned DNA
gggcactgctggcgtt

SEQ ID NO: 548 - DNA, 21 bp, Zea mays;
  source 1..21: mol_type = unassigned DNA
ccctcacctatgcaacagaac

SEQ ID NO: 549 - DNA, 19 bp, Zea mays;
  source 1..19: mol_type = unassigned DNA
tggctacactttaatcgaa

SEQ ID NO: 550 - DNA, 17 bp, Zea mays;
  source 1..17: mol_type = unassigned DNA
tggctacacttcaatcg

SEQ ID NO: 551 - DNA, 23 bp, Zea mays;
  source 1..23: mol_type = unassigned DNA
gacagctctcatcactgcatcag

SEQ ID NO: 552 - DNA, 22 bp, Zea mays;
  source 1..22: mol_type = unassigned DNA
gcactgctttcagagttctggt

SEQ ID NO: 553 - DNA, 21 bp, Zea mays;
  source 1..21: mol_type = unassigned DNA
aaaggtttgttttatttattg

SEQ ID NO: 554 - DNA, 21 bp, Zea mays;
  source 1..21: mol_type = unassigned DNA
taaaggtttgttttatttatc

SEQ ID NO: 555 - DNA, 21 bp, Zea mays;
  source 1..21: mol_type = unassigned DNA
cacgtcaggaaaggatgcaaa

SEQ ID NO: 556 - DNA, 22 bp, Zea mays;
  source 1..22: mol_type = unassigned DNA
gcggatcatcactcccatcttc

SEQ ID NO: 557 - DNA, 17 bp, Zea mays;
  source 1..17: mol_type = unassigned DNA
cagccatcttgctgata

SEQ ID NO: 558 - DNA, 16 bp, Zea mays;
  source 1..16: mol_type = unassigned DNA
cagccatcgtgctgat

SEQ ID NO: 559 - DNA, 24 bp, Zea mays;
  source 1..24: mol_type = unassigned DNA
cgtgtcgttgaaatatgcatggtt

SEQ ID NO: 560 - DNA, 22 bp, Zea mays;
  source 1..22: mol_type = unassigned DNA
tcacggtcctccatcatctaac

SEQ ID NO: 561 - DNA, 21 bp, Zea mays;
  source 1..21: mol_type = unassigned DNA
ctaaaagtgactaactaaagt

SEQ ID NO: 562 - DNA, 22 bp, Zea mays;
  source 1..22: mol_type = unassigned DNA
ctaaaagtgactaactaaaatt

SEQ ID NO: 563 - DNA, 22 bp, Zea mays;
  source 1..22: mol_type = unassigned DNA
gtcactctcttaaactctagtc

SEQ ID NO: 564 - DNA, 21 bp, Zea mays;
  source 1..21: mol_type = unassigned DNA
gctatcgcattgtactagtag

SEQ ID NO: 565 - DNA, 18 bp, Zea mays;
  source 1..18: mol_type = unassigned DNA
tcataagctgtctccaaa

SEQ ID NO: 566 - DNA, 19 bp, Zea mays;
  source 1..19: mol_type = unassigned DNA
ttcataagctgactccaaa

SEQ ID NO: 567 - DNA, 24 bp, Zea mays;
  source 1..24: mol_type = unassigned DNA
tgtgggtgtttgattcaatggatg

SEQ ID NO: 568 - DNA, 19 bp, Zea mays;
  source 1..19: mol_type = unassigned DNA
tccaaggctcagctcgaaa

SEQ ID NO: 569 - DNA, 19 bp, Zea mays;
  source 1..19: mol_type = unassigned DNA
catcgatgtacttcaaaag

SEQ ID NO: 570 - DNA, 19 bp, Zea mays;
  source 1..19: mol_type = unassigned DNA
catcgatgtacttcaaaaa

SEQ ID NO: 571 - DNA, 26 bp, Zea mays;
  source 1..26: mol_type = unassigned DNA
gcccaagtgatccagaactaatacac

SEQ ID NO: 572 - DNA, 26 bp, Zea mays;
  source 1..26: mol_type = unassigned DNA
tgcagttcatttttgcactatttgac

SEQ ID NO: 573 - DNA, 16 bp, Zea mays;
  source 1..16: mol_type = unassigned DNA
tggtggcagtttaggt

SEQ ID NO: 574 - DNA, 15 bp, Zea mays;
  source 1..15: mol_type = unassigned DNA
tggtggcagttcagg

SEQ ID NO: 575 - DNA, 24 bp, Zea mays;
  source 1..24: mol_type = unassigned DNA
ccttgaggcttggtttagattggt

SEQ ID NO: 576 - DNA, 24 bp, Zea mays;
  source 1..24: mol_type = unassigned DNA
ctcacccacatctttcgcactatt

SEQ ID NO: 577 - DNA, 16 bp, Zea mays;
  source 1..16: mol_type = unassigned DNA
ttaaacgctttgttga

SEQ ID NO: 578 - DNA, 15 bp, Zea mays;
  source 1..15: mol_type = unassigned DNA
aaacgctttgctgat

SEQ ID NO: 579 - DNA, 18 bp, Zea mays;
  source 1..18: mol_type = unassigned DNA
tggaactcttcagtcttg

SEQ ID NO: 580 - DNA, 16 bp, Zea mays;
  source 1..16: mol_type = unassigned DNA
gaacggtgttctaggg

SEQ ID NO: 581 - DNA, 18 bp, Zea mays;
  source 1..18: mol_type = unassigned DNA
tgatgtccatattgaagc

SEQ ID NO: 582 - DNA, 19 bp, Zea mays;
  source 1..19: mol_type = unassigned DNA
ttgatgtccatatagaagc

SEQ ID NO: 583 - DNA, 24 bp, Zea mays;
  source 1..24: mol_type = unassigned DNA
tgaagtgttagaagaagttgcaca

SEQ ID NO: 584 - DNA, 18 bp, Zea mays;
  source 1..18: mol_type = unassigned DNA
aagcacccttgaggcagt

SEQ ID NO: 585 - DNA, 14 bp, Zea mays;
  source 1..14: mol_type = unassigned DNA
cggctgggcgactt

SEQ ID NO: 586 - DNA, 14 bp, Zea mays;
  source 1..14: mol_type = unassigned DNA
cggctcggcgactt

SEQ ID NO: 587 - DNA, 20 bp, Zea mays;
  source 1..20: mol_type = unassigned DNA
tcatgctggactcgtcgttc

SEQ ID NO: 588 - DNA, 21 bp, Zea mays;
  source 1..21: mol_type = unassigned DNA
gtccgtgtaggaggtcttgtc

SEQ ID NO: 589 - DNA, 17 bp, Zea mays;
  source 1..17: mol_type = unassigned DNA
cagtagctgtgatagac

SEQ ID NO: 590 - DNA, 16 bp, Zea mays;
  source 1..16: mol_type = unassigned DNA
cagtagctgtgacaga

SEQ ID NO: 591 - DNA, 19 bp, Zea mays;
  source 1..19: mol_type = unassigned DNA
ttgcaaggaaaatggaaga

SEQ ID NO: 592 - DNA, 16 bp, Zea mays;
  source 1..16: mol_type = unassigned DNA
atcgtgatgggctgct

SEQ ID NO: 593 - DNA, 19 bp, Zea mays;
  source 1..19: mol_type = unassigned DNA
catgttagtttacccgaaa

SEQ ID NO: 594 - DNA, 19 bp, Zea mays;
  source 1..19: mol_type = unassigned DNA
agcatgttagtttaccaga

SEQ ID NO: 595 - DNA, 22 bp, Zea mays;
  source 1..22: mol_type = unassigned DNA
tgtgccagtgttatccaaggaa

SEQ ID NO: 596 - DNA, 21 bp, Zea mays;
  source 1..21: mol_type = unassigned DNA
tccatgcttcagtcacacagt

SEQ ID NO: 597 - DNA, 20 bp, Zea mays;
  source 1..20: mol_type = unassigned DNA
aagagtcaacactggagttg

SEQ ID NO: 598 - DNA, 23 bp, Zea mays;
  source 1..23: mol_type = unassigned DNA
agggaagagtcaacactagagtt

SEQ ID NO: 599 - DNA, 22 bp, Zea mays;
  source 1..22: mol_type = unassigned DNA
ccatgaaggcagagagcatgtg

SEQ ID NO: 600 - DNA, 20 bp, Zea mays;
  source 1..20: mol_type = unassigned DNA
tctcggttgtgtggatggaa

SEQ ID NO: 601 - DNA, 15 bp, Zea mays;
  source 1..15: mol_type = unassigned DNA
tactccctccgtttt

SEQ ID NO: 602 - DNA, 14 bp, Zea mays;
  source 1..14: mol_type = unassigned DNA
actccctccgtttc

SEQ ID NO: 603 - DNA, 21 bp, Zea mays;
  source 1..21: mol_type = unassigned DNA
ggtcgaggagagtgaaccttg

SEQ ID NO: 604 - DNA, 21 bp, Zea mays;
  source 1..21: mol_type = unassigned DNA
ggcagattgccaggatgagat

SEQ ID NO: 605 - DNA, 22 bp, Zea mays;
  source 1..22: mol_type = unassigned DNA
attctctattatagaaagaaat

SEQ ID NO: 606 - DNA, 22 bp, Zea mays;
  source 1..22: mol_type = unassigned DNA
attctctattatagaaagaaac

SEQ ID NO: 607 - DNA, 27 bp, Zea mays;
  source 1..27: mol_type = unassigned DNA
ggtagcagatgaagttccaatagtaaa

SEQ ID NO: 608 - DNA, 24 bp, Zea mays;
  source 1..24: mol_type = unassigned DNA
gctatctagccacttgttccattc

SEQ ID NO: 609 - DNA, 17 bp, Zea mays;
  source 1..17: mol_type = unassigned DNA
cacaacgtggaagtagg

SEQ ID NO: 610 - DNA, 18 bp, Zea mays;
  source 1..18: mol_type = unassigned DNA
ccacaacgtggaagtaga

SEQ ID NO: 611 - DNA, 23 bp, Zea mays;
  source 1..23: mol_type = unassigned DNA
gatcatcggatcacttgaaaggg

SEQ ID NO: 612 - DNA, 19 bp, Zea mays;
  source 1..19: mol_type = unassigned DNA
tggttcggccaagtaacac

SEQ ID NO: 613 - DNA, 13 bp, Zea mays;
  source 1..13: mol_type = unassigned DNA
accgctgctgcca

SEQ ID NO: 614 - DNA, 14 bp, Zea mays;
  source 1..14: mol_type = unassigned DNA
aagaccgccgctgc

SEQ ID NO: 615 - DNA, 17 bp, Zea mays;
  source 1..17: mol_type = unassigned DNA
tcctgctcggcctgtga

SEQ ID NO: 616 - DNA, 19 bp, Zea mays;
  source 1..19: mol_type = unassigned DNA
gcgccaagcaaatgtcgta

SEQ ID NO: 617 - DNA, 16 bp, Zea mays;
  source 1..16: mol_type = unassigned DNA
cgcggaaccttggatg

SEQ ID NO: 618 - DNA, 16 bp, Zea mays;
  source 1..16: mol_type = unassigned DNA
cgcggaagccttggat

SEQ ID NO: 619 - DNA, 18 bp, Zea mays;
  source 1..18: mol_type = unassigned DNA
aagaccgtcgcggactcg

SEQ ID NO: 620 - DNA, 21 bp, Zea mays;
  source 1..21: mol_type = unassigned DNA
gggcaaactcatgcgtagatg

SEQ ID NO: 621 - DNA, 17 bp, Zea mays;
  source 1..17: mol_type = unassigned DNA
atcaaccatctgtccat

SEQ ID NO: 622 - DNA, 15 bp, Zea mays;
  source 1..15: mol_type = unassigned DNA
caaccatctgcccat

SEQ ID NO: 623 - DNA, 18 bp, Zea mays;
  source 1..18: mol_type = unassigned DNA
cttcctaaactcgtccct

SEQ ID NO: 624 - DNA, 24 bp, Zea mays;
  source 1..24: mol_type = unassigned DNA
tcaaatctaagttattgagtgtta

SEQ ID NO: 625 - DNA, 20 bp, Zea mays;
  source 1..20: mol_type = unassigned DNA
tgatagtcagtagtatggtt

SEQ ID NO: 626 - DNA, 18 bp, Zea mays;
  source 1..18: mol_type = unassigned DNA
agtcagtagtatggcttg

SEQ ID NO: 627 - DNA, 24 bp, Zea mays;
  source 1..24: mol_type = unassigned DNA
ggtcaattggtagtcagaggacaa

SEQ ID NO: 628 - DNA, 21 bp, Zea mays;
  source 1..21: mol_type = unassigned DNA
gtgctccaacgaggactagtg

SEQ ID NO: 629 - DNA, 16 bp, Zea mays;
  source 1..16: mol_type = unassigned DNA
acccaagggctcaaca

SEQ ID NO: 630 - DNA, 16 bp, Zea mays;
  source 1..16: mol_type = unassigned DNA
cacccaagagctcaac

SEQ ID NO: 631 - DNA, 19 bp, Zea mays;
  source 1..19: mol_type = unassigned DNA
acagctcaaagggcaggtt

SEQ ID NO: 632 - DNA, 22 bp, Zea mays;
  source 1..22: mol_type = unassigned DNA
ggcttgaacagtgccaatagtc

SEQ ID NO: 633 - DNA, 19 bp, Zea mays;
  source 1..19: mol_type = unassigned DNA
attgcgtctcgataaatca

SEQ ID NO: 634 - DNA, 18 bp, Zea mays;
  source 1..18: mol_type = unassigned DNA
ttgcgtctcaataaatca

SEQ ID NO: 635 - DNA, 17 bp, Zea mays;
  source 1..17: mol_type = unassigned DNA
tccgagttcgctgtcca

SEQ ID NO: 636 - DNA, 23 bp, Zea mays;
  source 1..23: mol_type = unassigned DNA
cgttggcattgaagggaagtcta

SEQ ID NO: 637 - DNA, 15 bp, Zea mays;
  source 1..15: mol_type = unassigned DNA
attggcaatgccgca

SEQ ID NO: 638 - DNA, 16 bp, Zea mays;
  source 1..16: mol_type = unassigned DNA
cattggcaatgccaca

SEQ ID NO: 639 - DNA, 23 bp, Zea mays;
  source 1..23: mol_type = unassigned DNA
tgcctgatcttttccttcaccat

SEQ ID NO: 640 - DNA, 20 bp, Zea mays;
  source 1..20: mol_type = unassigned DNA
tgtaggccacctaggattgg

SEQ ID NO: 641 - DNA, 17 bp, Zea mays;
  source 1..17: mol_type = unassigned DNA
tttccattgtttccatc

SEQ ID NO: 642 - DNA, 18 bp, Zea mays;
  source 1..18: mol_type = unassigned DNA
agtttccattgtttccac

SEQ ID NO: 643 - DNA, 29 bp, Zea mays;
  source 1..29: mol_type = unassigned DNA
agttccttttctctactcctataaagcac

SEQ ID NO: 644 - DNA, 23 bp, Zea mays;
  source 1..23: mol_type = unassigned DNA
ggatgggatcatagccacagttc

SEQ ID NO: 645 - DNA, 14 bp, Zea mays;
  source 1..14: mol_type = unassigned DNA
cctccttgcgcgtg

SEQ ID NO: 646 - DNA, 13 bp, Zea mays;
  source 1..13: mol_type = unassigned DNA
ctcctcgcgcgtg

SEQ ID NO: 647 - DNA, 16 bp, Zea mays;
  source 1..16: mol_type = unassigned DNA
gcctgggaccgggaag

SEQ ID NO: 648 - DNA, 18 bp, Zea mays;
  source 1..18: mol_type = unassigned DNA
caccgacaccgacgaaga

SEQ ID NO: 649 - DNA, 19 bp, Zea mays;
  source 1..19: mol_type = unassigned DNA
tcacaaatcaataaagccc

SEQ ID NO: 650 - DNA, 19 bp, Zea mays;
  source 1..19: mol_type = unassigned DNA
ttcacaaatcaacaaagcc

SEQ ID NO: 651 - DNA, 22 bp, Zea mays;
  source 1..22: mol_type = unassigned DNA
atggtacaagtcacaggtaggg

SEQ ID NO: 652 - DNA, 22 bp, Zea mays;
  source 1..22: mol_type = unassigned DNA
gtcaagttagggccggatcata

SEQ ID NO: 653 - DNA, 22 bp, Zea mays;
  source 1..22: mol_type = unassigned DNA
agtatggaactaatttgacaaa

SEQ ID NO: 654 - DNA, 24 bp, Zea mays;
  source 1..24: mol_type = unassigned DNA
agagtatggaactaatttaacaaa

SEQ ID NO: 655 - DNA, 23 bp, Zea mays;
  source 1..23: mol_type = unassigned DNA
aaacagttggtgttggagttgga

SEQ ID NO: 656 - DNA, 19 bp, Zea mays;
  source 1..19: mol_type = unassigned DNA
tgtggatggcgtgttagca

SEQ ID NO: 657 - DNA, 20 bp, Zea mays;
  source 1..20: mol_type = unassigned DNA
tccattacttattgaaacac

SEQ ID NO: 658 - DNA, 19 bp, Zea mays;
  source 1..19: mol_type = unassigned DNA
ccattacttactgaaacac

SEQ ID NO: 659 - DNA, 21 bp, Zea mays;
  source 1..21: mol_type = unassigned DNA
accacctcggtctacacctta

SEQ ID NO: 660 - DNA, 21 bp, Zea mays;
  source 1..21: mol_type = unassigned DNA
tgccagaaagcatgggaagtc

SEQ ID NO: 661 - DNA, 15 bp, Zea mays;
  source 1..15: mol_type = unassigned DNA
taggcactgaccgga

SEQ ID NO: 662 - DNA, 15 bp, Zea mays;
  source 1..15: mol_type = unassigned DNA
taggcactgacccga

SEQ ID NO: 663 - DNA, 17 bp, Zea mays;
  source 1..17: mol_type = unassigned DNA
tggcgagacgaagcaga

SEQ ID NO: 664 - DNA, 20 bp, Zea mays;
  source 1..20: mol_type = unassigned DNA
gaccgaaccgaaccattagc

SEQ ID NO: 665 - DNA, 17 bp, Zea mays;
  source 1..17: mol_type = unassigned DNA
cttctgtgcatggatca

SEQ ID NO: 666 - DNA, 16 bp, Zea mays;
  source 1..16: mol_type = unassigned DNA
tctgtgcacggatcat

SEQ ID NO: 667 - DNA, 22 bp, Zea mays;
  source 1..22: mol_type = unassigned DNA
cgagaagttcccatcagctcaa

SEQ ID NO: 668 - DNA, 22 bp, Zea mays;
  source 1..22: mol_type = unassigned DNA
tggtgaacattggttgcttgtg

SEQ ID NO: 669 - DNA, 21 bp, Zea mays;
  source 1..21: mol_type = unassigned DNA
aaacaacagaatctttttaga

SEQ ID NO: 670 - DNA, 22 bp, Zea mays;
  source 1..22: mol_type = unassigned DNA
aaacaacagaatctttttaaaa

SEQ ID NO: 671 - DNA, 24 bp, Zea mays;
  source 1..24: mol_type = unassigned DNA
cagctctaaactcacagacgtttg

SEQ ID NO: 672 - DNA, 22 bp, Zea mays;
  source 1..22: mol_type = unassigned DNA
agcgctctaccatctgagctac

SEQ ID NO: 673 - DNA, 22 bp, Zea mays;
  source 1..22: mol_type = unassigned DNA
tcaaaataatgatatgagggaa

SEQ ID NO: 674 - DNA, 22 bp, Zea mays;
  source 1..22: mol_type = unassigned DNA
tcaaaataatgatatgaggaaa

SEQ ID NO: 675 - DNA, 25 bp, Zea mays;
  source 1..25: mol_type = unassigned DNA
aagactgaaagcatgaataaacggt

SEQ ID NO: 676 - DNA, 20 bp, Zea mays;
  source 1..20: mol_type = unassigned DNA
caggcgatcttgaccttggt

SEQ ID NO: 677 - DNA, 19 bp, Zea mays;
  source 1..19: mol_type = unassigned DNA
ctaaatttaagtgctgttg

SEQ ID NO: 678 - DNA, 22 bp, Zea mays;
  source 1..22: mol_type = unassigned DNA
aagatctaaatttaagtactgt

SEQ ID NO: 679 - DNA, 24 bp, Zea mays;
  source 1..24: mol_type = unassigned DNA
ttctggataaagcaatgaccaaca

SEQ ID NO: 680 - DNA, 22 bp, Zea mays;
  source 1..22: mol_type = unassigned DNA
gtgagtctgcttcctctccatt

SEQ ID NO: 681 - DNA, 18 bp, Zea mays;
  source 1..18: mol_type = unassigned DNA
tggttgctctgcatgtat

SEQ ID NO: 682 - DNA, 18 bp, Zea mays;
  source 1..18: mol_type = unassigned DNA
ttggttgctctgcatata

SEQ ID NO: 683 - DNA, 22 bp, Zea mays;
  source 1..22: mol_type = unassigned DNA
gcctttgcgaaggttttagcag

SEQ ID NO: 684 - DNA, 19 bp, Zea mays;
  source 1..19: mol_type = unassigned DNA
aactccgtggcagcatgtg

SEQ ID NO: 685 - DNA, 15 bp, Zea mays;
  source 1..15: mol_type = unassigned DNA
tgatctggggcatct

SEQ ID NO: 686 - DNA, 17 bp, Zea mays;
  source 1..17: mol_type = unassigned DNA
tgagtgatctgggacat

SEQ ID NO: 687 - DNA, 22 bp, Zea mays;
  source 1..22: mol_type = unassigned DNA
caccggtgccaaggatatagag

SEQ ID NO: 688 - DNA, 20 bp, Zea mays;
  source 1..20: mol_type = unassigned DNA
aggccgtctaacgaagtgtg

SEQ ID NO: 689 - DNA, 18 bp, Zea mays;
  source 1..18: mol_type = unassigned DNA
ttcatctatccactagaa

SEQ ID NO: 690 - DNA, 17 bp, Zea mays;
  source 1..17: mol_type = unassigned DNA
tcatctatccactacaa

SEQ ID NO: 691 - DNA, 22 bp, Zea mays;
  source 1..22: mol_type = unassigned DNA
gtatgtaaaacaaggttcaaaa

SEQ ID NO: 692 - DNA, 21 bp, Zea mays;
  source 1..21: mol_type = unassigned DNA
agggacaactatggatgaagt

SEQ ID NO: 693 - DNA, 17 bp, Zea mays;
  source 1..17: mol_type = unassigned DNA
ccgtcctagttaagtgc

SEQ ID NO: 694 - DNA, 17 bp, Zea mays;
  source 1..17: mol_type = unassigned DNA
tccgtcctagctaagtg

SEQ ID NO: 695 - DNA, 20 bp, Zea mays;
  source 1..20: mol_type = unassigned DNA
agtcggttctcttcgtctgc

SEQ ID NO: 696 - DNA, 23 bp, Zea mays;
  source 1..23: mol_type = unassigned DNA
cgcatgcccgtgatttatttctc

SEQ ID NO: 697 - DNA, 19 bp, Zea mays;
  source 1..19: mol_type = unassigned DNA
ctgagagaatggacacgaa

SEQ ID NO: 698 - DNA, 17 bp, Zea mays;
  source 1..17: mol_type = unassigned DNA
ctgagagaatgggcaca

SEQ ID NO: 699 - DNA, 20 bp, Zea mays;
  source 1..20: mol_type = unassigned DNA
gtgttactaggatacagtga

SEQ ID NO: 700 - DNA, 18 bp, Zea mays;
  source 1..18: mol_type = unassigned DNA
tgcccttacctgaagtct

SEQ ID NO: 701 - DNA, 15 bp, Zea mays;
  source 1..15: mol_type = unassigned DNA
tgctctgcttaccgt

SEQ ID NO: 702 - DNA, 14 bp, Zea mays;
  source 1..14: mol_type = unassigned DNA
tgctctgcctaccg

SEQ ID NO: 703 - DNA, 18 bp, Zea mays;
  source 1..18: mol_type = unassigned DNA
gtgagcaccagccacttc

SEQ ID NO: 704 - DNA, 19 bp, Zea mays;
  source 1..19: mol_type = unassigned DNA
gaacacgacggcattccaa

SEQ ID NO: 705 - DNA, 21 bp, Zea mays;
  source 1..21: mol_type = unassigned DNA
ataacacaagaatttgagcat

SEQ ID NO: 706 - DNA, 21 bp, Zea mays;
  source 1..21: mol_type = unassigned DNA
caataacacaagaatttaagc

SEQ ID NO: 707 - DNA, 18 bp, Zea mays;
  source 1..18: mol_type = unassigned DNA
cctgctacagatttcaac

SEQ ID NO: 708 - DNA, 19 bp, Zea mays;
  source 1..19: mol_type = unassigned DNA
ctgtttaggagccagatta

SEQ ID NO: 709 - DNA, 14 bp, Zea mays;
  source 1..14: mol_type = unassigned DNA
cgacgggagttggc

SEQ ID NO: 710 - DNA, 14 bp, Zea mays;
  source 1..14: mol_type = unassigned DNA
cgacgggagtaggc

SEQ ID NO: 711 - DNA, 15 bp, Zea mays;
  source 1..15: mol_type = unassigned DNA
agagccgggagccat

SEQ ID NO: 712 - DNA, 15 bp, Zea mays;
  source 1..15: mol_type = unassigned DNA
actcctccgccttgg

SEQ ID NO: 713 - DNA, 15 bp, Zea mays;
  source 1..15: mol_type = unassigned DNA
cggcgccttcttctg

SEQ ID NO: 714 - DNA, 14 bp, Zea mays;
  source 1..14: mol_type = unassigned DNA
cggcgcctccttct

SEQ ID NO: 715 - DNA, 23 bp, Zea mays;
  source 1..23: mol_type = unassigned DNA
gccgtgtccatcaaacttcatct

SEQ ID NO: 716 - DNA, 19 bp, Zea mays;
  source 1..19: mol_type = unassigned DNA
gggcttcttgcgcagagag

SEQ ID NO: 717 - DNA, 22 bp, Zea mays;
  source 1..22: mol_type = unassigned DNA
tattccaagaagtttatcttgt

SEQ ID NO: 718 - DNA, 19 bp, Zea mays;
  source 1..19: mol_type = unassigned DNA
tccaagaagtttaccttgt

SEQ ID NO: 719 - DNA, 18 bp, Zea mays;
  source 1..18: mol_type = unassigned DNA
agcacccagtcctccact

SEQ ID NO: 720 - DNA, 18 bp, Zea mays;
  source 1..18: mol_type = unassigned DNA
gctgcccaggatcgaact

SEQ ID NO: 721 - DNA, 19 bp, Zea mays;
  source 1..19: mol_type = unassigned DNA
ttccccagagaagggagtt

SEQ ID NO: 722 - DNA, 20 bp, Zea mays;
  source 1..20: mol_type = unassigned DNA
ttccccagagaaaggagtta

SEQ ID NO: 723 - DNA, 20 bp, Zea mays;
  source 1..20: mol_type = unassigned DNA
caggtagcttgccaaacgga

SEQ ID NO: 724 - DNA, 23 bp, Zea mays;
  source 1..23: mol_type = unassigned DNA
tgtctacacgaaggcaattgttg

SEQ ID NO: 725 - DNA, 14 bp, Zea mays;
  source 1..14: mol_type = unassigned DNA
tgttcgccgcagtc

SEQ ID NO: 726 - DNA, 15 bp, Zea mays;
  source 1..15: mol_type = unassigned DNA
tgttcgcagcagtcc

SEQ ID NO: 727 - DNA, 16 bp, Zea mays;
  source 1..16: mol_type = unassigned DNA
tgcccgggaagatcca

SEQ ID NO: 728 - DNA, 20 bp, Zea mays;
  source 1..20: mol_type = unassigned DNA
ttaaccctgaaggagacgga

SEQ ID NO: 729 - DNA, 18 bp, Zea mays;
  source 1..18: mol_type = unassigned DNA
acctccattcgcataaaa

SEQ ID NO: 730 - DNA, 20 bp, Zea mays;
  source 1..20: mol_type = unassigned DNA
atgacctccattcacataaa

SEQ ID NO: 731 - DNA, 22 bp, Zea mays;
  source 1..22: mol_type = unassigned DNA
ctggaacatgtcgaccattcac

SEQ ID NO: 732 - DNA, 21 bp, Zea mays;
  source 1..21: mol_type = unassigned DNA
ccctgaccacatgcatacaca

SEQ ID NO: 733 - DNA, 21 bp, Zea mays;
  source 1..21: mol_type = unassigned DNA
ctagtaaccaaatatgaatta

SEQ ID NO: 734 - DNA, 21 bp, Zea mays;
  source 1..21: mol_type = unassigned DNA
ctagtaaccaaatatgaaata

SEQ ID NO: 735 - DNA, 20 bp, Zea mays;
  source 1..20: mol_type = unassigned DNA
ctgttatgatacctggtctt

SEQ ID NO: 736 - DNA, 17 bp, Zea mays;
  source 1..17: mol_type = unassigned DNA
gactatgggcgtcttta

SEQ ID NO: 737 - DNA, 19 bp, Zea mays;
  source 1..19: mol_type = unassigned DNA
aggcccattttaggatttt

SEQ ID NO: 738 - DNA, 19 bp, Zea mays;
  source 1..19: mol_type = unassigned DNA
aggcccattttaggatatt

SEQ ID NO: 739 - DNA, 20 bp, Zea mays;
  source 1..20: mol_type = unassigned DNA
agagcagtcccaccttggtt

SEQ ID NO: 740 - DNA, 20 bp, Zea mays;
  source 1..20: mol_type = unassigned DNA
tgcttgaccggagtgagaag

SEQ ID NO: 741 - DNA, 20 bp, Zea mays;
  source 1..20: mol_type = unassigned DNA
aacaaataggagaatcagat

SEQ ID NO: 742 - DNA, 18 bp, Zea mays;
  source 1..18: mol_type = unassigned DNA
caaataggagaaccagat

SEQ ID NO: 743 - DNA, 23 bp, Zea mays;
  source 1..23: mol_type = unassigned DNA
ggtggtgcctgcatataagtaaa

SEQ ID NO: 744 - DNA, 20 bp, Zea mays;
  source 1..20: mol_type = unassigned DNA
atgtgccatgctgcactaag

SEQ ID NO: 745 - DNA, 19 bp, Zea mays;
  source 1..19: mol_type = unassigned DNA
tcgtaagatgggaatgtgg

SEQ ID NO: 746 - DNA, 21 bp, Zea mays;
  source 1..21: mol_type = unassigned DNA
tttcgtaagatgagaatgtgg

SEQ ID NO: 747 - DNA, 24 bp, Zea mays;
  source 1..24: mol_type = unassigned DNA
acctttggtgtgtgctatggtatg

SEQ ID NO: 748 - DNA, 20 bp, Zea mays;
  source 1..20: mol_type = unassigned DNA
accgtcccctgctcaaaacc

SEQ ID NO: 749 - DNA, 19 bp, Zea mays;
  source 1..19: mol_type = unassigned DNA
acatatttatagccctagg

SEQ ID NO: 750 - DNA, 19 bp, Zea mays;
  source 1..19: mol_type = unassigned DNA
acatatttatagcccaagg

SEQ ID NO: 751 - DNA, 25 bp, Zea mays;
  source 1..25: mol_type = unassigned DNA
caaacactacacaatgtcataccct

SEQ ID NO: 752 - DNA, 25 bp, Zea mays;
  source 1..25: mol_type = unassigned DNA
actgtcctctgtagtctctttagca

SEQ ID NO: 753 - DNA, 16 bp, Zea mays;
  source 1..16: mol_type = unassigned DNA
accagccctagtcatc

SEQ ID NO: 754 - DNA, 17 bp, Zea mays;
  source 1..17: mol_type = unassigned DNA
cagccctactcatcaaa

SEQ ID NO: 755 - DNA, 21 bp, Zea mays;
  source 1..21: mol_type = unassigned DNA
ttgtccacaacctcctactga

SEQ ID NO: 756 - DNA, 21 bp, Zea mays;
  source 1..21: mol_type = unassigned DNA
aaggctcaattgcaacccata

SEQ ID NO: 757 - DNA, 18 bp, Zea mays;
  source 1..18: mol_type = unassigned DNA
ccacctcgaatcagtata

SEQ ID NO: 758 - DNA, 18 bp, Zea mays;
  source 1..18: mol_type = unassigned DNA
ccacctcgaaacagtata

SEQ ID NO: 759 - DNA, 25 bp, Zea mays;
  source 1..25: mol_type = unassigned DNA
tctctattggctgagaacaattcac

SEQ ID NO: 760 - DNA, 21 bp, Zea mays;
  source 1..21: mol_type = unassigned DNA
tcgttggatcaatcgcaactc

SEQ ID NO: 761 - DNA, 19 bp, Zea mays;
  source 1..19: mol_type = unassigned DNA
ttggttgaactttagtatc

SEQ ID NO: 762 - DNA, 19 bp, Zea mays;
  source 1..19: mol_type = unassigned DNA
ttggttgaactttagaatc

SEQ ID NO: 763 - DNA, 20 bp, Zea mays;
  source 1..20: mol_type = unassigned DNA
ttgacactcattactgtttg

SEQ ID NO: 764 - DNA, 21 bp, Zea mays;
  source 1..21: mol_type = unassigned DNA
ggagaatgacttagaacttag

SEQ ID NO: 765 - DNA, 13 bp, Zea mays;
  source 1..13: mol_type = unassigned DNA
agcagcagcgggg

SEQ ID NO: 766 - DNA, 13 bp, Zea mays;
  source 1..13: mol_type = unassigned DNA
cagcagcaggggc

SEQ ID NO: 767 - DNA, 18 bp, Zea mays;
  source 1..18: mol_type = unassigned DNA
cacgcggtggtggacatg

SEQ ID NO: 768 - DNA, 20 bp, Zea mays;
  source 1..20: mol_type = unassigned DNA
tccacgctcatctccttgtg

SEQ ID NO: 769 - DNA, 20 bp, Zea mays;
  source 1..20: mol_type = unassigned DNA
atgatgccaggagaggcaag

SEQ ID NO: 770 - DNA, 16 bp, Zea mays;
  source 1..16: mol_type = unassigned DNA
tgccaggagacgcaag

SEQ ID NO: 771 - DNA, 25 bp, Zea mays;
  source 1..25: mol_type = unassigned DNA
gaacaagaagcatgagcattctgac

SEQ ID NO: 772 - DNA, 21 bp, Zea mays;
  source 1..21: mol_type = unassigned DNA
tcacggttgctctcatcactt

SEQ ID NO: 773 - DNA, 18 bp, Zea mays;
  source 1..18: mol_type = unassigned DNA
cattcctattcaaggtta

SEQ ID NO: 774 - DNA, 17 bp, Zea mays;
  source 1..17: mol_type = unassigned DNA
ttcctattcaaggctaa

SEQ ID NO: 775 - DNA, 17 bp, Zea mays;
  source 1..17: mol_type = unassigned DNA
aggcacgtggatatctg

SEQ ID NO: 776 - DNA, 15 bp, Zea mays;
  source 1..15: mol_type = unassigned DNA
gtgtggagcaaccaa

SEQ ID NO: 777 - DNA, 16 bp, Zea mays;
  source 1..16: mol_type = unassigned DNA
ctgatagcgcgcagtg

SEQ ID NO: 778 - DNA, 18 bp, Zea mays;
  source 1..18: mol_type = unassigned DNA
ctgatagcgagcagtgac

SEQ ID NO: 779 - DNA, 21 bp, Zea mays;
  source 1..21: mol_type = unassigned DNA
gcacctcagtgaaacgacaag

SEQ ID NO: 780 - DNA, 21 bp, Zea mays;
  source 1..21: mol_type = unassigned DNA
tgaggaaggtgagtgatttgc

SEQ ID NO: 781 - DNA, 19 bp, Zea mays;
  source 1..19: mol_type = unassigned DNA
cgatgcacactaagatgac

SEQ ID NO: 782 - DNA, 17 bp, Zea mays;
  source 1..17: mol_type = unassigned DNA
cgatgcacaccaagatg

SEQ ID NO: 783 - DNA, 20 bp, Zea mays;
  source 1..20: mol_type = unassigned DNA
gaagggccaaactgaggcat

SEQ ID NO: 784 - DNA, 19 bp, Zea mays;
  source 1..19: mol_type = unassigned DNA
acttcccggttgagcaaga

SEQ ID NO: 785 - DNA, 18 bp, Zea mays;
  source 1..18: mol_type = unassigned DNA
cctagttagggttatgtg

SEQ ID NO: 786 - DNA, 19 bp, Zea mays;
  source 1..19: mol_type = unassigned DNA
cctagttagggttatatgg

SEQ ID NO: 787 - DNA, 22 bp, Zea mays;
  source 1..22: mol_type = unassigned DNA
tgcgtttacgtctgcaattaga

SEQ ID NO: 788 - DNA, 23 bp, Zea mays;
  source 1..23: mol_type = unassigned DNA
ctggcctctttctcttctctgta

SEQ ID NO: 789 - DNA, 17 bp, Zea mays;
  source 1..17: mol_type = unassigned DNA
ccttgtgcctgattcaa

SEQ ID NO: 790 - DNA, 16 bp, Zea mays;
  source 1..16: mol_type = unassigned DNA
ttgtgcccgattcaac

SEQ ID NO: 791 - DNA, 23 bp, Zea mays;
  source 1..23: mol_type = unassigned DNA
cgcaagtcattgttcgctgtttg

SEQ ID NO: 792 - DNA, 23 bp, Zea mays;
  source 1..23: mol_type = unassigned DNA
gtcgtcaccgtctttctttcaac

SEQ ID NO: 793 - DNA, 19 bp, Zea mays;
  source 1..19: mol_type = unassigned DNA
agcaggctatgttttagtt

SEQ ID NO: 794 - DNA, 17 bp, Zea mays;
  source 1..17: mol_type = unassigned DNA
agcaggctatgtttcag

SEQ ID NO: 795 - DNA, 19 bp, Zea mays;
  source 1..19: mol_type = unassigned DNA
acttctcaagaggctaaac

SEQ ID NO: 796 - DNA, 18 bp, Zea mays;
  source 1..18: mol_type = unassigned DNA
gctgtaacctgtggtcta

SEQ ID NO: 797 - DNA, 20 bp, Zea mays;
  source 1..20: mol_type = unassigned DNA
ctgaggtagtatataagaag

SEQ ID NO: 798 - DNA, 20 bp, Zea mays;
  source 1..20: mol_type = unassigned DNA
tctgaggtagtatataaaaa

SEQ ID NO: 799 - DNA, 20 bp, Zea mays;
  source 1..20: mol_type = unassigned DNA
agagaatacttgagaaggct

SEQ ID NO: 800 - DNA, 18 bp, Zea mays;
  source 1..18: mol_type = unassigned DNA
gtactgatgggactggat

SEQ ID NO: 801 - DNA, 20 bp, Zea mays;
  source 1..20: mol_type = unassigned DNA
atattttattcctcgtttca

SEQ ID NO: 802 - DNA, 20 bp, Zea mays;
  source 1..20: mol_type = unassigned DNA
atattttattcctcatttca

SEQ ID NO: 803 - DNA, 21 bp, Zea mays;
  source 1..21: mol_type = unassigned DNA
gaaactctacatttgggagat

SEQ ID NO: 804 - DNA, 22 bp, Zea mays;
  source 1..22: mol_type = unassigned DNA
ggacacaattatatgacctctt

SEQ ID NO: 805 - DNA, 16 bp, Zea mays;
  source 1..16: mol_type = unassigned DNA
tttgggcggtcaatgg

SEQ ID NO: 806 - DNA, 13 bp, Zea mays;
  source 1..13: mol_type = unassigned DNA
tgggcggccaatg

SEQ ID NO: 807 - DNA, 18 bp, Zea mays;
  source 1..18: mol_type = unassigned DNA
tgcgttccggccttactc

SEQ ID NO: 808 - DNA, 21 bp, Zea mays;
  source 1..21: mol_type = unassigned DNA
actgcgtttctccctttgctt

SEQ ID NO: 809 - DNA, 14 bp, Zea mays;
  source 1..14: mol_type = unassigned DNA
ccgcgatgcccttg

SEQ ID NO: 810 - DNA, 13 bp, Zea mays;
  source 1..13: mol_type = unassigned DNA
cgcgacgcccttg

SEQ ID NO: 811 - DNA, 20 bp, Zea mays;
  source 1..20: mol_type = unassigned DNA
ggcaggtttcgtaccacatc

SEQ ID NO: 812 - DNA, 21 bp, Zea mays;
  source 1..21: mol_type = unassigned DNA
cgaggatccgtgctcttctaa

SEQ ID NO: 813 - DNA, 17 bp, Zea mays;
  source 1..17: mol_type = unassigned DNA
cagcagccttgatctgt

SEQ ID NO: 814 - DNA, 15 bp, Zea mays;
  source 1..15: mol_type = unassigned DNA
cagcagcctcgatct

SEQ ID NO: 815 - DNA, 22 bp, Zea mays;
  source 1..22: mol_type = unassigned DNA
cctccaagatgtgctccatgat

SEQ ID NO: 816 - DNA, 17 bp, Zea mays;
  source 1..17: mol_type = unassigned DNA
tcgccgaggtcctgtct

SEQ ID NO: 817 - DNA, 14 bp, Zea mays;
  source 1..14: mol_type = unassigned DNA
cggcggtgggatga

SEQ ID NO: 818 - DNA, 13 bp, Zea mays;
  source 1..13: mol_type = unassigned DNA
cggcggcgggatg

SEQ ID NO: 819 - DNA, 20 bp, Zea mays;
  source 1..20: mol_type = unassigned DNA
gcgtgtgagagggacaaagg

SEQ ID NO: 820 - DNA, 18 bp, Zea mays;
  source 1..18: mol_type = unassigned DNA
gtgcacaacgcactgttc

SEQ ID NO: 821 - DNA, 13 bp, Zea mays;
  source 1..13: mol_type = unassigned DNA
ccttggtgcctgc

SEQ ID NO: 822 - DNA, 14 bp, Zea mays;
  source 1..14: mol_type = unassigned DNA
cccttggtgcctac

SEQ ID NO: 823 - DNA, 28 bp, Zea mays;
  source 1..28: mol_type = unassigned DNA
cccaagatccaagaagcgatatatatgc

SEQ ID NO: 824 - DNA, 19 bp, Zea mays;
  source 1..19: mol_type = unassigned DNA
ggcgatcgggtgcaatttg

SEQ ID NO: 825 - DNA, 16 bp, Zea mays;
  source 1..16: mol_type = unassigned DNA
ttaggccttgtttgtt

SEQ ID NO: 826 - DNA, 14 bp, Zea mays;
  source 1..14: mol_type = unassigned DNA
aggccttgttcgtt

SEQ ID NO: 827 - DNA, 18 bp, Zea mays;
  source 1..18: mol_type = unassigned DNA
cagtggcagtaactgata

SEQ ID NO: 828 - DNA, 19 bp, Zea mays;
  source 1..19: mol_type = unassigned DNA
aagcaatccggttaggaat

SEQ ID NO: 829 - DNA, 18 bp, Zea mays;
  source 1..18: mol_type = unassigned DNA
ccgacgatcatattcgta

SEQ ID NO: 830 - DNA, 17 bp, Zea mays;
  source 1..17: mol_type = unassigned DNA
cgacgatcacattcgta

SEQ ID NO: 831 - DNA, 21 bp, Zea mays;
  source 1..21: mol_type = unassigned DNA
ctgctgctgcaagcaattgta

SEQ ID NO: 832 - DNA, 24 bp, Zea mays;
  source 1..24: mol_type = unassigned DNA
tggcactgactaacagtctaacag

SEQ ID NO: 833 - DNA, 14 bp, Zea mays;
  source 1..14: mol_type = unassigned DNA
ctgcagatccccag

SEQ ID NO: 834 - DNA, 13 bp, Zea mays;
  source 1..13: mol_type = unassigned DNA
tgcagacccccag

SEQ ID NO: 835 - DNA, 15 bp, Zea mays;
  source 1..15: mol_type = unassigned DNA
ctgctccgacgactg

SEQ ID NO: 836 - DNA, 16 bp, Zea mays;
  source 1..16: mol_type = unassigned DNA
ctgagctgctcaaggt

SEQ ID NO: 837 - DNA, 20 bp, Zea mays;
  source 1..20: mol_type = unassigned DNA
aaacgttacctgataaatct

SEQ ID NO: 838 - DNA, 19 bp, Zea mays;
  source 1..19: mol_type = unassigned DNA
aacgttacctgataaacct

SEQ ID NO: 839 - DNA, 19 bp, Zea mays;
  source 1..19: mol_type = unassigned DNA
tgtttgcagcccctctcaa

SEQ ID NO: 840 - DNA, 17 bp, Zea mays;
  source 1..17: mol_type = unassigned DNA
ttctggcccgtgttgct

SEQ ID NO: 841 - DNA, 16 bp, Zea mays;
  source 1..16: mol_type = unassigned DNA
tcattctggtgctcat

SEQ ID NO: 842 - DNA, 16 bp, Zea mays;
  source 1..16: mol_type = unassigned DNA
tcattctggtgcacat

SEQ ID NO: 843 - DNA, 22 bp, Zea mays;
  source 1..22: mol_type = unassigned DNA
tctaggtttcggctagtggtta

SEQ ID NO: 844 - DNA, 25 bp, Zea mays;
  source 1..25: mol_type = unassigned DNA
actattacacttcgtctctgggttt

SEQ ID NO: 845 - DNA, 20 bp, Zea mays;
  source 1..20: mol_type = unassigned DNA
agctctccttgatatgaacc

SEQ ID NO: 846 - DNA, 17 bp, Zea mays;
  source 1..17: mol_type = unassigned DNA
ctccttgatacgaaccc

SEQ ID NO: 847 - DNA, 24 bp, Zea mays;
  source 1..24: mol_type = unassigned DNA
tctcctaaacccattgcaaacagt

SEQ ID NO: 848 - DNA, 22 bp, Zea mays;
  source 1..22: mol_type = unassigned DNA
tcaagacttgcacttgctcagt

SEQ ID NO: 849 - DNA, 19 bp, Zea mays;
  source 1..19: mol_type = unassigned DNA
caagaaccgagattttact

SEQ ID NO: 850 - DNA, 20 bp, Zea mays;
  source 1..20: mol_type = unassigned DNA
caagaaccgagagtttactt

SEQ ID NO: 851 - DNA, 22 bp, Zea mays;
  source 1..22: mol_type = unassigned DNA
aggttgcattgatgttggttgt

SEQ ID NO: 852 - DNA, 20 bp, Zea mays;
  source 1..20: mol_type = unassigned DNA
cagcactcctggaattcaca

SEQ ID NO: 853 - DNA, 13 bp, Zea mays;
  source 1..13: mol_type = unassigned DNA
tgggcctctggtc

SEQ ID NO: 854 - DNA, 14 bp, Zea mays;
  source 1..14: mol_type = unassigned DNA
ctgggcctctgatc

SEQ ID NO: 855 - DNA, 18 bp, Zea mays;
  source 1..18: mol_type = unassigned DNA
acaggactgtatctggtg

SEQ ID NO: 856 - DNA, 17 bp, Zea mays;
  source 1..17: mol_type = unassigned DNA
tgcagggtagttagcat

SEQ ID NO: 857 - DNA, 20 bp, Zea mays;
  source 1..20: mol_type = unassigned DNA
ttagtctcttggatgcataa

SEQ ID NO: 858 - DNA, 18 bp, Zea mays;
  source 1..18: mol_type = unassigned DNA
agtctcttggacgcataa

SEQ ID NO: 859 - DNA, 24 bp, Zea mays;
  source 1..24: mol_type = unassigned DNA
gaagctagtattgtccacctcctt

SEQ ID NO: 860 - DNA, 25 bp, Zea mays;
  source 1..25: mol_type = unassigned DNA
tcgagagagttagatgagacagtga

SEQ ID NO: 861 - DNA, 16 bp, Zea mays;
  source 1..16: mol_type = unassigned DNA
ataaatccccatcggg

SEQ ID NO: 862 - DNA, 16 bp, Zea mays;
  source 1..16: mol_type = unassigned DNA
ataaatccccaacggg

SEQ ID NO: 863 - DNA, 19 bp, Zea mays;
  source 1..19: mol_type = unassigned DNA
ggatccccacgaacgcttg

SEQ ID NO: 864 - DNA, 21 bp, Zea mays;
  source 1..21: mol_type = unassigned DNA
gcacggacactcagctagtta

SEQ ID NO: 865 - DNA, 13 bp, Zea mays;
  source 1..13: mol_type = unassigned DNA
cggctacggcgag

SEQ ID NO: 866 - DNA, 14 bp, Zea mays;
  source 1..14: mol_type = unassigned DNA
agcggctacgacga

SEQ ID NO: 867 - DNA, 20 bp, Zea mays;
  source 1..20: mol_type = unassigned DNA
aggcacgagtcaactaggga

SEQ ID NO: 868 - DNA, 21 bp, Zea mays;
  source 1..21: mol_type = unassigned DNA
cagcccatctgcatcctcatc

SEQ ID NO: 869 - DNA, 21 bp, Zea mays;
  source 1..21: mol_type = unassigned DNA
cttgtttgaaaggaaatgacc

SEQ ID NO: 870 - DNA, 19 bp, Zea mays;
  source 1..19: mol_type = unassigned DNA
tgtttgaaagcaaatgacc

SEQ ID NO: 871 - DNA, 24 bp, Zea mays;
  source 1..24: mol_type = unassigned DNA
gtgtccgcttgaccctatatcttc

SEQ ID NO: 872 - DNA, 20 bp, Zea mays;
  source 1..20: mol_type = unassigned DNA
gcagcagcctttccgttcag

SEQ ID NO: 873 - DNA, 14 bp, Zea mays;
  source 1..14: mol_type = unassigned DNA
cttcggcaggcacg

SEQ ID NO: 874 - DNA, 15 bp, Zea mays;
  source 1..15: mol_type = unassigned DNA
acgcttcgacaggca

SEQ ID NO: 875 - DNA, 18 bp, Zea mays;
  source 1..18: mol_type = unassigned DNA
acacggccacacggacac

SEQ ID NO: 876 - DNA, 16 bp, Zea mays;
  source 1..16: mol_type = unassigned DNA
tcgcgctcccgacaag

SEQ ID NO: 877 - DNA, 18 bp, Zea mays;
  source 1..18: mol_type = unassigned DNA
aaagggcgctatagtgga

SEQ ID NO: 878 - DNA, 17 bp, Zea mays;
  source 1..17: mol_type = unassigned DNA
agggcgctacagtggac

SEQ ID NO: 879 - DNA, 25 bp, Zea mays;
  source 1..25: mol_type = unassigned DNA
cttctaaattctgacgagcacgaaa

SEQ ID NO: 880 - DNA, 22 bp, Zea mays;
  source 1..22: mol_type = unassigned DNA
ggctgcagtgattcagtttgac

SEQ ID NO: 881 - DNA, 15 bp, Zea mays;
  source 1..15: mol_type = unassigned DNA
acggtgtgtccgtct

SEQ ID NO: 882 - DNA, 15 bp, Zea mays;
  source 1..15: mol_type = unassigned DNA
acggtgtgtccgtca

SEQ ID NO: 883 - DNA, 20 bp, Zea mays;
  source 1..20: mol_type = unassigned DNA
gctctgccactctgttgcat

SEQ ID NO: 884 - DNA, 19 bp, Zea mays;
  source 1..19: mol_type = unassigned DNA
ccacggtgtggagtgtgag

SEQ ID NO: 885 - DNA, 19 bp, Zea mays;
  source 1..19: mol_type = unassigned DNA
cctcaatcgatatggatta

SEQ ID NO: 886 - DNA, 18 bp, Zea mays;
  source 1..18: mol_type = unassigned DNA
cacctcaatcgatatgaa

SEQ ID NO: 887 - DNA, 15 bp, Zea mays;
  source 1..15: mol_type = unassigned DNA
ctcactacgcggcag

SEQ ID NO: 888 - DNA, 19 bp, Zea mays;
  source 1..19: mol_type = unassigned DNA
tcatgactggatacgtatg

SEQ ID NO: 889 - DNA, 14 bp, Zea mays;
  source 1..14: mol_type = unassigned DNA
aggcactggtcgtt

SEQ ID NO: 890 - DNA, 16 bp, Zea mays;
  source 1..16: mol_type = unassigned DNA
taggcactggtcattg

SEQ ID NO: 891 - DNA, 20 bp, Zea mays;
  source 1..20: mol_type = unassigned DNA
gccagtaccaggtacaccat

SEQ ID NO: 892 - DNA, 25 bp, Zea mays;
  source 1..25: mol_type = unassigned DNA
cctaagtcattaccttgcagggata

SEQ ID NO: 893 - DNA, 21 bp, Zea mays;
  source 1..21: mol_type = unassigned DNA
cttagtatgtttttgtcatga

SEQ ID NO: 894 - DNA, 23 bp, Zea mays;
  source 1..23: mol_type = unassigned DNA
tacttagtatgtttttatcatga

SEQ ID NO: 895 - DNA, 25 bp, Zea mays;
  source 1..25: mol_type = unassigned DNA
gtttaacttctctttgctagccgat

SEQ ID NO: 896 - DNA, 22 bp, Zea mays;
  source 1..22: mol_type = unassigned DNA
ccggaatgctactgaacaacac

SEQ ID NO: 897 - DNA, 15 bp, Zea mays;
  source 1..15: mol_type = unassigned DNA
tgtcacacggctatc

SEQ ID NO: 898 - DNA, 17 bp, Zea mays;
  source 1..17: mol_type = unassigned DNA
caaatgtcacacagcta

SEQ ID NO: 899 - DNA, 19 bp, Zea mays;
  source 1..19: mol_type = unassigned DNA
gaactgatacgctactctt

SEQ ID NO: 900 - DNA, 22 bp, Zea mays;
  source 1..22: mol_type = unassigned DNA
accatattggataaaactcttg

SEQ ID NO: 901 - DNA, 15 bp, Zea mays;
  source 1..15: mol_type = unassigned DNA
catgctttgcgcggt

SEQ ID NO: 902 - DNA, 16 bp, Zea mays;
  source 1..16: mol_type = unassigned DNA
tcatgctatgcgcggt

SEQ ID NO: 903 - DNA, 16 bp, Zea mays;
  source 1..16: mol_type = unassigned DNA
atcgtcgccgccgtgt

SEQ ID NO: 904 - DNA, 21 bp, Zea mays;
  source 1..21: mol_type = unassigned DNA
agctcccggtgtgatatcctt

SEQ ID NO: 905 - DNA, 16 bp, Zea mays;
  source 1..16: mol_type = unassigned DNA
agtgtggcgatctcct

SEQ ID NO: 906 - DNA, 16 bp, Zea mays;
  source 1..16: mol_type = unassigned DNA
agtgtggcgatctccc

SEQ ID NO: 907 - DNA, 20 bp, Zea mays;
  source 1..20: mol_type = unassigned DNA
cgacactgctctgctgaatc

SEQ ID NO: 908 - DNA, 23 bp, Zea mays;
  source 1..23: mol_type = unassigned DNA
acggtcattcatctcatcgaaca

SEQ ID NO: 909 - DNA, 20 bp, Zea mays;
  source 1..20: mol_type = unassigned DNA
atttattaataggctacgtt

SEQ ID NO: 910 - DNA, 21 bp, Zea mays;
  source 1..21: mol_type = unassigned DNA
tgtatttattaataggctaca

SEQ ID NO: 911 - DNA, 20 bp, Zea mays;
  source 1..20: mol_type = unassigned DNA
agcaacagacgcctcacttc

SEQ ID NO: 912 - DNA, 23 bp, Zea mays;
  source 1..23: mol_type = unassigned DNA
tccaagcacaggagacaactaag

SEQ ID NO: 913 - DNA, 18 bp, Zea mays;
  source 1..18: mol_type = unassigned DNA
tgagaacagtcatgcctt

SEQ ID NO: 914 - DNA, 18 bp, Zea mays;
  source 1..18: mol_type = unassigned DNA
agaacagtcacgcctttg

SEQ ID NO: 915 - DNA, 23 bp, Zea mays;
  source 1..23: mol_type = unassigned DNA
tgttgaaatacgatgcgctatgg

SEQ ID NO: 916 - DNA, 23 bp, Zea mays;
  source 1..23: mol_type = unassigned DNA
gccaatgttgacaaccaaacagc

SEQ ID NO: 917 - DNA, 17 bp, Zea mays;
  source 1..17: mol_type = unassigned DNA
aggtgtagtcgtcgtgt

SEQ ID NO: 918 - DNA, 17 bp, Zea mays;
  source 1..17: mol_type = unassigned DNA
aggtgtagtcgtcctgt

SEQ ID NO: 919 - DNA, 24 bp, Zea mays;
  source 1..24: mol_type = unassigned DNA
ctcaatcgatgttaaataagtatc

SEQ ID NO: 920 - DNA, 17 bp, Zea mays;
  source 1..17: mol_type = unassigned DNA
gagattggcgtagtcaa

SEQ ID NO: 921 - DNA, 18 bp, Zea mays;
  source 1..18: mol_type = unassigned DNA
ctatggccggtatgtcat

SEQ ID NO: 922 - DNA, 15 bp, Zea mays;
  source 1..15: mol_type = unassigned DNA
tggccggtatgccat

SEQ ID NO: 923 - DNA, 21 bp, Zea mays;
  source 1..21: mol_type = unassigned DNA
tgcaggatttgttcaatctat

SEQ ID NO: 924 - DNA, 16 bp, Zea mays;
  source 1..16: mol_type = unassigned DNA
gacgacgacttcatca

SEQ ID NO: 925 - DNA, 16 bp, Zea mays;
  source 1..16: mol_type = unassigned DNA
ttctcactccttactt

SEQ ID NO: 926 - DNA, 15 bp, Zea mays;
  source 1..15: mol_type = unassigned DNA
ctcactccttacctt

SEQ ID NO: 927 - DNA, 20 bp, Zea mays;
  source 1..20: mol_type = unassigned DNA
agcgtgtttggtttgaggaa

SEQ ID NO: 928 - DNA, 25 bp, Zea mays;
  source 1..25: mol_type = unassigned DNA
gtggagtcactttatgcttcatgag

SEQ ID NO: 929 - DNA, 17 bp, Zea mays;
  source 1..17: mol_type = unassigned DNA
ctagctcctgtgggatg

SEQ ID NO: 930 - DNA, 16 bp, Zea mays;
  source 1..16: mol_type = unassigned DNA
ctagctcccgtgggat

SEQ ID NO: 931 - DNA, 17 bp, Zea mays;
  source 1..17: mol_type = unassigned DNA
cgagctgtgggtcgtga

SEQ ID NO: 932 - DNA, 20 bp, Zea mays;
  source 1..20: mol_type = unassigned DNA
gaaggcaaccgtctcggtat

SEQ ID NO: 933 - DNA, 13 bp, Zea mays;
  source 1..13: mol_type = unassigned DNA
acttccgcctgct

SEQ ID NO: 934 - DNA, 13 bp, Zea mays;
  source 1..13: mol_type = unassigned DNA
acttccgcctgcc

SEQ ID NO: 935 - DNA, 19 bp, Zea mays;
  source 1..19: mol_type = unassigned DNA
ccttcgccgcgttacactg

SEQ ID NO: 936 - DNA, 21 bp, Zea mays;
  source 1..21: mol_type = unassigned DNA
ggtgtggagtggacgtgatac

SEQ ID NO: 937 - DNA, 15 bp, Zea mays;
  source 1..15: mol_type = unassigned DNA
tggcccgacatcagg

SEQ ID NO: 938 - DNA, 16 bp, Zea mays;
  source 1..16: mol_type = unassigned DNA
tgtggcccaacatcag

SEQ ID NO: 939 - DNA, 18 bp, Zea mays;
  source 1..18: mol_type = unassigned DNA
cggactgctcgactggaa

SEQ ID NO: 940 - DNA, 21 bp, Zea mays;
  source 1..21: mol_type = unassigned DNA
gtcgagggtgagccaatactc

SEQ ID NO: 941 - DNA, 19 bp, Zea mays;
  source 1..19: mol_type = unassigned DNA
tttggcaaaacggtttata

SEQ ID NO: 942 - DNA, 19 bp, Zea mays;
  source 1..19: mol_type = unassigned DNA
tttggcaaaacggcttata

SEQ ID NO: 943 - DNA, 22 bp, Zea mays;
  source 1..22: mol_type = unassigned DNA
ggtgcagccacttctttagatg

SEQ ID NO: 944 - DNA, 22 bp, Zea mays;
  source 1..22: mol_type = unassigned DNA
cctagccacgtacaggagagat

SEQ ID NO: 945 - DNA, 18 bp, Zea mays;
  source 1..18: mol_type = unassigned DNA
cagtgacccatttctttt

SEQ ID NO: 946 - DNA, 19 bp, Zea mays;
  source 1..19: mol_type = unassigned DNA
agtgacccatttctttctt

SEQ ID NO: 947 - DNA, 24 bp, Zea mays;
  source 1..24: mol_type = unassigned DNA
aaggacgaagtagcagctggaaag

SEQ ID NO: 948 - DNA, 25 bp, Zea mays;
  source 1..25: mol_type = unassigned DNA
agggctactttgggaacctcaaatc

SEQ ID NO: 949 - DNA, 17 bp, Zea mays;
  source 1..17: mol_type = unassigned DNA
tacaactcagcgagcta

SEQ ID NO: 950 - DNA, 18 bp, Zea mays;
  source 1..18: mol_type = unassigned DNA
atgtacaactcaccgagc

SEQ ID NO: 951 - DNA, 22 bp, Zea mays;
  source 1..22: mol_type = unassigned DNA
agtgggcagtgcacatatgatg

SEQ ID NO: 952 - DNA, 22 bp, Zea mays;
  source 1..22: mol_type = unassigned DNA
caactccaaccgccaataatgc

SEQ ID NO: 953 - DNA, 18 bp, Zea mays;
  source 1..18: mol_type = unassigned DNA
ccttttggattacttcac

SEQ ID NO: 954 - DNA, 17 bp, Zea mays;
  source 1..17: mol_type = unassigned DNA
ttttggatcacttcaca

SEQ ID NO: 955 - DNA, 20 bp, Zea mays;
  source 1..20: mol_type = unassigned DNA
gccgcagtaaagtacacgaa

SEQ ID NO: 956 - DNA, 25 bp, Zea mays;
  source 1..25: mol_type = unassigned DNA
atgggcctaaagaacaaatgcacaa

SEQ ID NO: 957 - DNA, 17 bp, Zea mays;
  source 1..17: mol_type = unassigned DNA
actttggctatgctttg

SEQ ID NO: 958 - DNA, 19 bp, Zea mays;
  source 1..19: mol_type = unassigned DNA
tgttactttggctatgatt

SEQ ID NO: 959 - DNA, 24 bp, Zea mays;
  source 1..24: mol_type = unassigned DNA
acaatgaacgactcctgtcagaat

SEQ ID NO: 960 - DNA, 20 bp, Zea mays;
  source 1..20: mol_type = unassigned DNA
ggctctagggaccatgaaca

SEQ ID NO: 961 - DNA, 18 bp, Zea mays;
  source 1..18: mol_type = unassigned DNA
ttaaattgtcgagcttgt

SEQ ID NO: 962 - DNA, 16 bp, Zea mays;
  source 1..16: mol_type = unassigned DNA
aaattgtcgagcctgt

SEQ ID NO: 963 - DNA, 25 bp, Zea mays;
  source 1..25: mol_type = unassigned DNA
actcatgtttatccttagcagcaaa

SEQ ID NO: 964 - DNA, 25 bp, Zea mays;
  source 1..25: mol_type = unassigned DNA
gcacattgataatctcagctccatt

SEQ ID NO: 965 - DNA, 18 bp, Zea mays;
  source 1..18: mol_type = unassigned DNA
caactgagagactgtatg

SEQ ID NO: 966 - DNA, 16 bp, Zea mays;
  source 1..16: mol_type = unassigned DNA
ctgagagactgcatga

SEQ ID NO: 967 - DNA, 27 bp, Zea mays;
  source 1..27: mol_type = unassigned DNA
gatggtgaataattggcatgtataacc

SEQ ID NO: 968 - DNA, 23 bp, Zea mays;
  source 1..23: mol_type = unassigned DNA
gtgcttggagaaccgaaacatag

SEQ ID NO: 969 - DNA, 15 bp, Zea mays;
  source 1..15: mol_type = unassigned DNA
ctgggcattcggttt

SEQ ID NO: 970 - DNA, 16 bp, Zea mays;
  source 1..16: mol_type = unassigned DNA
ctgggcattcgatttt

SEQ ID NO: 971 - DNA, 20 bp, Zea mays;
  source 1..20: mol_type = unassigned DNA
acaactgtatcttactgcta

SEQ ID NO: 972 - DNA, 16 bp, Zea mays;
  source 1..16: mol_type = unassigned DNA
ccgaagttctcggttt

SEQ ID NO: 973 - DNA, 18 bp, Zea mays;
  source 1..18: mol_type = unassigned DNA
agcagtcagttgtccaac

SEQ ID NO: 974 - DNA, 18 bp, Zea mays;
  source 1..18: mol_type = unassigned DNA
agcagtcagtagtccaac

SEQ ID NO: 975 - DNA, 23 bp, Zea mays;
  source 1..23: mol_type = unassigned DNA
ggatgaagttatcaagcctgtga

SEQ ID NO: 976 - DNA, 24 bp, Zea mays;
  source 1..24: mol_type = unassigned DNA
tttgcaagagattctgtgaactgt

SEQ ID NO: 977 - DNA, 17 bp, Zea mays;
  source 1..17: mol_type = unassigned DNA
ccgttccttcaatgcta

SEQ ID NO: 978 - DNA, 19 bp, Zea mays;
  source 1..19: mol_type = unassigned DNA
tccgttccttaaatgctac

SEQ ID NO: 979 - DNA, 21 bp, Zea mays;
  source 1..21: mol_type = unassigned DNA
gtctgccagtggttcctaacg

SEQ ID NO: 980 - DNA, 23 bp, Zea mays;
  source 1..23: mol_type = unassigned DNA
tcaccccgggaattaggatgatg

SEQ ID NO: 981 - DNA, 17 bp, Zea mays;
  source 1..17: mol_type = unassigned DNA
atcaccgagccagatat

SEQ ID NO: 982 - DNA, 16 bp, Zea mays;
  source 1..16: mol_type = unassigned DNA
accgagccagacatta

SEQ ID NO: 983 - DNA, 22 bp, Zea mays;
  source 1..22: mol_type = unassigned DNA
ttgtttcctcccccaagtacag

SEQ ID NO: 984 - DNA, 21 bp, Zea mays;
  source 1..21: mol_type = unassigned DNA
cgcaggcatgtctatgacaac

SEQ ID NO: 985 - DNA, 19 bp, Zea mays;
  source 1..19: mol_type = unassigned DNA
ttctggttttgtatgtatg

SEQ ID NO: 986 - DNA, 20 bp, Zea mays;
  source 1..20: mol_type = unassigned DNA
tagagttctggttttgtata

SEQ ID NO: 987 - DNA, 24 bp, Zea mays;
  source 1..24: mol_type = unassigned DNA
tgtttcctgatgttttggttgaca

SEQ ID NO: 988 - DNA, 22 bp, Zea mays;
  source 1..22: mol_type = unassigned DNA
ccactcatgtgggagttgtctc

SEQ ID NO: 989 - DNA, 17 bp, Zea mays;
  source 1..17: mol_type = unassigned DNA
aggaacaaggcctttcg

SEQ ID NO: 990 - DNA, 18 bp, Zea mays;
  source 1..18: mol_type = unassigned DNA
aaggaacaaggccttacg

SEQ ID NO: 991 - DNA, 24 bp, Zea mays;
  source 1..24: mol_type = unassigned DNA
cacctgaaatcgttccacccaatt

SEQ ID NO: 992 - DNA, 22 bp, Zea mays;
  source 1..22: mol_type = unassigned DNA
ttggcggaatcactagctgttc

SEQ ID NO: 993 - DNA, 20 bp, Zea mays;
  source 1..20: mol_type = unassigned DNA
ccacaattgaaggaaatgga

SEQ ID NO: 994 - DNA, 20 bp, Zea mays;
  source 1..20: mol_type = unassigned DNA
tgccacaattgaaagaaatg

SEQ ID NO: 995 - DNA, 24 bp, Zea mays;
  source 1..24: mol_type = unassigned DNA
gggatttatagagggttcgagacg

SEQ ID NO: 996 - DNA, 17 bp, Zea mays;
  source 1..17: mol_type = unassigned DNA
tcctatgctgcggtcca

SEQ ID NO: 997 - DNA, 14 bp, Zea mays;
  source 1..14: mol_type = unassigned DNA
cggactcggctctc

SEQ ID NO: 998 - DNA, 14 bp, Zea mays;
  source 1..14: mol_type = unassigned DNA
cggactccgctctc

SEQ ID NO: 999 - DNA, 21 bp, Zea mays;
  source 1..21: mol_type = unassigned DNA
ggtttggaaggagcccgttct

SEQ ID NO: 1000 - DNA, 17 bp, Zea mays;
  source 1..17: mol_type = unassigned DNA
agcttgccgccggagta

SEQ ID NO: 1001 - DNA, 15 bp, Zea mays;
  source 1..15: mol_type = unassigned DNA
accctaccctaccct

SEQ ID NO: 1002 - DNA, 15 bp, Zea mays;
  source 1..15: mol_type = unassigned DNA
caccctacactaccc

SEQ ID NO: 1003 - DNA, 20 bp, Zea mays;
  source 1..20: mol_type = unassigned DNA
gatcttggcaggaccaacac

SEQ ID NO: 1004 - DNA, 21 bp, Zea mays;
  source 1..21: mol_type = unassigned DNA
gcgaagcgataagcacacatc

SEQ ID NO: 1005 - DNA, 18 bp, Zea mays;
  source 1..18: mol_type = unassigned DNA
tgttagtgggtatgggta

SEQ ID NO: 1006 - DNA, 18 bp, Zea mays;
  source 1..18: mol_type = unassigned DNA
ttagtgggtatggatacc

SEQ ID NO: 1007 - DNA, 20 bp, Zea mays;
  source 1..20: mol_type = unassigned DNA
ggtacttacatttgcgattc

SEQ ID NO: 1008 - DNA, 15 bp, Zea mays;
  source 1..15: mol_type = unassigned DNA
cacgggtagcaggta

SEQ ID NO: 1009 - DNA, 22 bp, Zea mays;
  source 1..22: mol_type = unassigned DNA
tattgagaattaatgtctaagc

SEQ ID NO: 1010 - DNA, 19 bp, Zea mays;
  source 1..19: mol_type = unassigned DNA
tgagaattaatggctaagc

SEQ ID NO: 1011 - DNA, 21 bp, Zea mays;
  source 1..21: mol_type = unassigned DNA
gtgtctgagacagcagatcga

SEQ ID NO: 1012 - DNA, 23 bp, Zea mays;
  source 1..23: mol_type = unassigned DNA
ggaggcttagatcgtcatattgc

SEQ ID NO: 1013 - DNA, 15 bp, Zea mays;
  source 1..15: mol_type = unassigned DNA
tgggtggtctgctac

SEQ ID NO: 1014 - DNA, 13 bp, Zea mays;
  source 1..13: mol_type = unassigned DNA
tggtccgctacca

SEQ ID NO: 1015 - DNA, 22 bp, Zea mays;
  source 1..22: mol_type = unassigned DNA
acattgcattcttgaatttaga

SEQ ID NO: 1016 - DNA, 17 bp, Zea mays;
  source 1..17: mol_type = unassigned DNA
acttggtcggacgtaag

SEQ ID NO: 1017 - DNA, 21 bp, Zea mays;
  source 1..21: mol_type = unassigned DNA
aaattctggtatttatatatc

SEQ ID NO: 1018 - DNA, 18 bp, Zea mays;
  source 1..18: mol_type = unassigned DNA
ttctggtatttagatatc

SEQ ID NO: 1019 - DNA, 24 bp, Zea mays;
  source 1..24: mol_type = unassigned DNA
tgtacaattatgccattcgggttt

SEQ ID NO: 1020 - DNA, 22 bp, Zea mays;
  source 1..22: mol_type = unassigned DNA
ccgagacaattcgagtgaccta

SEQ ID NO: 1021 - DNA, 20 bp, Zea mays;
  source 1..20: mol_type = unassigned DNA
cttgcttatggattatcata

SEQ ID NO: 1022 - DNA, 20 bp, Zea mays;
  source 1..20: mol_type = unassigned DNA
cacttgcttatggattataa

SEQ ID NO: 1023 - DNA, 20 bp, Zea mays;
  source 1..20: mol_type = unassigned DNA
gaaaacttgaaagggtagtg

SEQ ID NO: 1024 - DNA, 21 bp, Zea mays;
  source 1..21: mol_type = unassigned DNA
acaaacagtccagcttatttg

SEQ ID NO: 1025 - DNA, 16 bp, Zea mays;
  source 1..16: mol_type = unassigned DNA
taggagggcatgggca

SEQ ID NO: 1026 - DNA, 15 bp, Zea mays;
  source 1..15: mol_type = unassigned DNA
agggcacgggcaact

SEQ ID NO: 1027 - DNA, 22 bp, Zea mays;
  source 1..22: mol_type = unassigned DNA
tgtagcgggtatcttaccgaca

SEQ ID NO: 1028 - DNA, 24 bp, Zea mays;
  source 1..24: mol_type = unassigned DNA
tcacttctttctctgcacaaatcc

SEQ ID NO: 1029 - DNA, 13 bp, Zea mays;
  source 1..13: mol_type = unassigned DNA
ccgaacaggcagc

SEQ ID NO: 1030 - DNA, 13 bp, Zea mays;
  source 1..13: mol_type = unassigned DNA
cgaacagccagca

SEQ ID NO: 1031 - DNA, 18 bp, Zea mays;
  source 1..18: mol_type = unassigned DNA
ttccagatatcgagagga

SEQ ID NO: 1032 - DNA, 18 bp, Zea mays;
  source 1..18: mol_type = unassigned DNA
acttgcgaaggtagacag

SEQ ID NO: 1033 - DNA, 13 bp, Zea mays;
  source 1..13: mol_type = unassigned DNA
tctcggccctccg

SEQ ID NO: 1034 - DNA, 15 bp, Zea mays;
  source 1..15: mol_type = unassigned DNA
cttctcgaccctccg

SEQ ID NO: 1035 - DNA, 16 bp, Zea mays;
  source 1..16: mol_type = unassigned DNA
tccgtcgcgcacatcg

SEQ ID NO: 1036 - DNA, 25 bp, Zea mays;
  source 1..25: mol_type = unassigned DNA
gctgttgttacagtgggaatttacc

SEQ ID NO: 1037 - DNA, 21 bp, Zea mays;
  source 1..21: mol_type = unassigned DNA
taaattattagtatctactat

SEQ ID NO: 1038 - DNA, 21 bp, Zea mays;
  source 1..21: mol_type = unassigned DNA
ttttaaattattagtatatac

SEQ ID NO: 1039 - DNA, 25 bp, Zea mays;
  source 1..25: mol_type = unassigned DNA
tgcgacgtttattgaaacacagtta

SEQ ID NO: 1040 - DNA, 19 bp, Zea mays;
  source 1..19: mol_type = unassigned DNA
ccgcacggcttatgtacac

SEQ ID NO: 1041 - DNA, 18 bp, Zea mays;
  source 1..18: mol_type = unassigned DNA
ttgtgaattgaccggtat

SEQ ID NO: 1042 - DNA, 16 bp, Zea mays;
  source 1..16: mol_type = unassigned DNA
tgaattgaccggcatg

SEQ ID NO: 1043 - DNA, 25 bp, Zea mays;
  source 1..25: mol_type = unassigned DNA
acccttgatgtttctcatacgatgc

SEQ ID NO: 1044 - DNA, 20 bp, Zea mays;
  source 1..20: mol_type = unassigned DNA
cgcggatattcagcgtctac

SEQ ID NO: 1045 - DNA, 13 bp, Zea mays;
  source 1..13: mol_type = unassigned DNA
cgatcccaccggc

SEQ ID NO: 1046 - DNA, 13 bp, Zea mays;
  source 1..13: mol_type = unassigned DNA
cgatcccacccgc

SEQ ID NO: 1047 - DNA, 17 bp, Zea mays;
  source 1..17: mol_type = unassigned DNA
aaaacagccgagtatcc

SEQ ID NO: 1048 - DNA, 16 bp, Zea mays;
  source 1..16: mol_type = unassigned DNA
gggtggttttgttcgt

SEQ ID NO: 1049 - DNA, 16 bp, Zea mays;
  source 1..16: mol_type = unassigned DNA
tgtttccagactagtc

SEQ ID NO: 1050 - DNA, 15 bp, Zea mays;
  source 1..15: mol_type = unassigned DNA
ttccagactagcctt

SEQ ID NO: 1051 - DNA, 28 bp, Zea mays;
  source 1..28: mol_type = unassigned DNA
acaagggattctaatttttccaatgaaa

SEQ ID NO: 1052 - DNA, 26 bp, Zea mays;
  source 1..26: mol_type = unassigned DNA
cgctaatcatatataggcgactcttc

SEQ ID NO: 1053 - DNA, 19 bp, Zea mays;
  source 1..19: mol_type = unassigned DNA
tgtggtccaaattttgtat

SEQ ID NO: 1054 - DNA, 17 bp, Zea mays;
  source 1..17: mol_type = unassigned DNA
tggtccaaattttgcat

SEQ ID NO: 1055 - DNA, 21 bp, Zea mays;
  source 1..21: mol_type = unassigned DNA
acacgtcatgcttacctacga

SEQ ID NO: 1056 - DNA, 21 bp, Zea mays;
  source 1..21: mol_type = unassigned DNA
gcttcactcgcaagacagttg

SEQ ID NO: 1057 - DNA, 16 bp, Zea mays;
  source 1..16: mol_type = unassigned DNA
cggttgccattatcat

SEQ ID NO: 1058 - DNA, 14 bp, Zea mays;
  source 1..14: mol_type = unassigned DNA
cggttgccattacc

SEQ ID NO: 1059 - DNA, 16 bp, Zea mays;
  source 1..16: mol_type = unassigned DNA
ggtggtccccctgacc

SEQ ID NO: 1060 - DNA, 22 bp, Zea mays;
  source 1..22: mol_type = unassigned DNA
gtggtcgacgtcgttcaatttc

SEQ ID NO: 1061 - DNA, 15 bp, Zea mays;
  source 1..15: mol_type = unassigned DNA
cggccagttcacctt

SEQ ID NO: 1062 - DNA, 14 bp, Zea mays;
  source 1..14: mol_type = unassigned DNA
ccggccaattcacc

SEQ ID NO: 1063 - DNA, 16 bp, Zea mays;
  source 1..16: mol_type = unassigned DNA
ggttcgccgaatgcca

SEQ ID NO: 1064 - DNA, 19 bp, Zea mays;
  source 1..19: mol_type = unassigned DNA
gcatggattccgcactgaa

SEQ ID NO: 1065 - DNA, 20 bp, Zea mays;
  source 1..20: mol_type = unassigned DNA
cagaggacagaaagtatagg

SEQ ID NO: 1066 - DNA, 19 bp, Zea mays;
  source 1..19: mol_type = unassigned DNA
cagaggacagaaagtacag

SEQ ID NO: 1067 - DNA, 18 bp, Zea mays;
  source 1..18: mol_type = unassigned DNA
ccctggaggctggagcag

SEQ ID NO: 1068 - DNA, 21 bp, Zea mays;
  source 1..21: mol_type = unassigned DNA
atctgttggcgcccctaaacc

SEQ ID NO: 1069 - DNA, 18 bp, Zea mays;
  source 1..18: mol_type = unassigned DNA
actagttgtgtgcgaatt

SEQ ID NO: 1070 - DNA, 17 bp, Zea mays;
  source 1..17: mol_type = unassigned DNA
actagttgtgtgccaat

SEQ ID NO: 1071 - DNA, 18 bp, Zea mays;
  source 1..18: mol_type = unassigned DNA
ctactggttcggtgtttc

SEQ ID NO: 1072 - DNA, 21 bp, Zea mays;
  source 1..21: mol_type = unassigned DNA
acctttgagggaattatttca

SEQ ID NO: 1073 - DNA, 20 bp, Zea mays;
  source 1..20: mol_type = unassigned DNA
atgtactacagacatttgaa

SEQ ID NO: 1074 - DNA, 19 bp, Zea mays;
  source 1..19: mol_type = unassigned DNA
tgtactacagacatttcaa

SEQ ID NO: 1075 - DNA, 22 bp, Zea mays;
  source 1..22: mol_type = unassigned DNA
ggtgctactacaggtttggact

SEQ ID NO: 1076 - DNA, 22 bp, Zea mays;
  source 1..22: mol_type = unassigned DNA
actagcctagctgcttccaact

SEQ ID NO: 1077 - DNA, 20 bp, Zea mays;
  source 1..20: mol_type = unassigned DNA
ctttctattatacttgcatg

SEQ ID NO: 1078 - DNA, 18 bp, Zea mays;
  source 1..18: mol_type = unassigned DNA
ttctattatacttgcacg

SEQ ID NO: 1079 - DNA, 18 bp, Zea mays;
  source 1..18: mol_type = unassigned DNA
ccctgcgtatgggctctg

SEQ ID NO: 1080 - DNA, 21 bp, Zea mays;
  source 1..21: mol_type = unassigned DNA
gcgtgaactacacggtgaaag

SEQ ID NO: 1081 - DNA, 13 bp, Zea mays;
  source 1..13: mol_type = unassigned DNA
cacgtcggggccg

SEQ ID NO: 1082 - DNA, 14 bp, Zea mays;
  source 1..14: mol_type = unassigned DNA
acgtcggggccacg

SEQ ID NO: 1083 - DNA, 16 bp, Zea mays;
  source 1..16: mol_type = unassigned DNA
gcacgcgccgtgaact

SEQ ID NO: 1084 - DNA, 16 bp, Zea mays;
  source 1..16: mol_type = unassigned DNA
ggcccagcgtgcctat

SEQ ID NO: 1085 - DNA, 19 bp, Zea mays;
  source 1..19: mol_type = unassigned DNA
aatctcaagtttgtacatc

SEQ ID NO: 1086 - DNA, 19 bp, Zea mays;
  source 1..19: mol_type = unassigned DNA
aatctcaagtttctacatc

SEQ ID NO: 1087 - DNA, 22 bp, Zea mays;
  source 1..22: mol_type = unassigned DNA
tgatagatcttaggaaagtgat

SEQ ID NO: 1088 - DNA, 16 bp, Zea mays;
  source 1..16: mol_type = unassigned DNA
caaccacaagggtgtc

SEQ ID NO: 1089 - DNA, 18 bp, Zea mays;
  source 1..18: mol_type = unassigned DNA
atcgaaccagttctgtgc

SEQ ID NO: 1090 - DNA, 16 bp, Zea mays;
  source 1..16: mol_type = unassigned DNA
aaccagtcctgtgcac

SEQ ID NO: 1091 - DNA, 24 bp, Zea mays;
  source 1..24: mol_type = unassigned DNA
ggcgtagaggatatgtgagaacag

SEQ ID NO: 1092 - DNA, 20 bp, Zea mays;
  source 1..20: mol_type = unassigned DNA
gtgggaaggaagccgacttt

SEQ ID NO: 1093 - DNA, 22 bp, Zea mays;
  source 1..22: mol_type = unassigned DNA
ccataatctcctaatctaagaa

SEQ ID NO: 1094 - DNA, 20 bp, Zea mays;
  source 1..20: mol_type = unassigned DNA
ccataatctcctaacctaag

SEQ ID NO: 1095 - DNA, 23 bp, Zea mays;
  source 1..23: mol_type = unassigned DNA
tgcaatggtgtttataggcaagt

SEQ ID NO: 1096 - DNA, 24 bp, Zea mays;
  source 1..24: mol_type = unassigned DNA
tggtgagccctactgtattgttac

SEQ ID NO: 1097 - DNA, 19 bp, Zea mays;
  source 1..19: mol_type = unassigned DNA
aagtttgtgatttctgttg

SEQ ID NO: 1098 - DNA, 15 bp, Zea mays;
  source 1..15: mol_type = unassigned DNA
tgtgatttccgttgg

SEQ ID NO: 1099 - DNA, 21 bp, Zea mays;
  source 1..21: mol_type = unassigned DNA
aaattattgtcatgcatacac

SEQ ID NO: 1100 - DNA, 20 bp, Zea mays;
  source 1..20: mol_type = unassigned DNA
ctcaaggcctatgaactatc

SEQ ID NO: 1101 - DNA, 14 bp, Zea mays;
  source 1..14: mol_type = unassigned DNA
atccggcggagtgg

SEQ ID NO: 1102 - DNA, 13 bp, Zea mays;
  source 1..13: mol_type = unassigned DNA
atccggcggagcg

SEQ ID NO: 1103 - DNA, 15 bp, Zea mays;
  source 1..15: mol_type = unassigned DNA
tccgactccgccagc

SEQ ID NO: 1104 - DNA, 18 bp, Zea mays;
  source 1..18: mol_type = unassigned DNA
gttcgtggtggacgagga

SEQ ID NO: 1105 - DNA, 20 bp, Zea mays;
  source 1..20: mol_type = unassigned DNA
agtactacatagcatattac

SEQ ID NO: 1106 - DNA, 19 bp, Zea mays;
  source 1..19: mol_type = unassigned DNA
agtactacatagcacatta

SEQ ID NO: 1107 - DNA, 24 bp, Zea mays;
  source 1..24: mol_type = unassigned DNA
aaccatccattcaacacaccaaag

SEQ ID NO: 1108 - DNA, 19 bp, Zea mays;
  source 1..19: mol_type = unassigned DNA
cccgctaacccgtgggtat

SEQ ID NO: 1109 - DNA, 13 bp, Zea mays;
  source 1..13: mol_type = unassigned DNA
ccgcagcgaaggc

SEQ ID NO: 1110 - DNA, 13 bp, Zea mays;
  source 1..13: mol_type = unassigned DNA
ccgcagccaaggc

SEQ ID NO: 1111 - DNA, 19 bp, Zea mays;
  source 1..19: mol_type = unassigned DNA
tcccttccaagagcacacg

SEQ ID NO: 1112 - DNA, 21 bp, Zea mays;
  source 1..21: mol_type = unassigned DNA
gtgctcaggtactacgcctac

SEQ ID NO: 1113 - DNA, 18 bp, Zea mays;
  source 1..18: mol_type = unassigned DNA
ccttcatactgggccaat

SEQ ID NO: 1114 - DNA, 17 bp, Zea mays;
  source 1..17: mol_type = unassigned DNA
cttcataccgggccaat

SEQ ID NO: 1115 - DNA, 22 bp, Zea mays;
  source 1..22: mol_type = unassigned DNA
ggcctcttgacaaatagcacaa

SEQ ID NO: 1116 - DNA, 23 bp, Zea mays;
  source 1..23: mol_type = unassigned DNA
cggagtaccagcaacatatagca

SEQ ID NO: 1117 - DNA, 14 bp, Zea mays;
  source 1..14: mol_type = unassigned DNA
cgggtacaggtggc

SEQ ID NO: 1118 - DNA, 15 bp, Zea mays;
  source 1..15: mol_type = unassigned DNA
cgggtacagatggcg

SEQ ID NO: 1119 - DNA, 17 bp, Zea mays;
  source 1..17: mol_type = unassigned DNA
gcacagccgcgtcaagt

SEQ ID NO: 1120 - DNA, 18 bp, Zea mays;
  source 1..18: mol_type = unassigned DNA
cgttgcccaccagagtcg

SEQ ID NO: 1121 - DNA, 13 bp, Zea mays;
  source 1..13: mol_type = unassigned DNA
cgacgccgctgct

SEQ ID NO: 1122 - DNA, 15 bp, Zea mays;
  source 1..15: mol_type = unassigned DNA
agagcgacaccgctg

SEQ ID NO: 1123 - DNA, 19 bp, Zea mays;
  source 1..19: mol_type = unassigned DNA
gagctcgtcacagccttcc

SEQ ID NO: 1124 - DNA, 19 bp, Zea mays;
  source 1..19: mol_type = unassigned DNA
aacccgagcctcgccgatt

SEQ ID NO: 1125 - DNA, 19 bp, Zea mays;
  source 1..19: mol_type = unassigned DNA
tgctgatactactcataca

SEQ ID NO: 1126 - DNA, 19 bp, Zea mays;
  source 1..19: mol_type = unassigned DNA
ctgatactgctactcatac

SEQ ID NO: 1127 - DNA, 21 bp, Zea mays;
  source 1..21: mol_type = unassigned DNA
gaatctttggttgcagcttgc

SEQ ID NO: 1128 - DNA, 21 bp, Zea mays;
  source 1..21: mol_type = unassigned DNA
tctgtgtcgatcccatgtgta

SEQ ID NO: 1129 - DNA, 18 bp, Zea mays;
  source 1..18: mol_type = unassigned DNA
accttttgatgagttcca

SEQ ID NO: 1130 - DNA, 17 bp, Zea mays;
  source 1..17: mol_type = unassigned DNA
accttttgatgagctcc

SEQ ID NO: 1131 - DNA, 19 bp, Zea mays;
  source 1..19: mol_type = unassigned DNA
aaacttgaattggtggagc

SEQ ID NO: 1132 - DNA, 18 bp, Zea mays;
  source 1..18: mol_type = unassigned DNA
gtgcacgtgtctctatac

SEQ ID NO: 1133 - DNA, 17 bp, Zea mays;
  source 1..17: mol_type = unassigned DNA
ttcatcaggaaacaact

SEQ ID NO: 1134 - DNA, 17 bp, Zea mays;
  source 1..17: mol_type = unassigned DNA
ttcatcaggaaacaaca

SEQ ID NO: 1135 - DNA, 17 bp, Zea mays;
  source 1..17: mol_type = unassigned DNA
ctcttgccaaggctgca

SEQ ID NO: 1136 - DNA, 22 bp, Zea mays;
  source 1..22: mol_type = unassigned DNA
ttcaagcattcgctgacttctg

SEQ ID NO: 1137 - DNA, 20 bp, Zea mays;
  source 1..20: mol_type = unassigned DNA
agtggtgaaccttgtgttat

SEQ ID NO: 1138 - DNA, 18 bp, Zea mays;
  source 1..18: mol_type = unassigned DNA
tggtgaacctcgtgttat

SEQ ID NO: 1139 - DNA, 20 bp, Zea mays;
  source 1..20: mol_type = unassigned DNA
gcgcacttgattggcattct

SEQ ID NO: 1140 - DNA, 20 bp, Zea mays;
  source 1..20: mol_type = unassigned DNA
cgcacacacacaaccaagac

SEQ ID NO: 1141 - DNA, 20 bp, Zea mays;
  source 1..20: mol_type = unassigned DNA
acaacgttcaccactaacac

SEQ ID NO: 1142 - DNA, 20 bp, Zea mays;
  source 1..20: mol_type = unassigned DNA
acaaggttcaccactaacac

SEQ ID NO: 1143 - DNA, 20 bp, Zea mays;
  source 1..20: mol_type = unassigned DNA
agagtgcgaagagcaacaca

SEQ ID NO: 1144 - DNA, 20 bp, Zea mays;
  source 1..20: mol_type = unassigned DNA
tagctgccttggggctataa

SEQ ID NO: 1145 - DNA, 17 bp, Zea mays;
  source 1..17: mol_type = unassigned DNA
tgccccccaggcggggt

SEQ ID NO: 1146 - DNA, 17 bp, Zea mays;
  source 1..17: mol_type = unassigned DNA
tgctccccaggcggggt

SEQ ID NO: 1147 - DNA, 20 bp, Zea mays;
  source 1..20: mol_type = unassigned DNA
agcagtgctcaatcggtctt

SEQ ID NO: 1148 - DNA, 20 bp, Zea mays;
  source 1..20: mol_type = unassigned DNA
gacccctccacctccttatc

SEQ ID NO: 1149 - DNA, 16 bp, Zea mays;
  source 1..16: mol_type = unassigned DNA
ctcaagcctgctggta

SEQ ID NO: 1150 - DNA, 17 bp, Zea mays;
  source 1..17: mol_type = unassigned DNA
tcaagcctgatggtaca

SEQ ID NO: 1151 - DNA, 22 bp, Zea mays;
  source 1..22: mol_type = unassigned DNA
gtgggttgtaagtgggtgttta

SEQ ID NO: 1152 - DNA, 25 bp, Zea mays;
  source 1..25: mol_type = unassigned DNA
ttctccttctttctgagtatagcct

SEQ ID NO: 1153 - DNA, 23 bp, Zea mays;
  source 1..23: mol_type = unassigned DNA
tccaaaaacttgttgttctccca

SEQ ID NO: 1154 - DNA, 23 bp, Zea mays;
  source 1..23: mol_type = unassigned DNA
tccaaaaaattgttgttctccca

SEQ ID NO: 1155 - DNA, 20 bp, Zea mays;
  source 1..20: mol_type = unassigned DNA
tcgtcttctcgtatgcatgg

SEQ ID NO: 1156 - DNA, 20 bp, Zea mays;
  source 1..20: mol_type = unassigned DNA
tgcgacaaaattgacgaaga

SEQ ID NO: 1157 - DNA, 21 bp, Zea mays;
  source 1..21: mol_type = unassigned DNA
aatgggagaacaacaagtttt

SEQ ID NO: 1158 - DNA, 19 bp, Zea mays;
  source 1..19: mol_type = unassigned DNA
tgggagaacaacacgtttt

SEQ ID NO: 1159 - DNA, 19 bp, Zea mays;
  source 1..19: mol_type = unassigned DNA
cagtgcatccacggtggtc

SEQ ID NO: 1160 - DNA, 25 bp, Zea mays;
  source 1..25: mol_type = unassigned DNA
ctttgctttcttgaacagacttggt

SEQ ID NO: 1161 - DNA, 17 bp, Zea mays;
  source 1..17: mol_type = unassigned DNA
attcgtaacaccagcct

SEQ ID NO: 1162 - DNA, 14 bp, Zea mays;
  source 1..14: mol_type = unassigned DNA
cgtaaccccagcct

SEQ ID NO: 1163 - DNA, 15 bp, Zea mays;
  source 1..15: mol_type = unassigned DNA
tgcgcatcgcagcag

SEQ ID NO: 1164 - DNA, 19 bp, Zea mays;
  source 1..19: mol_type = unassigned DNA
acagacagcaggcctcaac

SEQ ID NO: 1165 - DNA, 19 bp, Zea mays;
  source 1..19: mol_type = unassigned DNA
tgattaattcgtctgacca

SEQ ID NO: 1166 - DNA, 20 bp, Zea mays;
  source 1..20: mol_type = unassigned DNA
ttgattaattcatctgacca

SEQ ID NO: 1167 - DNA, 24 bp, Zea mays;
  source 1..24: mol_type = unassigned DNA
tgagatggttgtgttatgactcca

SEQ ID NO: 1168 - DNA, 22 bp, Zea mays;
  source 1..22: mol_type = unassigned DNA
tccgacacccagaatcaaatgg

SEQ ID NO: 1169 - DNA, 17 bp, Zea mays;
  source 1..17: mol_type = unassigned DNA
cccgacacctgtccttc

SEQ ID NO: 1170 - DNA, 17 bp, Zea mays;
  source 1..17: mol_type = unassigned DNA
cccgacagctgtccttc

SEQ ID NO: 1171 - DNA, 20 bp, Zea mays;
  source 1..20: mol_type = unassigned DNA
ggagacgtcagcaaggactc

SEQ ID NO: 1172 - DNA, 20 bp, Zea mays;
  source 1..20: mol_type = unassigned DNA
agccctggaccttcctttta

SEQ ID NO: 1173 - DNA, 24 bp, Zea mays;
  source 1..24: mol_type = unassigned DNA
aaagatgaagaaacaatcaatgta

SEQ ID NO: 1174 - DNA, 21 bp, Zea mays;
  source 1..21: mol_type = unassigned DNA
tgaagaaacaatccatgtata

SEQ ID NO: 1175 - DNA, 17 bp, Zea mays;
  source 1..17: mol_type = unassigned DNA
gtggtgcaagcgtggtc

SEQ ID NO: 1176 - DNA, 24 bp, Zea mays;
  source 1..24: mol_type = unassigned DNA
gtgcaaaggttgcttggaattgag

SEQ ID NO: 1177 - DNA, 21 bp, Zea mays;
  source 1..21: mol_type = unassigned DNA
ttcaaggtttttttgcaaata

SEQ ID NO: 1178 - DNA, 21 bp, Zea mays;
  source 1..21: mol_type = unassigned DNA
ttcaaggttcttttgcaaata

SEQ ID NO: 1179 - DNA, 20 bp, Zea mays;
  source 1..20: mol_type = unassigned DNA
gtgcaaaggttgcttggaat

SEQ ID NO: 1180 - DNA, 20 bp, Zea mays;
  source 1..20: mol_type = unassigned DNA
ccaaaggaaaggcatttgaa

SEQ ID NO: 1181 - DNA, 21 bp, Zea mays;
  source 1..21: mol_type = unassigned DNA
catttacctttgattatttgc

SEQ ID NO: 1182 - DNA, 19 bp, Zea mays;
  source 1..19: mol_type = unassigned DNA
ttacctttgactatttgca

SEQ ID NO: 1183 - DNA, 25 bp, Zea mays;
  source 1..25: mol_type = unassigned DNA
ccaaaggaaaggcatttgaaacagg

SEQ ID NO: 1184 - DNA, 19 bp, Zea mays;
  source 1..19: mol_type = unassigned DNA
gaccacgcttgcaccacat

SEQ ID NO: 1185 - DNA, 18 bp, Zea mays;
  source 1..18: mol_type = unassigned DNA
tcagggcgagatgaaacg

SEQ ID NO: 1186 - DNA, 18 bp, Zea mays;
  source 1..18: mol_type = unassigned DNA
atcagggcgagacgaaac

SEQ ID NO: 1187 - DNA, 23 bp, Zea mays;
  source 1..23: mol_type = unassigned DNA
gggtagctttgttcccaaggatt

SEQ ID NO: 1188 - DNA, 22 bp, Zea mays;
  source 1..22: mol_type = unassigned DNA
tggagaggtggacaggtagtag

SEQ ID NO: 1189 - DNA, 17 bp, Zea mays;
  source 1..17: mol_type = unassigned DNA
cgactggatcagcgaag

SEQ ID NO: 1190 - DNA, 18 bp, Zea mays;
  source 1..18: mol_type = unassigned DNA
cacgactggattagcgaa

SEQ ID NO: 1191 - DNA, 17 bp, Zea mays;
  source 1..17: mol_type = unassigned DNA
gcgcacaagccgtctac

SEQ ID NO: 1192 - DNA, 21 bp, Zea mays;
  source 1..21: mol_type = unassigned DNA
gacgcccttgctgtatgtatg

SEQ ID NO: 1193 - DNA, 17 bp, Zea mays;
  source 1..17: mol_type = unassigned DNA
tcttggagttgcttgac

SEQ ID NO: 1194 - DNA, 17 bp, Zea mays;
  source 1..17: mol_type = unassigned DNA
ctcttggagtggcttga

SEQ ID NO: 1195 - DNA, 24 bp, Zea mays;
  source 1..24: mol_type = unassigned DNA
tgagtgtacttcgtttggctaatg

SEQ ID NO: 1196 - DNA, 25 bp, Zea mays;
  source 1..25: mol_type = unassigned DNA
aggatcatgacacagaaattcgaga

SEQ ID NO: 1197 - DNA, 17 bp, Zea mays;
  source 1..17: mol_type = unassigned DNA
tcttggagttgcttgac

SEQ ID NO: 1198 - DNA, 17 bp, Zea mays;
  source 1..17: mol_type = unassigned DNA
ctcttggaggtgcttga

SEQ ID NO: 1199 - DNA, 24 bp, Zea mays;
  source 1..24: mol_type = unassigned DNA
tgagtgtacttcgtttggctaatg

SEQ ID NO: 1200 - DNA, 25 bp, Zea mays;
  source 1..25: mol_type = unassigned DNA
aggatcatgacacagaaattcgaga

SEQ ID NO: 1201 - DNA, 27 bp, Zea mays;
  source 1..27: mol_type = unassigned DNA
acttctagagaaaaaaaaaaaaataga

SEQ ID NO: 1202 - DNA, 27 bp, Zea mays;
  source 1..27: mol_type = unassigned DNA
acttctagagaaaaaataaaaaataga

SEQ ID NO: 1203 - DNA, 20 bp, Zea mays;
  source 1..20: mol_type = unassigned DNA
acctccttttggtccgtttt

SEQ ID NO: 1204 - DNA, 20 bp, Zea mays;
  source 1..20: mol_type = unassigned DNA
ggaggcaagtgaggagactg

SEQ ID NO: 1205 - DNA, 19 bp, Zea mays;
  source 1..19: mol_type = unassigned DNA
attaggttgtttccagcaa

SEQ ID NO: 1206 - DNA, 16 bp, Zea mays;
  source 1..16: mol_type = unassigned DNA
aggttgttcccagcaa

SEQ ID NO: 1207 - DNA, 22 bp, Zea mays;
  source 1..22: mol_type = unassigned DNA
tgttgggcaatcaaacttcagg

SEQ ID NO: 1208 - DNA, 21 bp, Zea mays;
  source 1..21: mol_type = unassigned DNA
aggccacggtgaccatgtaag

SEQ ID NO: 1209 - DNA, 19 bp, Zea mays;
  source 1..19: mol_type = unassigned DNA
tctactctgaggctgtatt

SEQ ID NO: 1210 - DNA, 21 bp, Zea mays;
  source 1..21: mol_type = unassigned DNA
tctactctgaggttgtatttg

SEQ ID NO: 1211 - DNA, 24 bp, Zea mays;
  source 1..24: mol_type = unassigned DNA
gcaacatgatctcttcaccaatga

SEQ ID NO: 1212 - DNA, 22 bp, Zea mays;
  source 1..22: mol_type = unassigned DNA
caaccagctcaccagaacaatg

SEQ ID NO: 1213 - DNA, 17 bp, Zea mays;
  source 1..17: mol_type = unassigned DNA
cgtcgagatcctcattc

SEQ ID NO: 1214 - DNA, 19 bp, Zea mays;
  source 1..19: mol_type = unassigned DNA
acgtcgagatcttcattca

SEQ ID NO: 1215 - DNA, 19 bp, Zea mays;
  source 1..19: mol_type = unassigned DNA
tcggagccttggatcatca

SEQ ID NO: 1216 - DNA, 21 bp, Zea mays;
  source 1..21: mol_type = unassigned DNA
gcccgatcttccgtgagatac

SEQ ID NO: 1217 - DNA, 15 bp, Zea mays;
  source 1..15: mol_type = unassigned DNA
accctccctccgaaa

SEQ ID NO: 1218 - DNA, 15 bp, Zea mays;
  source 1..15: mol_type = unassigned DNA
accctcgctccgaaa

SEQ ID NO: 1219 - DNA, 21 bp, Zea mays;
  source 1..21: mol_type = unassigned DNA
cgccttccagtccacaatctc

SEQ ID NO: 1220 - DNA, 21 bp, Zea mays;
  source 1..21: mol_type = unassigned DNA
gcggtctctctctctctctct

SEQ ID NO: 1221 - DNA, 20 bp, Zea mays;
  source 1..20: mol_type = unassigned DNA
aacagtagtatcttgtgcat

SEQ ID NO: 1222 - DNA, 20 bp, Zea mays;
  source 1..20: mol_type = unassigned DNA
aacagtagtattttgtgcat

SEQ ID NO: 1223 - DNA, 25 bp, Zea mays;
  source 1..25: mol_type = unassigned DNA
agccgctcactttgtggtattcatc

SEQ ID NO: 1224 - DNA, 22 bp, Zea mays;
  source 1..22: mol_type = unassigned DNA
agtacggatagtcccatgttca

SEQ ID NO: 1225 - DNA, 17 bp, Zea mays;
  source 1..17: mol_type = unassigned DNA
cacaaagtgagcggctt

SEQ ID NO: 1226 - DNA, 17 bp, Zea mays;
  source 1..17: mol_type = unassigned DNA
cacaaagtgtgcggctt

SEQ ID NO: 1227 - DNA, 23 bp, Zea mays;
  source 1..23: mol_type = unassigned DNA
tctagcttcattgtgcagggatg

SEQ ID NO: 1228 - DNA, 22 bp, Zea mays;
  source 1..22: mol_type = unassigned DNA
gagatcttgagggtgtcccaaa

SEQ ID NO: 1229 - DNA, 20 bp, Zea mays;
  source 1..20: mol_type = unassigned DNA
ccattgctcaggagttagaa

SEQ ID NO: 1230 - DNA, 18 bp, Zea mays;
  source 1..18: mol_type = unassigned DNA
tgctcaggagctagaaac

SEQ ID NO: 1231 - DNA, 22 bp, Zea mays;
  source 1..22: mol_type = unassigned DNA
catcaagggactccgagcttct

SEQ ID NO: 1232 - DNA, 24 bp, Zea mays;
  source 1..24: mol_type = unassigned DNA
cagcttcctcggcaactttaacag

SEQ ID NO: 1233 - DNA, 18 bp, Zea mays;
  source 1..18: mol_type = unassigned DNA
catcctttgctgatagca

SEQ ID NO: 1234 - DNA, 16 bp, Zea mays;
  source 1..16: mol_type = unassigned DNA
tcctttgccgatagca

SEQ ID NO: 1235 - DNA, 21 bp, Zea mays;
  source 1..21: mol_type = unassigned DNA
agctcggagtcccttgatggt

SEQ ID NO: 1236 - DNA, 20 bp, Zea mays;
  source 1..20: mol_type = unassigned DNA
cgaagtgacccgccttacac

SEQ ID NO: 1237 - DNA, 18 bp, Zea mays;
  source 1..18: mol_type = unassigned DNA
tgttggaatctcggtaca

SEQ ID NO: 1238 - DNA, 17 bp, Zea mays;
  source 1..17: mol_type = unassigned DNA
tgttggaatcccggtac

SEQ ID NO: 1239 - DNA, 19 bp, Zea mays;
  source 1..19: mol_type = unassigned DNA
tccaagatggtcagcgagt

SEQ ID NO: 1240 - DNA, 19 bp, Zea mays;
  source 1..19: mol_type = unassigned DNA
cgcgacaacctggacagat

SEQ ID NO: 1241 - DNA, 20 bp, Zea mays;
  source 1..20: mol_type = unassigned DNA
tcaggtactctacaaactct

SEQ ID NO: 1242 - DNA, 19 bp, Zea mays;
  source 1..19: mol_type = unassigned DNA
caggtactctaccaactct

SEQ ID NO: 1243 - DNA, 21 bp, Zea mays;
  source 1..21: mol_type = unassigned DNA
gaccagagagctgacaggaac

SEQ ID NO: 1244 - DNA, 22 bp, Zea mays;
  source 1..22: mol_type = unassigned DNA
gctctgtggcgtgagatagatg

SEQ ID NO: 1245 - DNA, 16 bp, Zea mays;
  source 1..16: mol_type = unassigned DNA
catatccgggcagtcc

SEQ ID NO: 1246 - DNA, 17 bp, Zea mays;
  source 1..17: mol_type = unassigned DNA
ccatatccggacagtcc

SEQ ID NO: 1247 - DNA, 20 bp, Zea mays;
  source 1..20: mol_type = unassigned DNA
gagttggatggtccagcgta

SEQ ID NO: 1248 - DNA, 19 bp, Zea mays;
  source 1..19: mol_type = unassigned DNA
ggaccgtccgccatcttac

SEQ ID NO: 1249 - DNA, 20 bp, Zea mays;
  source 1..20: mol_type = unassigned DNA
aagcctttttcacctctttt

SEQ ID NO: 1250 - DNA, 20 bp, Zea mays;
  source 1..20: mol_type = unassigned DNA
aagcctttttcacttctttt

SEQ ID NO: 1251 - DNA, 21 bp, Zea mays;
  source 1..21: mol_type = unassigned DNA
gctgagtcttggctgtacaca

SEQ ID NO: 1252 - DNA, 21 bp, Zea mays;
  source 1..21: mol_type = unassigned DNA
gagtgccaacacaagtgctta

SEQ ID NO: 1253 - DNA, 21 bp, Zea mays;
  source 1..21: mol_type = unassigned DNA
aataatgtgtggtgaatgcga

SEQ ID NO: 1254 - DNA, 21 bp, Zea mays;
  source 1..21: mol_type = unassigned DNA
aataatgcgtggtgaatgcga

SEQ ID NO: 1255 - DNA, 20 bp, Zea mays;
  source 1..20: mol_type = unassigned DNA
aaatgcaatcgaggctgaac

SEQ ID NO: 1256 - DNA, 20 bp, Zea mays;
  source 1..20: mol_type = unassigned DNA
ttcatgccatttgccagata

SEQ ID NO: 1257 - DNA, 16 bp, Zea mays;
  source 1..16: mol_type = unassigned DNA
tcttgtgggagaccca

SEQ ID NO: 1258 - DNA, 19 bp, Zea mays;
  source 1..19: mol_type = unassigned DNA
caaggtcttgtgagagacc

SEQ ID NO: 1259 - DNA, 25 bp, Zea mays;
  source 1..25: mol_type = unassigned DNA
gttcggacatttatgggcactattg

SEQ ID NO: 1260 - DNA, 25 bp, Zea mays;
  source 1..25: mol_type = unassigned DNA
cctaggatctcatgatggatcttca

SEQ ID NO: 1261 - DNA, 16 bp, Zea mays;
  source 1..16: mol_type = unassigned DNA
agcaaagtgggcgtcc

SEQ ID NO: 1262 - DNA, 17 bp, Zea mays;
  source 1..17: mol_type = unassigned DNA
agcaaagtaggcgtcca

SEQ ID NO: 1263 - DNA, 25 bp, Zea mays;
  source 1..25: mol_type = unassigned DNA
gctatctcaattctttggtcacatc

SEQ ID NO: 1264 - DNA, 21 bp, Zea mays;
  source 1..21: mol_type = unassigned DNA
aggtggcaaccagttgttagg

SEQ ID NO: 1265 - DNA, 21 bp, Zea mays;
  source 1..21: mol_type = unassigned DNA
ttggtatcttattattgtcaa

SEQ ID NO: 1266 - DNA, 20 bp, Zea mays;
  source 1..20: mol_type = unassigned DNA
tggtatcttattcttgtcaa

SEQ ID NO: 1267 - DNA, 22 bp, Zea mays;
  source 1..22: mol_type = unassigned DNA
ctttgagtagtgcggcagtgat

SEQ ID NO: 1268 - DNA, 20 bp, Zea mays;
  source 1..20: mol_type = unassigned DNA
ggtggtggacgcctactttg

SEQ ID NO: 1269 - DNA, 15 bp, Zea mays;
  source 1..15: mol_type = unassigned DNA
cctcgggggctaaaa

SEQ ID NO: 1270 - DNA, 15 bp, Zea mays;
  source 1..15: mol_type = unassigned DNA
cctcgggggctcaaa

SEQ ID NO: 1271 - DNA, 20 bp, Zea mays;
  source 1..20: mol_type = unassigned DNA
cagctacgtcgcttctaccc

SEQ ID NO: 1272 - DNA, 20 bp, Zea mays;
  source 1..20: mol_type = unassigned DNA
acgtgtacctcgtcgtttcc

SEQ ID NO: 1273 - DNA, 17 bp, Zea mays;
  source 1..17: mol_type = unassigned DNA
tgtaaaatctggccgta

SEQ ID NO: 1274 - DNA, 19 bp, Zea mays;
  source 1..19: mol_type = unassigned DNA
tgtaaaatctggctgtaag

SEQ ID NO: 1275 - DNA, 20 bp, Zea mays;
  source 1..20: mol_type = unassigned DNA
caccagtttcgtgtcaagga

SEQ ID NO: 1276 - DNA, 22 bp, Zea mays;
  source 1..22: mol_type = unassigned DNA
ttccgcccgagagatttagaag

SEQ ID NO: 1277 - DNA, 18 bp, Zea mays;
  source 1..18: mol_type = unassigned DNA
ttaccaggaacagtaaac

SEQ ID NO: 1278 - DNA, 18 bp, Zea mays;
  source 1..18: mol_type = unassigned DNA
taccaggaacaataaaca

SEQ ID NO: 1279 - DNA, 17 bp, Zea mays;
  source 1..17: mol_type = unassigned DNA
ttccactatcgaccgaa

SEQ ID NO: 1280 - DNA, 20 bp, Zea mays;
  source 1..20: mol_type = unassigned DNA
gggatttgaggttatgttct

SEQ ID NO: 1281 - DNA, 17 bp, Zea mays;
  source 1..17: mol_type = unassigned DNA
ccgagcgtgagttactt

SEQ ID NO: 1282 - DNA, 18 bp, Zea mays;
  source 1..18: mol_type = unassigned DNA
ccgagcgtgaattacttt

SEQ ID NO: 1283 - DNA, 21 bp, Zea mays;
  source 1..21: mol_type = unassigned DNA
ttcgtcggtagcagaatcact

SEQ ID NO: 1284 - DNA, 23 bp, Zea mays;
  source 1..23: mol_type = unassigned DNA
acggatacctcactcatcacctt

SEQ ID NO: 1285 - DNA, 19 bp, Zea mays;
  source 1..19: mol_type = unassigned DNA
tcacatcttgcataaataa

SEQ ID NO: 1286 - DNA, 19 bp, Zea mays;
  source 1..19: mol_type = unassigned DNA
cacatcttgcataaagaat

SEQ ID NO: 1287 - DNA, 22 bp, Zea mays;
  source 1..22: mol_type = unassigned DNA
atgggacaaagagtctagcatt

SEQ ID NO: 1288 - DNA, 19 bp, Zea mays;
  source 1..19: mol_type = unassigned DNA
ggttcaatcaacaatcaca

SEQ ID NO: 1289 - DNA, 19 bp, Zea mays;
  source 1..19: mol_type = unassigned DNA
cttgattcagtccgagaag

SEQ ID NO: 1290 - DNA, 16 bp, Zea mays;
  source 1..16: mol_type = unassigned DNA
ttgattcagcccgaga

SEQ ID NO: 1291 - DNA, 22 bp, Zea mays;
  source 1..22: mol_type = unassigned DNA
cagtatagctcggtgttgctca

SEQ ID NO: 1292 - DNA, 19 bp, Zea mays;
  source 1..19: mol_type = unassigned DNA
cgcgtggaacagggtagag

SEQ ID NO: 1293 - DNA, 19 bp, Zea mays;
  source 1..19: mol_type = unassigned DNA
cctccataatgattagatc

SEQ ID NO: 1294 - DNA, 19 bp, Zea mays;
  source 1..19: mol_type = unassigned DNA
cctccataatgagtagatc

SEQ ID NO: 1295 - DNA, 25 bp, Zea mays;
  source 1..25: mol_type = unassigned DNA
cctacgatcgatttctaagcgtcta

SEQ ID NO: 1296 - DNA, 22 bp, Zea mays;
  source 1..22: mol_type = unassigned DNA
gcgacaactctccaacaacaac

SEQ ID NO: 1297 - DNA, 17 bp, Zea mays;
  source 1..17: mol_type = unassigned DNA
agtccattggaggttcg

SEQ ID NO: 1298 - DNA, 17 bp, Zea mays;
  source 1..17: mol_type = unassigned DNA
agtccattggagattcg

SEQ ID NO: 1299 - DNA, 21 bp, Zea mays;
  source 1..21: mol_type = unassigned DNA
tttgggcatcacttgtctcaa

SEQ ID NO: 1300 - DNA, 19 bp, Zea mays;
  source 1..19: mol_type = unassigned DNA
gcgatgccacggaacataa

SEQ ID NO: 1301 - DNA, 15 bp, Zea mays;
  source 1..15: mol_type = unassigned DNA
acgatcatggcctgg

SEQ ID NO: 1302 - DNA, 15 bp, Zea mays;
  source 1..15: mol_type = unassigned DNA
acgatcatggcgtgg

SEQ ID NO: 1303 - DNA, 18 bp, Zea mays;
  source 1..18: mol_type = unassigned DNA
cggcgtggcatacaagga

SEQ ID NO: 1304 - DNA, 20 bp, Zea mays;
  source 1..20: mol_type = unassigned DNA
caacgcggctcgttcatcag

SEQ ID NO: 1305 - DNA, 16 bp, Zea mays;
  source 1..16: mol_type = unassigned DNA
tgatgaccctgttggg

SEQ ID NO: 1306 - DNA, 15 bp, Zea mays;
  source 1..15: mol_type = unassigned DNA
tgatgaccccgttgg

SEQ ID NO: 1307 - DNA, 18 bp, Zea mays;
  source 1..18: mol_type = unassigned DNA
gcgtgtcggtacgtggat

SEQ ID NO: 1308 - DNA, 20 bp, Zea mays;
  source 1..20: mol_type = unassigned DNA
accatgctacgccaagttca

SEQ ID NO: 1309 - DNA, 20 bp, Zea mays;
  source 1..20: mol_type = unassigned DNA
ttttcaggcagcttttataa

SEQ ID NO: 1310 - DNA, 19 bp, Zea mays;
  source 1..19: mol_type = unassigned DNA
ttcaggcagcttctataaa

SEQ ID NO: 1311 - DNA, 21 bp, Zea mays;
  source 1..21: mol_type = unassigned DNA
gcagactgcaaaacacttagc

SEQ ID NO: 1312 - DNA, 25 bp, Zea mays;
  source 1..25: mol_type = unassigned DNA
ggtttgaccctatttctctttcaca

SEQ ID NO: 1313 - DNA, 13 bp, Zea mays;
  source 1..13: mol_type = unassigned DNA
cccggcggtggaa

SEQ ID NO: 1314 - DNA, 13 bp, Zea mays;
  source 1..13: mol_type = unassigned DNA
tcgcccgacggtg

SEQ ID NO: 1315 - DNA, 16 bp, Zea mays;
  source 1..16: mol_type = unassigned DNA
tgtcggccgccattgt

SEQ ID NO: 1316 - DNA, 22 bp, Zea mays;
  source 1..22: mol_type = unassigned DNA
gacgacagctacgacatgatac

SEQ ID NO: 1317 - DNA, 18 bp, Zea mays;
  source 1..18: mol_type = unassigned DNA
attggatggcctggaggc

SEQ ID NO: 1318 - DNA, 16 bp, Zea mays;
  source 1..16: mol_type = unassigned DNA
ttggatggcccggagg

SEQ ID NO: 1319 - DNA, 25 bp, Zea mays;
  source 1..25: mol_type = unassigned DNA
gacgttagagaccttgaagttagga

SEQ ID NO: 1320 - DNA, 21 bp, Zea mays;
  source 1..21: mol_type = unassigned DNA
gtcgcgaacatcgacaagaag

SEQ ID NO: 1321 - DNA, 15 bp, Zea mays;
  source 1..15: mol_type = unassigned DNA
cttttcgctacagct

SEQ ID NO: 1322 - DNA, 17 bp, Zea mays;
  source 1..17: mol_type = unassigned DNA
ttcttttcgctacaact

SEQ ID NO: 1323 - DNA, 18 bp, Zea mays;
  source 1..18: mol_type = unassigned DNA
ggtagcacattgcatagg

SEQ ID NO: 1324 - DNA, 22 bp, Zea mays;
  source 1..22: mol_type = unassigned DNA
gctcaatacagtaattcctcat

SEQ ID NO: 1325 - DNA, 15 bp, Zea mays;
  source 1..15: mol_type = unassigned DNA
caacgctcacttacc

SEQ ID NO: 1326 - DNA, 14 bp, Zea mays;
  source 1..14: mol_type = unassigned DNA
aacgctcgcttacc

SEQ ID NO: 1327 - DNA, 23 bp, Zea mays;
  source 1..23: mol_type = unassigned DNA
caagcagaggaagggacattcat

SEQ ID NO: 1328 - DNA, 27 bp, Zea mays;
  source 1..27: mol_type = unassigned DNA
gggtagctgtccgaatttaatagaaga

SEQ ID NO: 1329 - DNA, 18 bp, Zea mays;
  source 1..18: mol_type = unassigned DNA
tttatttgaatggctata

SEQ ID NO: 1330 - DNA, 20 bp, Zea mays;
  source 1..20: mol_type = unassigned DNA
tttatttgaatgactatata

SEQ ID NO: 1331 - DNA, 24 bp, Zea mays;
  source 1..24: mol_type = unassigned DNA
agggcagtcagcacaagttagaag

SEQ ID NO: 1332 - DNA, 18 bp, Zea mays;
  source 1..18: mol_type = unassigned DNA
atgtggccggtgaagtgt

SEQ ID NO: 1333 - DNA, 15 bp, Zea mays;
  source 1..15: mol_type = unassigned DNA
ctgccgtcatcgtcg

SEQ ID NO: 1334 - DNA, 13 bp, Zea mays;
  source 1..13: mol_type = unassigned DNA
ccgtcaccgtcgc

SEQ ID NO: 1335 - DNA, 18 bp, Zea mays;
  source 1..18: mol_type = unassigned DNA
ccggtcgtcaccgtcatc

SEQ ID NO: 1336 - DNA, 22 bp, Zea mays;
  source 1..22: mol_type = unassigned DNA
tggactctccgactcctctaag

SEQ ID NO: 1337 - DNA, 17 bp, Zea mays;
  source 1..17: mol_type = unassigned DNA
ctaaggtccgtcaaagc

SEQ ID NO: 1338 - DNA, 19 bp, Zea mays;
  source 1..19: mol_type = unassigned DNA
aactaaggtccatcaaagc

SEQ ID NO: 1339 - DNA, 25 bp, Zea mays;
  source 1..25: mol_type = unassigned DNA
cgaggcccactaaatatagactcag

SEQ ID NO: 1340 - DNA, 24 bp, Zea mays;
  source 1..24: mol_type = unassigned DNA
aggtattggttctcgaaggcttat

SEQ ID NO: 1341 - DNA, 23 bp, Zea mays;
  source 1..23: mol_type = unassigned DNA
taaatgagacaacgatagatata

SEQ ID NO: 1342 - DNA, 20 bp, Zea mays;
  source 1..20: mol_type = unassigned DNA
tgagacaacgacagatataa

SEQ ID NO: 1343 - DNA, 20 bp, Zea mays;
  source 1..20: mol_type = unassigned DNA
accatagctcttgctcacga

SEQ ID NO: 1344 - DNA, 22 bp, Zea mays;
  source 1..22: mol_type = unassigned DNA
ccacttgttatgaggcaggtca

SEQ ID NO: 1345 - DNA, 12 bp, Zea mays;
  source 1..12: mol_type = unassigned DNA
cggcagacgcgc

SEQ ID NO: 1346 - DNA, 13 bp, Zea mays;
  source 1..13: mol_type = unassigned DNA
cggcagacgcacc

SEQ ID NO: 1347 - DNA, 16 bp, Zea mays;
  source 1..16: mol_type = unassigned DNA
cgggttcggcgagacg

SEQ ID NO: 1348 - DNA, 18 bp, Zea mays;
  source 1..18: mol_type = unassigned DNA
tggcctcacggttctgaa

SEQ ID NO: 1349 - DNA, 17 bp, Zea mays;
  source 1..17: mol_type = unassigned DNA
agagttctttgggtctc

SEQ ID NO: 1350 - DNA, 20 bp, Zea mays;
  source 1..20: mol_type = unassigned DNA
agagttctttgagtctcttt

SEQ ID NO: 1351 - DNA, 25 bp, Zea mays;
  source 1..25: mol_type = unassigned DNA
tgtcagtattgttccatgcacagtt

SEQ ID NO: 1352 - DNA, 22 bp, Zea mays;
  source 1..22: mol_type = unassigned DNA
tgatgccactaccacgattgtc

SEQ ID NO: 1353 - DNA, 18 bp, Zea mays;
  source 1..18: mol_type = unassigned DNA
agaggtaccgtccgtttc

SEQ ID NO: 1354 - DNA, 18 bp, Zea mays;
  source 1..18: mol_type = unassigned DNA
caagaggtaccatccgtt

SEQ ID NO: 1355 - DNA, 19 bp, Zea mays;
  source 1..19: mol_type = unassigned DNA
gacgcgacttcgtcaccat

SEQ ID NO: 1356 - DNA, 18 bp, Zea mays;
  source 1..18: mol_type = unassigned DNA
gcgggtcgaagctgaatc

SEQ ID NO: 1357 - DNA, 23 bp, Zea mays;
  source 1..23: mol_type = unassigned DNA
cgaataacagaatagttgagaac

SEQ ID NO: 1358 - DNA, 23 bp, Zea mays;
  source 1..23: mol_type = unassigned DNA
cgaataacagaatacttgagaac

SEQ ID NO: 1359 - DNA, 24 bp, Zea mays;
  source 1..24: mol_type = unassigned DNA
gggcaactgaatatacaaccttga

SEQ ID NO: 1360 - DNA, 21 bp, Zea mays;
  source 1..21: mol_type = unassigned DNA
gacacctttgggcatattgga

SEQ ID NO: 1361 - DNA, 19 bp, Zea mays;
  source 1..19: mol_type = unassigned DNA
tgcgttaaggtttatttct

SEQ ID NO: 1362 - DNA, 18 bp, Zea mays;
  source 1..18: mol_type = unassigned DNA
tgcgttaaggtttagttc

SEQ ID NO: 1363 - DNA, 25 bp, Zea mays;
  source 1..25: mol_type = unassigned DNA
tcacgattttgaagtagtcgagtca

SEQ ID NO: 1364 - DNA, 18 bp, Zea mays;
  source 1..18: mol_type = unassigned DNA
tgcagcccaaaacagcaa

SEQ ID NO: 1365 - DNA, 15 bp, Zea mays;
  source 1..15: mol_type = unassigned DNA
cacagccctgccttg

SEQ ID NO: 1366 - DNA, 14 bp, Zea mays;
  source 1..14: mol_type = unassigned DNA
acagccccgccttg

SEQ ID NO: 1367 - DNA, 19 bp, Zea mays;
  source 1..19: mol_type = unassigned DNA
atagacggcctccggtcac

SEQ ID NO: 1368 - DNA, 24 bp, Zea mays;
  source 1..24: mol_type = unassigned DNA
tgctacggcacaataaatgaatga

SEQ ID NO: 1369 - DNA, 19 bp, Zea mays;
  source 1..19: mol_type = unassigned DNA
aatcccttaatgtgtcttc

SEQ ID NO: 1370 - DNA, 18 bp, Zea mays;
  source 1..18: mol_type = unassigned DNA
aatcccttaatgcgtctt

SEQ ID NO: 1371 - DNA, 18 bp, Zea mays;
  source 1..18: mol_type = unassigned DNA
ttgcatcgccaataccca

SEQ ID NO: 1372 - DNA, 25 bp, Zea mays;
  source 1..25: mol_type = unassigned DNA
tttgtgaacattactcctttgtgtc

SEQ ID NO: 1373 - DNA, 20 bp, Zea mays;
  source 1..20: mol_type = unassigned DNA
cattgtttattacagttcct

SEQ ID NO: 1374 - DNA, 21 bp, Zea mays;
  source 1..21: mol_type = unassigned DNA
cattgtttattaaagttccta

SEQ ID NO: 1375 - DNA, 20 bp, Zea mays;
  source 1..20: mol_type = unassigned DNA
agccgagcaagggtaatggt

SEQ ID NO: 1376 - DNA, 25 bp, Zea mays;
  source 1..25: mol_type = unassigned DNA
ggaagtaaaggaccctctgaaatgt

SEQ ID NO: 1377 - DNA, 18 bp, Zea mays;
  source 1..18: mol_type = unassigned DNA
aatccgtgtcttctctgt

SEQ ID NO: 1378 - DNA, 19 bp, Zea mays;
  source 1..19: mol_type = unassigned DNA
aaatccgtgtattctctgt

SEQ ID NO: 1379 - DNA, 15 bp, Zea mays;
  source 1..15: mol_type = unassigned DNA
cggcgcccgtggttt

SEQ ID NO: 1380 - DNA, 25 bp, Zea mays;
  source 1..25: mol_type = unassigned DNA
gagagatagagggagtcagggagat

SEQ ID NO: 1381 - DNA, 14 bp, Zea mays;
  source 1..14: mol_type = unassigned DNA
cgtctgcagctgac

SEQ ID NO: 1382 - DNA, 13 bp, Zea mays;
  source 1..13: mol_type = unassigned DNA
cgtctgcagccga

SEQ ID NO: 1383 - DNA, 20 bp, Zea mays;
  source 1..20: mol_type = unassigned DNA
acactcgacaaggcgtcgtc

SEQ ID NO: 1384 - DNA, 22 bp, Zea mays;
  source 1..22: mol_type = unassigned DNA
ctcgagactcacaagctatcac

SEQ ID NO: 1385 - DNA, 14 bp, Zea mays;
  source 1..14: mol_type = unassigned DNA
acagtccggtgcac

SEQ ID NO: 1386 - DNA, 14 bp, Zea mays;
  source 1..14: mol_type = unassigned DNA
cggacagtccgctg

SEQ ID NO: 1387 - DNA, 16 bp, Zea mays;
  source 1..16: mol_type = unassigned DNA
cgagagcagcaagttc

SEQ ID NO: 1388 - DNA, 18 bp, Zea mays;
  source 1..18: mol_type = unassigned DNA
gaagagatggccttgttc

SEQ ID NO: 1389 - DNA, 18 bp, Zea mays;
  source 1..18: mol_type = unassigned DNA
ccaaaaggtactgtccgt

SEQ ID NO: 1390 - DNA, 17 bp, Zea mays;
  source 1..17: mol_type = unassigned DNA
caaaaggtaccgtccgt

SEQ ID NO: 1391 - DNA, 18 bp, Zea mays;
  source 1..18: mol_type = unassigned DNA
acgcgacttcaccaccgt

SEQ ID NO: 1392 - DNA, 21 bp, Zea mays;
  source 1..21: mol_type = unassigned DNA
ttggtggatcgaagctgaatc